European Patent Application EP 4 748 936 A1, published May 27, 2026. Title: フルクトシルアミノ酸オキシダーゼ、遺伝子、発現ベクター、糖化タンパク質センサ、糖化タンパク質の測定方法、及びフルクトシルアミノ酸オキシダーゼの製造方法. Applicant: PROVIGATE Inc. The sequence listing filed with the application follows.

SEQUENCE LISTING (218 sequences)

SEQ ID NO: 1 - protein, 446 aa, Aspergillus pseudotamarii
MASSNLTLTSSILIVGAGTWGCSTALHLARRGYKNVTVLDPHPVPSPIAAGNDINKIMEHREVKASETDPWSIAFSTCTRAALKGWKTDPVFQPYFHETGAIVSGHTPSLIKHIEEHEIDSSDAEFVKLNTAEDFRKTMPPGILTGNFPGWKGWLNKTGAGWIHAKKAMFSAYTEAKRLGVTFITGSPEGDVVSLVYENGDVAGARTADGTIHRAEHTILSAGAGSDRLLDFKKQLRPTAWTLCHIKMTPEEAKKYRNLPVLFNVAKGFFMEPDEDKHELKICDEHPGYCNFIPDPKHGGEVRSIPFAKHQIPLEAEARARDFLRDTMPHLADRPLSFARICWDADTVDRAFLIDRHPEYRSLLLAVGGSGNGAMQMSTIGGFITDALEGHLQKELKHALRWRPEIATERDWKDTQNRFGGPNKVMDFQKVGENEWTKIGDDKCRL

SEQ ID NO: 2 - protein, 446 aa, synthetic construct
MASSDLTLTSSILIVGAGTWGCSTALHLARRGYKNVTVLDPHPVPSPIAAGNDINKIMEHREVKASETDPWSIAFSTCTRAALKGWKTDPVFQPYFHETGAIVSGHTPSLIKHIEEHEIDSSDAEFVKLNTAEDFRKTMPPGILTGNFPGWKGWLNKTGAGWIHAKKAMFSAYTEAKRLGVTFITGSPEGDVVSLVYENGDVAGARTADGTIHRAEHTILSAGAGSDRLLDFKKQLRPTAWTLCHIKMTPEEAKKYRNLPVLFNVAKGFFMEPDEDKHELKICDEHPGYCNFIPDPKHGGEVRSIPFAKHQIPLEAEARARDFLRDTMPHLADRPLSFARICWDADTVDRAFLIDRHPEYRSLLLAVGGSGNGAMQMSTIGGFITDALEGHLQKELKHALRWRPEIATERDWKDTQNRFGGPNKVMDFQKVGENEWTKIGDDKCRL

SEQ ID NO: 3 - protein, 446 aa, synthetic construct
MASSELTLTSSILIVGAGTWGCSTALHLARRGYKNVTVLDPHPVPSPIAAGNDINKIMEHREVKASETDPWSIAFSTCTRAALKGWKTDPVFQPYFHETGAIVSGHTPSLIKHIEEHEIDSSDAEFVKLNTAEDFRKTMPPGILTGNFPGWKGWLNKTGAGWIHAKKAMFSAYTEAKRLGVTFITGSPEGDVVSLVYENGDVAGARTADGTIHRAEHTILSAGAGSDRLLDFKKQLRPTAWTLCHIKMTPEEAKKYRNLPVLFNVAKGFFMEPDEDKHELKICDEHPGYCNFIPDPKHGGEVRSIPFAKHQIPLEAEARARDFLRDTMPHLADRPLSFARICWDADTVDRAFLIDRHPEYRSLLLAVGGSGNGAMQMSTIGGFITDALEGHLQKELKHALRWRPEIATERDWKDTQNRFGGPNKVMDFQKVGENEWTKIGDDKCRL

SEQ ID NO: 4 - protein, 446 aa, synthetic construct
MASSKLTLTSSILIVGAGTWGCSTALHLARRGYKNVTVLDPHPVPSPIAAGNDINKIMEHREVKASETDPWSIAFSTCTRAALKGWKTDPVFQPYFHETGAIVSGHTPSLIKHIEEHEIDSSDAEFVKLNTAEDFRKTMPPGILTGNFPGWKGWLNKTGAGWIHAKKAMFSAYTEAKRLGVTFITGSPEGDVVSLVYENGDVAGARTADGTIHRAEHTILSAGAGSDRLLDFKKQLRPTAWTLCHIKMTPEEAKKYRNLPVLFNVAKGFFMEPDEDKHELKICDEHPGYCNFIPDPKHGGEVRSIPFAKHQIPLEAEARARDFLRDTMPHLADRPLSFARICWDADTVDRAFLIDRHPEYRSLLLAVGGSGNGAMQMSTIGGFITDALEGHLQKELKHALRWRPEIATERDWKDTQNRFGGPNKVMDFQKVGENEWTKIGDDKCRL

SEQ ID NO: 5 - protein, 446 aa, synthetic construct
MASSRLTLTSSILIVGAGTWGCSTALHLARRGYKNVTVLDPHPVPSPIAAGNDINKIMEHREVKASETDPWSIAFSTCTRAALKGWKTDPVFQPYFHETGAIVSGHTPSLIKHIEEHEIDSSDAEFVKLNTAEDFRKTMPPGILTGNFPGWKGWLNKTGAGWIHAKKAMFSAYTEAKRLGVTFITGSPEGDVVSLVYENGDVAGARTADGTIHRAEHTILSAGAGSDRLLDFKKQLRPTAWTLCHIKMTPEEAKKYRNLPVLFNVAKGFFMEPDEDKHELKICDEHPGYCNFIPDPKHGGEVRSIPFAKHQIPLEAEARARDFLRDTMPHLADRPLSFARICWDADTVDRAFLIDRHPEYRSLLLAVGGSGNGAMQMSTIGGFITDALEGHLQKELKHALRWRPEIATERDWKDTQNRFGGPNKVMDFQKVGENEWTKIGDDKCRL

SEQ ID NO: 6 - protein, 446 aa, synthetic construct
MASSHLTLTSSILIVGAGTWGCSTALHLARRGYKNVTVLDPHPVPSPIAAGNDINKIMEHREVKASETDPWSIAFSTCTRAALKGWKTDPVFQPYFHETGAIVSGHTPSLIKHIEEHEIDSSDAEFVKLNTAEDFRKTMPPGILTGNFPGWKGWLNKTGAGWIHAKKAMFSAYTEAKRLGVTFITGSPEGDVVSLVYENGDVAGARTADGTIHRAEHTILSAGAGSDRLLDFKKQLRPTAWTLCHIKMTPEEAKKYRNLPVLFNVAKGFFMEPDEDKHELKICDEHPGYCNFIPDPKHGGEVRSIPFAKHQIPLEAEARARDFLRDTMPHLADRPLSFARICWDADTVDRAFLIDRHPEYRSLLLAVGGSGNGAMQMSTIGGFITDALEGHLQKELKHALRWRPEIATERDWKDTQNRFGGPNKVMDFQKVGENEWTKIGDDKCRL

SEQ ID NO: 7 - protein, 446 aa, synthetic construct
MASSQLTLTSSILIVGAGTWGCSTALHLARRGYKNVTVLDPHPVPSPIAAGNDINKIMEHREVKASETDPWSIAFSTCTRAALKGWKTDPVFQPYFHETGAIVSGHTPSLIKHIEEHEIDSSDAEFVKLNTAEDFRKTMPPGILTGNFPGWKGWLNKTGAGWIHAKKAMFSAYTEAKRLGVTFITGSPEGDVVSLVYENGDVAGARTADGTIHRAEHTILSAGAGSDRLLDFKKQLRPTAWTLCHIKMTPEEAKKYRNLPVLFNVAKGFFMEPDEDKHELKICDEHPGYCNFIPDPKHGGEVRSIPFAKHQIPLEAEARARDFLRDTMPHLADRPLSFARICWDADTVDRAFLIDRHPEYRSLLLAVGGSGNGAMQMSTIGGFITDALEGHLQKELKHALRWRPEIATERDWKDTQNRFGGPNKVMDFQKVGENEWTKIGDDKCRL

SEQ ID NO: 8 - protein, 446 aa, synthetic construct
MASSSLTLTSSILIVGAGTWGCSTALHLARRGYKNVTVLDPHPVPSPIAAGNDINKIMEHREVKASETDPWSIAFSTCTRAALKGWKTDPVFQPYFHETGAIVSGHTPSLIKHIEEHEIDSSDAEFVKLNTAEDFRKTMPPGILTGNFPGWKGWLNKTGAGWIHAKKAMFSAYTEAKRLGVTFITGSPEGDVVSLVYENGDVAGARTADGTIHRAEHTILSAGAGSDRLLDFKKQLRPTAWTLCHIKMTPEEAKKYRNLPVLFNVAKGFFMEPDEDKHELKICDEHPGYCNFIPDPKHGGEVRSIPFAKHQIPLEAEARARDFLRDTMPHLADRPLSFARICWDADTVDRAFLIDRHPEYRSLLLAVGGSGNGAMQMSTIGGFITDALEGHLQKELKHALRWRPEIATERDWKDTQNRFGGPNKVMDFQKVGENEWTKIGDDKCRL

SEQ ID NO: 9 - protein, 446 aa, synthetic construct
MASSTLTLTSSILIVGAGTWGCSTALHLARRGYKNVTVLDPHPVPSPIAAGNDINKIMEHREVKASETDPWSIAFSTCTRAALKGWKTDPVFQPYFHETGAIVSGHTPSLIKHIEEHEIDSSDAEFVKLNTAEDFRKTMPPGILTGNFPGWKGWLNKTGAGWIHAKKAMFSAYTEAKRLGVTFITGSPEGDVVSLVYENGDVAGARTADGTIHRAEHTILSAGAGSDRLLDFKKQLRPTAWTLCHIKMTPEEAKKYRNLPVLFNVAKGFFMEPDEDKHELKICDEHPGYCNFIPDPKHGGEVRSIPFAKHQIPLEAEARARDFLRDTMPHLADRPLSFARICWDADTVDRAFLIDRHPEYRSLLLAVGGSGNGAMQMSTIGGFITDALEGHLQKELKHALRWRPEIATERDWKDTQNRFGGPNKVMDFQKVGENEWTKIGDDKCRL

SEQ ID NO: 10 - protein, 446 aa, synthetic construct
MASSYLTLTSSILIVGAGTWGCSTALHLARRGYKNVTVLDPHPVPSPIAAGNDINKIMEHREVKASETDPWSIAFSTCTRAALKGWKTDPVFQPYFHETGAIVSGHTPSLIKHIEEHEIDSSDAEFVKLNTAEDFRKTMPPGILTGNFPGWKGWLNKTGAGWIHAKKAMFSAYTEAKRLGVTFITGSPEGDVVSLVYENGDVAGARTADGTIHRAEHTILSAGAGSDRLLDFKKQLRPTAWTLCHIKMTPEEAKKYRNLPVLFNVAKGFFMEPDEDKHELKICDEHPGYCNFIPDPKHGGEVRSIPFAKHQIPLEAEARARDFLRDTMPHLADRPLSFARICWDADTVDRAFLIDRHPEYRSLLLAVGGSGNGAMQMSTIGGFITDALEGHLQKELKHALRWRPEIATERDWKDTQNRFGGPNKVMDFQKVGENEWTKIGDDKCRL

SEQ ID NO: 11 - protein, 446 aa, synthetic construct
MASSCLTLTSSILIVGAGTWGCSTALHLARRGYKNVTVLDPHPVPSPIAAGNDINKIMEHREVKASETDPWSIAFSTCTRAALKGWKTDPVFQPYFHETGAIVSGHTPSLIKHIEEHEIDSSDAEFVKLNTAEDFRKTMPPGILTGNFPGWKGWLNKTGAGWIHAKKAMFSAYTEAKRLGVTFITGSPEGDVVSLVYENGDVAGARTADGTIHRAEHTILSAGAGSDRLLDFKKQLRPTAWTLCHIKMTPEEAKKYRNLPVLFNVAKGFFMEPDEDKHELKICDEHPGYCNFIPDPKHGGEVRSIPFAKHQIPLEAEARARDFLRDTMPHLADRPLSFARICWDADTVDRAFLIDRHPEYRSLLLAVGGSGNGAMQMSTIGGFITDALEGHLQKELKHALRWRPEIATERDWKDTQNRFGGPNKVMDFQKVGENEWTKIGDDKCRL

SEQ ID NO: 12 - protein, 446 aa, synthetic construct
MASSGLTLTSSILIVGAGTWGCSTALHLARRGYKNVTVLDPHPVPSPIAAGNDINKIMEHREVKASETDPWSIAFSTCTRAALKGWKTDPVFQPYFHETGAIVSGHTPSLIKHIEEHEIDSSDAEFVKLNTAEDFRKTMPPGILTGNFPGWKGWLNKTGAGWIHAKKAMFSAYTEAKRLGVTFITGSPEGDVVSLVYENGDVAGARTADGTIHRAEHTILSAGAGSDRLLDFKKQLRPTAWTLCHIKMTPEEAKKYRNLPVLFNVAKGFFMEPDEDKHELKICDEHPGYCNFIPDPKHGGEVRSIPFAKHQIPLEAEARARDFLRDTMPHLADRPLSFARICWDADTVDRAFLIDRHPEYRSLLLAVGGSGNGAMQMSTIGGFITDALEGHLQKELKHALRWRPEIATERDWKDTQNRFGGPNKVMDFQKVGENEWTKIGDDKCRL

SEQ ID NO: 13 - protein, 446 aa, synthetic construct
MASSALTLTSSILIVGAGTWGCSTALHLARRGYKNVTVLDPHPVPSPIAAGNDINKIMEHREVKASETDPWSIAFSTCTRAALKGWKTDPVFQPYFHETGAIVSGHTPSLIKHIEEHEIDSSDAEFVKLNTAEDFRKTMPPGILTGNFPGWKGWLNKTGAGWIHAKKAMFSAYTEAKRLGVTFITGSPEGDVVSLVYENGDVAGARTADGTIHRAEHTILSAGAGSDRLLDFKKQLRPTAWTLCHIKMTPEEAKKYRNLPVLFNVAKGFFMEPDEDKHELKICDEHPGYCNFIPDPKHGGEVRSIPFAKHQIPLEAEARARDFLRDTMPHLADRPLSFARICWDADTVDRAFLIDRHPEYRSLLLAVGGSGNGAMQMSTIGGFITDALEGHLQKELKHALRWRPEIATERDWKDTQNRFGGPNKVMDFQKVGENEWTKIGDDKCRL

SEQ ID NO: 14 - protein, 446 aa, synthetic construct
MASSVLTLTSSILIVGAGTWGCSTALHLARRGYKNVTVLDPHPVPSPIAAGNDINKIMEHREVKASETDPWSIAFSTCTRAALKGWKTDPVFQPYFHETGAIVSGHTPSLIKHIEEHEIDSSDAEFVKLNTAEDFRKTMPPGILTGNFPGWKGWLNKTGAGWIHAKKAMFSAYTEAKRLGVTFITGSPEGDVVSLVYENGDVAGARTADGTIHRAEHTILSAGAGSDRLLDFKKQLRPTAWTLCHIKMTPEEAKKYRNLPVLFNVAKGFFMEPDEDKHELKICDEHPGYCNFIPDPKHGGEVRSIPFAKHQIPLEAEARARDFLRDTMPHLADRPLSFARICWDADTVDRAFLIDRHPEYRSLLLAVGGSGNGAMQMSTIGGFITDALEGHLQKELKHALRWRPEIATERDWKDTQNRFGGPNKVMDFQKVGENEWTKIGDDKCRL

SEQ ID NO: 15 - protein, 446 aa, synthetic construct
MASSPLTLTSSILIVGAGTWGCSTALHLARRGYKNVTVLDPHPVPSPIAAGNDINKIMEHREVKASETDPWSIAFSTCTRAALKGWKTDPVFQPYFHETGAIVSGHTPSLIKHIEEHEIDSSDAEFVKLNTAEDFRKTMPPGILTGNFPGWKGWLNKTGAGWIHAKKAMFSAYTEAKRLGVTFITGSPEGDVVSLVYENGDVAGARTADGTIHRAEHTILSAGAGSDRLLDFKKQLRPTAWTLCHIKMTPEEAKKYRNLPVLFNVAKGFFMEPDEDKHELKICDEHPGYCNFIPDPKHGGEVRSIPFAKHQIPLEAEARARDFLRDTMPHLADRPLSFARICWDADTVDRAFLIDRHPEYRSLLLAVGGSGNGAMQMSTIGGFITDALEGHLQKELKHALRWRPEIATERDWKDTQNRFGGPNKVMDFQKVGENEWTKIGDDKCRL

SEQ ID NO: 16 - protein, 446 aa, synthetic construct
MASSLLTLTSSILIVGAGTWGCSTALHLARRGYKNVTVLDPHPVPSPIAAGNDINKIMEHREVKASETDPWSIAFSTCTRAALKGWKTDPVFQPYFHETGAIVSGHTPSLIKHIEEHEIDSSDAEFVKLNTAEDFRKTMPPGILTGNFPGWKGWLNKTGAGWIHAKKAMFSAYTEAKRLGVTFITGSPEGDVVSLVYENGDVAGARTADGTIHRAEHTILSAGAGSDRLLDFKKQLRPTAWTLCHIKMTPEEAKKYRNLPVLFNVAKGFFMEPDEDKHELKICDEHPGYCNFIPDPKHGGEVRSIPFAKHQIPLEAEARARDFLRDTMPHLADRPLSFARICWDADTVDRAFLIDRHPEYRSLLLAVGGSGNGAMQMSTIGGFITDALEGHLQKELKHALRWRPEIATERDWKDTQNRFGGPNKVMDFQKVGENEWTKIGDDKCRL

SEQ ID NO: 17 - protein, 446 aa, synthetic construct
MASSILTLTSSILIVGAGTWGCSTALHLARRGYKNVTVLDPHPVPSPIAAGNDINKIMEHREVKASETDPWSIAFSTCTRAALKGWKTDPVFQPYFHETGAIVSGHTPSLIKHIEEHEIDSSDAEFVKLNTAEDFRKTMPPGILTGNFPGWKGWLNKTGAGWIHAKKAMFSAYTEAKRLGVTFITGSPEGDVVSLVYENGDVAGARTADGTIHRAEHTILSAGAGSDRLLDFKKQLRPTAWTLCHIKMTPEEAKKYRNLPVLFNVAKGFFMEPDEDKHELKICDEHPGYCNFIPDPKHGGEVRSIPFAKHQIPLEAEARARDFLRDTMPHLADRPLSFARICWDADTVDRAFLIDRHPEYRSLLLAVGGSGNGAMQMSTIGGFITDALEGHLQKELKHALRWRPEIATERDWKDTQNRFGGPNKVMDFQKVGENEWTKIGDDKCRL

SEQ ID NO: 18 - protein, 446 aa, synthetic construct
MASSFLTLTSSILIVGAGTWGCSTALHLARRGYKNVTVLDPHPVPSPIAAGNDINKIMEHREVKASETDPWSIAFSTCTRAALKGWKTDPVFQPYFHETGAIVSGHTPSLIKHIEEHEIDSSDAEFVKLNTAEDFRKTMPPGILTGNFPGWKGWLNKTGAGWIHAKKAMFSAYTEAKRLGVTFITGSPEGDVVSLVYENGDVAGARTADGTIHRAEHTILSAGAGSDRLLDFKKQLRPTAWTLCHIKMTPEEAKKYRNLPVLFNVAKGFFMEPDEDKHELKICDEHPGYCNFIPDPKHGGEVRSIPFAKHQIPLEAEARARDFLRDTMPHLADRPLSFARICWDADTVDRAFLIDRHPEYRSLLLAVGGSGNGAMQMSTIGGFITDALEGHLQKELKHALRWRPEIATERDWKDTQNRFGGPNKVMDFQKVGENEWTKIGDDKCRL

SEQ ID NO: 19 - protein, 446 aa, synthetic construct
MASSMLTLTSSILIVGAGTWGCSTALHLARRGYKNVTVLDPHPVPSPIAAGNDINKIMEHREVKASETDPWSIAFSTCTRAALKGWKTDPVFQPYFHETGAIVSGHTPSLIKHIEEHEIDSSDAEFVKLNTAEDFRKTMPPGILTGNFPGWKGWLNKTGAGWIHAKKAMFSAYTEAKRLGVTFITGSPEGDVVSLVYENGDVAGARTADGTIHRAEHTILSAGAGSDRLLDFKKQLRPTAWTLCHIKMTPEEAKKYRNLPVLFNVAKGFFMEPDEDKHELKICDEHPGYCNFIPDPKHGGEVRSIPFAKHQIPLEAEARARDFLRDTMPHLADRPLSFARICWDADTVDRAFLIDRHPEYRSLLLAVGGSGNGAMQMSTIGGFITDALEGHLQKELKHALRWRPEIATERDWKDTQNRFGGPNKVMDFQKVGENEWTKIGDDKCRL

SEQ ID NO: 20 - protein, 446 aa, synthetic construct
MASSWLTLTSSILIVGAGTWGCSTALHLARRGYKNVTVLDPHPVPSPIAAGNDINKIMEHREVKASETDPWSIAFSTCTRAALKGWKTDPVFQPYFHETGAIVSGHTPSLIKHIEEHEIDSSDAEFVKLNTAEDFRKTMPPGILTGNFPGWKGWLNKTGAGWIHAKKAMFSAYTEAKRLGVTFITGSPEGDVVSLVYENGDVAGARTADGTIHRAEHTILSAGAGSDRLLDFKKQLRPTAWTLCHIKMTPEEAKKYRNLPVLFNVAKGFFMEPDEDKHELKICDEHPGYCNFIPDPKHGGEVRSIPFAKHQIPLEAEARARDFLRDTMPHLADRPLSFARICWDADTVDRAFLIDRHPEYRSLLLAVGGSGNGAMQMSTIGGFITDALEGHLQKELKHALRWRPEIATERDWKDTQNRFGGPNKVMDFQKVGENEWTKIGDDKCRL

SEQ ID NO: 21 - protein, 446 aa, synthetic construct
MASSNLTLTSSILIVGAGTWGCSTALHLARRGYKNVTVLDPHPVPSPIAAGNDINKIDEHREVKASETDPWSIAFSTCTRAALKGWKTDPVFQPYFHETGAIVSGHTPSLIKHIEEHEIDSSDAEFVKLNTAEDFRKTMPPGILTGNFPGWKGWLNKTGAGWIHAKKAMFSAYTEAKRLGVTFITGSPEGDVVSLVYENGDVAGARTADGTIHRAEHTILSAGAGSDRLLDFKKQLRPTAWTLCHIKMTPEEAKKYRNLPVLFNVAKGFFMEPDEDKHELKICDEHPGYCNFIPDPKHGGEVRSIPFAKHQIPLEAEARARDFLRDTMPHLADRPLSFARICWDADTVDRAFLIDRHPEYRSLLLAVGGSGNGAMQMSTIGGFITDALEGHLQKELKHALRWRPEIATERDWKDTQNRFGGPNKVMDFQKVGENEWTKIGDDKCRL

SEQ ID NO: 22 - protein, 446 aa, synthetic construct
MASSNLTLTSSILIVGAGTWGCSTALHLARRGYKNVTVLDPHPVPSPIAAGNDINKIEEHREVKASETDPWSIAFSTCTRAALKGWKTDPVFQPYFHETGAIVSGHTPSLIKHIEEHEIDSSDAEFVKLNTAEDFRKTMPPGILTGNFPGWKGWLNKTGAGWIHAKKAMFSAYTEAKRLGVTFITGSPEGDVVSLVYENGDVAGARTADGTIHRAEHTILSAGAGSDRLLDFKKQLRPTAWTLCHIKMTPEEAKKYRNLPVLFNVAKGFFMEPDEDKHELKICDEHPGYCNFIPDPKHGGEVRSIPFAKHQIPLEAEARARDFLRDTMPHLADRPLSFARICWDADTVDRAFLIDRHPEYRSLLLAVGGSGNGAMQMSTIGGFITDALEGHLQKELKHALRWRPEIATERDWKDTQNRFGGPNKVMDFQKVGENEWTKIGDDKCRL

SEQ ID NO: 23 - protein, 446 aa, synthetic construct
MASSNLTLTSSILIVGAGTWGCSTALHLARRGYKNVTVLDPHPVPSPIAAGNDINKIKEHREVKASETDPWSIAFSTCTRAALKGWKTDPVFQPYFHETGAIVSGHTPSLIKHIEEHEIDSSDAEFVKLNTAEDFRKTMPPGILTGNFPGWKGWLNKTGAGWIHAKKAMFSAYTEAKRLGVTFITGSPEGDVVSLVYENGDVAGARTADGTIHRAEHTILSAGAGSDRLLDFKKQLRPTAWTLCHIKMTPEEAKKYRNLPVLFNVAKGFFMEPDEDKHELKICDEHPGYCNFIPDPKHGGEVRSIPFAKHQIPLEAEARARDFLRDTMPHLADRPLSFARICWDADTVDRAFLIDRHPEYRSLLLAVGGSGNGAMQMSTIGGFITDALEGHLQKELKHALRWRPEIATERDWKDTQNRFGGPNKVMDFQKVGENEWTKIGDDKCRL

SEQ ID NO: 24 - protein, 446 aa, synthetic construct
MASSNLTLTSSILIVGAGTWGCSTALHLARRGYKNVTVLDPHPVPSPIAAGNDINKIREHREVKASETDPWSIAFSTCTRAALKGWKTDPVFQPYFHETGAIVSGHTPSLIKHIEEHEIDSSDAEFVKLNTAEDFRKTMPPGILTGNFPGWKGWLNKTGAGWIHAKKAMFSAYTEAKRLGVTFITGSPEGDVVSLVYENGDVAGARTADGTIHRAEHTILSAGAGSDRLLDFKKQLRPTAWTLCHIKMTPEEAKKYRNLPVLFNVAKGFFMEPDEDKHELKICDEHPGYCNFIPDPKHGGEVRSIPFAKHQIPLEAEARARDFLRDTMPHLADRPLSFARICWDADTVDRAFLIDRHPEYRSLLLAVGGSGNGAMQMSTIGGFITDALEGHLQKELKHALRWRPEIATERDWKDTQNRFGGPNKVMDFQKVGENEWTKIGDDKCRL

SEQ ID NO: 25 - protein, 446 aa, synthetic construct
MASSNLTLTSSILIVGAGTWGCSTALHLARRGYKNVTVLDPHPVPSPIAAGNDINKIHEHREVKASETDPWSIAFSTCTRAALKGWKTDPVFQPYFHETGAIVSGHTPSLIKHIEEHEIDSSDAEFVKLNTAEDFRKTMPPGILTGNFPGWKGWLNKTGAGWIHAKKAMFSAYTEAKRLGVTFITGSPEGDVVSLVYENGDVAGARTADGTIHRAEHTILSAGAGSDRLLDFKKQLRPTAWTLCHIKMTPEEAKKYRNLPVLFNVAKGFFMEPDEDKHELKICDEHPGYCNFIPDPKHGGEVRSIPFAKHQIPLEAEARARDFLRDTMPHLADRPLSFARICWDADTVDRAFLIDRHPEYRSLLLAVGGSGNGAMQMSTIGGFITDALEGHLQKELKHALRWRPEIATERDWKDTQNRFGGPNKVMDFQKVGENEWTKIGDDKCRL

SEQ ID NO: 26 - protein, 446 aa, synthetic construct
MASSNLTLTSSILIVGAGTWGCSTALHLARRGYKNVTVLDPHPVPSPIAAGNDINKINEHREVKASETDPWSIAFSTCTRAALKGWKTDPVFQPYFHETGAIVSGHTPSLIKHIEEHEIDSSDAEFVKLNTAEDFRKTMPPGILTGNFPGWKGWLNKTGAGWIHAKKAMFSAYTEAKRLGVTFITGSPEGDVVSLVYENGDVAGARTADGTIHRAEHTILSAGAGSDRLLDFKKQLRPTAWTLCHIKMTPEEAKKYRNLPVLFNVAKGFFMEPDEDKHELKICDEHPGYCNFIPDPKHGGEVRSIPFAKHQIPLEAEARARDFLRDTMPHLADRPLSFARICWDADTVDRAFLIDRHPEYRSLLLAVGGSGNGAMQMSTIGGFITDALEGHLQKELKHALRWRPEIATERDWKDTQNRFGGPNKVMDFQKVGENEWTKIGDDKCRL

SEQ ID NO: 27 - protein, 446 aa, synthetic construct
MASSNLTLTSSILIVGAGTWGCSTALHLARRGYKNVTVLDPHPVPSPIAAGNDINKIQEHREVKASETDPWSIAFSTCTRAALKGWKTDPVFQPYFHETGAIVSGHTPSLIKHIEEHEIDSSDAEFVKLNTAEDFRKTMPPGILTGNFPGWKGWLNKTGAGWIHAKKAMFSAYTEAKRLGVTFITGSPEGDVVSLVYENGDVAGARTADGTIHRAEHTILSAGAGSDRLLDFKKQLRPTAWTLCHIKMTPEEAKKYRNLPVLFNVAKGFFMEPDEDKHELKICDEHPGYCNFIPDPKHGGEVRSIPFAKHQIPLEAEARARDFLRDTMPHLADRPLSFARICWDADTVDRAFLIDRHPEYRSLLLAVGGSGNGAMQMSTIGGFITDALEGHLQKELKHALRWRPEIATERDWKDTQNRFGGPNKVMDFQKVGENEWTKIGDDKCRL

SEQ ID NO: 28 - protein, 446 aa, synthetic construct
MASSNLTLTSSILIVGAGTWGCSTALHLARRGYKNVTVLDPHPVPSPIAAGNDINKISEHREVKASETDPWSIAFSTCTRAALKGWKTDPVFQPYFHETGAIVSGHTPSLIKHIEEHEIDSSDAEFVKLNTAEDFRKTMPPGILTGNFPGWKGWLNKTGAGWIHAKKAMFSAYTEAKRLGVTFITGSPEGDVVSLVYENGDVAGARTADGTIHRAEHTILSAGAGSDRLLDFKKQLRPTAWTLCHIKMTPEEAKKYRNLPVLFNVAKGFFMEPDEDKHELKICDEHPGYCNFIPDPKHGGEVRSIPFAKHQIPLEAEARARDFLRDTMPHLADRPLSFARICWDADTVDRAFLIDRHPEYRSLLLAVGGSGNGAMQMSTIGGFITDALEGHLQKELKHALRWRPEIATERDWKDTQNRFGGPNKVMDFQKVGENEWTKIGDDKCRL

SEQ ID NO: 29 - protein, 446 aa, synthetic construct
MASSNLTLTSSILIVGAGTWGCSTALHLARRGYKNVTVLDPHPVPSPIAAGNDINKITEHREVKASETDPWSIAFSTCTRAALKGWKTDPVFQPYFHETGAIVSGHTPSLIKHIEEHEIDSSDAEFVKLNTAEDFRKTMPPGILTGNFPGWKGWLNKTGAGWIHAKKAMFSAYTEAKRLGVTFITGSPEGDVVSLVYENGDVAGARTADGTIHRAEHTILSAGAGSDRLLDFKKQLRPTAWTLCHIKMTPEEAKKYRNLPVLFNVAKGFFMEPDEDKHELKICDEHPGYCNFIPDPKHGGEVRSIPFAKHQIPLEAEARARDFLRDTMPHLADRPLSFARICWDADTVDRAFLIDRHPEYRSLLLAVGGSGNGAMQMSTIGGFITDALEGHLQKELKHALRWRPEIATERDWKDTQNRFGGPNKVMDFQKVGENEWTKIGDDKCRL

SEQ ID NO: 30 - protein, 446 aa, synthetic construct
MASSNLTLTSSILIVGAGTWGCSTALHLARRGYKNVTVLDPHPVPSPIAAGNDINKIYEHREVKASETDPWSIAFSTCTRAALKGWKTDPVFQPYFHETGAIVSGHTPSLIKHIEEHEIDSSDAEFVKLNTAEDFRKTMPPGILTGNFPGWKGWLNKTGAGWIHAKKAMFSAYTEAKRLGVTFITGSPEGDVVSLVYENGDVAGARTADGTIHRAEHTILSAGAGSDRLLDFKKQLRPTAWTLCHIKMTPEEAKKYRNLPVLFNVAKGFFMEPDEDKHELKICDEHPGYCNFIPDPKHGGEVRSIPFAKHQIPLEAEARARDFLRDTMPHLADRPLSFARICWDADTVDRAFLIDRHPEYRSLLLAVGGSGNGAMQMSTIGGFITDALEGHLQKELKHALRWRPEIATERDWKDTQNRFGGPNKVMDFQKVGENEWTKIGDDKCRL

SEQ ID NO: 31 - protein, 446 aa, synthetic construct
MASSNLTLTSSILIVGAGTWGCSTALHLARRGYKNVTVLDPHPVPSPIAAGNDINKICEHREVKASETDPWSIAFSTCTRAALKGWKTDPVFQPYFHETGAIVSGHTPSLIKHIEEHEIDSSDAEFVKLNTAEDFRKTMPPGILTGNFPGWKGWLNKTGAGWIHAKKAMFSAYTEAKRLGVTFITGSPEGDVVSLVYENGDVAGARTADGTIHRAEHTILSAGAGSDRLLDFKKQLRPTAWTLCHIKMTPEEAKKYRNLPVLFNVAKGFFMEPDEDKHELKICDEHPGYCNFIPDPKHGGEVRSIPFAKHQIPLEAEARARDFLRDTMPHLADRPLSFARICWDADTVDRAFLIDRHPEYRSLLLAVGGSGNGAMQMSTIGGFITDALEGHLQKELKHALRWRPEIATERDWKDTQNRFGGPNKVMDFQKVGENEWTKIGDDKCRL

SEQ ID NO: 32 - protein, 446 aa, synthetic construct
MASSNLTLTSSILIVGAGTWGCSTALHLARRGYKNVTVLDPHPVPSPIAAGNDINKIGEHREVKASETDPWSIAFSTCTRAALKGWKTDPVFQPYFHETGAIVSGHTPSLIKHIEEHEIDSSDAEFVKLNTAEDFRKTMPPGILTGNFPGWKGWLNKTGAGWIHAKKAMFSAYTEAKRLGVTFITGSPEGDVVSLVYENGDVAGARTADGTIHRAEHTILSAGAGSDRLLDFKKQLRPTAWTLCHIKMTPEEAKKYRNLPVLFNVAKGFFMEPDEDKHELKICDEHPGYCNFIPDPKHGGEVRSIPFAKHQIPLEAEARARDFLRDTMPHLADRPLSFARICWDADTVDRAFLIDRHPEYRSLLLAVGGSGNGAMQMSTIGGFITDALEGHLQKELKHALRWRPEIATERDWKDTQNRFGGPNKVMDFQKVGENEWTKIGDDKCRL

SEQ ID NO: 33 - protein, 446 aa, synthetic construct
MASSNLTLTSSILIVGAGTWGCSTALHLARRGYKNVTVLDPHPVPSPIAAGNDINKIAEHREVKASETDPWSIAFSTCTRAALKGWKTDPVFQPYFHETGAIVSGHTPSLIKHIEEHEIDSSDAEFVKLNTAEDFRKTMPPGILTGNFPGWKGWLNKTGAGWIHAKKAMFSAYTEAKRLGVTFITGSPEGDVVSLVYENGDVAGARTADGTIHRAEHTILSAGAGSDRLLDFKKQLRPTAWTLCHIKMTPEEAKKYRNLPVLFNVAKGFFMEPDEDKHELKICDEHPGYCNFIPDPKHGGEVRSIPFAKHQIPLEAEARARDFLRDTMPHLADRPLSFARICWDADTVDRAFLIDRHPEYRSLLLAVGGSGNGAMQMSTIGGFITDALEGHLQKELKHALRWRPEIATERDWKDTQNRFGGPNKVMDFQKVGENEWTKIGDDKCRL

SEQ ID NO: 34 - protein, 446 aa, synthetic construct
MASSNLTLTSSILIVGAGTWGCSTALHLARRGYKNVTVLDPHPVPSPIAAGNDINKIVEHREVKASETDPWSIAFSTCTRAALKGWKTDPVFQPYFHETGAIVSGHTPSLIKHIEEHEIDSSDAEFVKLNTAEDFRKTMPPGILTGNFPGWKGWLNKTGAGWIHAKKAMFSAYTEAKRLGVTFITGSPEGDVVSLVYENGDVAGARTADGTIHRAEHTILSAGAGSDRLLDFKKQLRPTAWTLCHIKMTPEEAKKYRNLPVLFNVAKGFFMEPDEDKHELKICDEHPGYCNFIPDPKHGGEVRSIPFAKHQIPLEAEARARDFLRDTMPHLADRPLSFARICWDADTVDRAFLIDRHPEYRSLLLAVGGSGNGAMQMSTIGGFITDALEGHLQKELKHALRWRPEIATERDWKDTQNRFGGPNKVMDFQKVGENEWTKIGDDKCRL

SEQ ID NO: 35 - protein, 446 aa, synthetic construct
MASSNLTLTSSILIVGAGTWGCSTALHLARRGYKNVTVLDPHPVPSPIAAGNDINKIPEHREVKASETDPWSIAFSTCTRAALKGWKTDPVFQPYFHETGAIVSGHTPSLIKHIEEHEIDSSDAEFVKLNTAEDFRKTMPPGILTGNFPGWKGWLNKTGAGWIHAKKAMFSAYTEAKRLGVTFITGSPEGDVVSLVYENGDVAGARTADGTIHRAEHTILSAGAGSDRLLDFKKQLRPTAWTLCHIKMTPEEAKKYRNLPVLFNVAKGFFMEPDEDKHELKICDEHPGYCNFIPDPKHGGEVRSIPFAKHQIPLEAEARARDFLRDTMPHLADRPLSFARICWDADTVDRAFLIDRHPEYRSLLLAVGGSGNGAMQMSTIGGFITDALEGHLQKELKHALRWRPEIATERDWKDTQNRFGGPNKVMDFQKVGENEWTKIGDDKCRL

SEQ ID NO: 36 - protein, 446 aa, synthetic construct
MASSNLTLTSSILIVGAGTWGCSTALHLARRGYKNVTVLDPHPVPSPIAAGNDINKILEHREVKASETDPWSIAFSTCTRAALKGWKTDPVFQPYFHETGAIVSGHTPSLIKHIEEHEIDSSDAEFVKLNTAEDFRKTMPPGILTGNFPGWKGWLNKTGAGWIHAKKAMFSAYTEAKRLGVTFITGSPEGDVVSLVYENGDVAGARTADGTIHRAEHTILSAGAGSDRLLDFKKQLRPTAWTLCHIKMTPEEAKKYRNLPVLFNVAKGFFMEPDEDKHELKICDEHPGYCNFIPDPKHGGEVRSIPFAKHQIPLEAEARARDFLRDTMPHLADRPLSFARICWDADTVDRAFLIDRHPEYRSLLLAVGGSGNGAMQMSTIGGFITDALEGHLQKELKHALRWRPEIATERDWKDTQNRFGGPNKVMDFQKVGENEWTKIGDDKCRL

SEQ ID NO: 37 - protein, 446 aa, synthetic construct
MASSNLTLTSSILIVGAGTWGCSTALHLARRGYKNVTVLDPHPVPSPIAAGNDINKIIEHREVKASETDPWSIAFSTCTRAALKGWKTDPVFQPYFHETGAIVSGHTPSLIKHIEEHEIDSSDAEFVKLNTAEDFRKTMPPGILTGNFPGWKGWLNKTGAGWIHAKKAMFSAYTEAKRLGVTFITGSPEGDVVSLVYENGDVAGARTADGTIHRAEHTILSAGAGSDRLLDFKKQLRPTAWTLCHIKMTPEEAKKYRNLPVLFNVAKGFFMEPDEDKHELKICDEHPGYCNFIPDPKHGGEVRSIPFAKHQIPLEAEARARDFLRDTMPHLADRPLSFARICWDADTVDRAFLIDRHPEYRSLLLAVGGSGNGAMQMSTIGGFITDALEGHLQKELKHALRWRPEIATERDWKDTQNRFGGPNKVMDFQKVGENEWTKIGDDKCRL

SEQ ID NO: 38 - protein, 446 aa, synthetic construct
MASSNLTLTSSILIVGAGTWGCSTALHLARRGYKNVTVLDPHPVPSPIAAGNDINKIFEHREVKASETDPWSIAFSTCTRAALKGWKTDPVFQPYFHETGAIVSGHTPSLIKHIEEHEIDSSDAEFVKLNTAEDFRKTMPPGILTGNFPGWKGWLNKTGAGWIHAKKAMFSAYTEAKRLGVTFITGSPEGDVVSLVYENGDVAGARTADGTIHRAEHTILSAGAGSDRLLDFKKQLRPTAWTLCHIKMTPEEAKKYRNLPVLFNVAKGFFMEPDEDKHELKICDEHPGYCNFIPDPKHGGEVRSIPFAKHQIPLEAEARARDFLRDTMPHLADRPLSFARICWDADTVDRAFLIDRHPEYRSLLLAVGGSGNGAMQMSTIGGFITDALEGHLQKELKHALRWRPEIATERDWKDTQNRFGGPNKVMDFQKVGENEWTKIGDDKCRL

SEQ ID NO: 39 - protein, 446 aa, synthetic construct
MASSNLTLTSSILIVGAGTWGCSTALHLARRGYKNVTVLDPHPVPSPIAAGNDINKIWEHREVKASETDPWSIAFSTCTRAALKGWKTDPVFQPYFHETGAIVSGHTPSLIKHIEEHEIDSSDAEFVKLNTAEDFRKTMPPGILTGNFPGWKGWLNKTGAGWIHAKKAMFSAYTEAKRLGVTFITGSPEGDVVSLVYENGDVAGARTADGTIHRAEHTILSAGAGSDRLLDFKKQLRPTAWTLCHIKMTPEEAKKYRNLPVLFNVAKGFFMEPDEDKHELKICDEHPGYCNFIPDPKHGGEVRSIPFAKHQIPLEAEARARDFLRDTMPHLADRPLSFARICWDADTVDRAFLIDRHPEYRSLLLAVGGSGNGAMQMSTIGGFITDALEGHLQKELKHALRWRPEIATERDWKDTQNRFGGPNKVMDFQKVGENEWTKIGDDKCRL

SEQ ID NO: 40 - protein, 446 aa, synthetic construct
MASSNLTLTSSILIVGAGTWGCSTALHLARRGYKNVTVLDPHPVPSPIAAGNDINKIMEHREVKASETDPWSIAFSTCTRAALKGWKTDPVFQPYFHETGAIVSGHTPSLIKHIEEHEIDSSDAEFVKLNTAEDFRKTMPPGILTGNFPGWKGWLNKTGAGWIHAKKAMFSAYTEAKRLGVTFITGSPEGDVVSLVYENGDVAGARTADGTIHRAEHTILSAGADSDRLLDFKKQLRPTAWTLCHIKMTPEEAKKYRNLPVLFNVAKGFFMEPDEDKHELKICDEHPGYCNFIPDPKHGGEVRSIPFAKHQIPLEAEARARDFLRDTMPHLADRPLSFARICWDADTVDRAFLIDRHPEYRSLLLAVGGSGNGAMQMSTIGGFITDALEGHLQKELKHALRWRPEIATERDWKDTQNRFGGPNKVMDFQKVGENEWTKIGDDKCRL

SEQ ID NO: 41 - protein, 446 aa, synthetic construct
MASSNLTLTSSILIVGAGTWGCSTALHLARRGYKNVTVLDPHPVPSPIAAGNDINKIMEHREVKASETDPWSIAFSTCTRAALKGWKTDPVFQPYFHETGAIVSGHTPSLIKHIEEHEIDSSDAEFVKLNTAEDFRKTMPPGILTGNFPGWKGWLNKTGAGWIHAKKAMFSAYTEAKRLGVTFITGSPEGDVVSLVYENGDVAGARTADGTIHRAEHTILSAGAESDRLLDFKKQLRPTAWTLCHIKMTPEEAKKYRNLPVLFNVAKGFFMEPDEDKHELKICDEHPGYCNFIPDPKHGGEVRSIPFAKHQIPLEAEARARDFLRDTMPHLADRPLSFARICWDADTVDRAFLIDRHPEYRSLLLAVGGSGNGAMQMSTIGGFITDALEGHLQKELKHALRWRPEIATERDWKDTQNRFGGPNKVMDFQKVGENEWTKIGDDKCRL

SEQ ID NO: 42 - protein, 446 aa, synthetic construct
MASSNLTLTSSILIVGAGTWGCSTALHLARRGYKNVTVLDPHPVPSPIAAGNDINKIMEHREVKASETDPWSIAFSTCTRAALKGWKTDPVFQPYFHETGAIVSGHTPSLIKHIEEHEIDSSDAEFVKLNTAEDFRKTMPPGILTGNFPGWKGWLNKTGAGWIHAKKAMFSAYTEAKRLGVTFITGSPEGDVVSLVYENGDVAGARTADGTIHRAEHTILSAGAKSDRLLDFKKQLRPTAWTLCHIKMTPEEAKKYRNLPVLFNVAKGFFMEPDEDKHELKICDEHPGYCNFIPDPKHGGEVRSIPFAKHQIPLEAEARARDFLRDTMPHLADRPLSFARICWDADTVDRAFLIDRHPEYRSLLLAVGGSGNGAMQMSTIGGFITDALEGHLQKELKHALRWRPEIATERDWKDTQNRFGGPNKVMDFQKVGENEWTKIGDDKCRL

SEQ ID NO: 43 - protein, 446 aa, synthetic construct
MASSNLTLTSSILIVGAGTWGCSTALHLARRGYKNVTVLDPHPVPSPIAAGNDINKIMEHREVKASETDPWSIAFSTCTRAALKGWKTDPVFQPYFHETGAIVSGHTPSLIKHIEEHEIDSSDAEFVKLNTAEDFRKTMPPGILTGNFPGWKGWLNKTGAGWIHAKKAMFSAYTEAKRLGVTFITGSPEGDVVSLVYENGDVAGARTADGTIHRAEHTILSAGARSDRLLDFKKQLRPTAWTLCHIKMTPEEAKKYRNLPVLFNVAKGFFMEPDEDKHELKICDEHPGYCNFIPDPKHGGEVRSIPFAKHQIPLEAEARARDFLRDTMPHLADRPLSFARICWDADTVDRAFLIDRHPEYRSLLLAVGGSGNGAMQMSTIGGFITDALEGHLQKELKHALRWRPEIATERDWKDTQNRFGGPNKVMDFQKVGENEWTKIGDDKCRL

SEQ ID NO: 44 - protein, 446 aa, synthetic construct
MASSNLTLTSSILIVGAGTWGCSTALHLARRGYKNVTVLDPHPVPSPIAAGNDINKIMEHREVKASETDPWSIAFSTCTRAALKGWKTDPVFQPYFHETGAIVSGHTPSLIKHIEEHEIDSSDAEFVKLNTAEDFRKTMPPGILTGNFPGWKGWLNKTGAGWIHAKKAMFSAYTEAKRLGVTFITGSPEGDVVSLVYENGDVAGARTADGTIHRAEHTILSAGAHSDRLLDFKKQLRPTAWTLCHIKMTPEEAKKYRNLPVLFNVAKGFFMEPDEDKHELKICDEHPGYCNFIPDPKHGGEVRSIPFAKHQIPLEAEARARDFLRDTMPHLADRPLSFARICWDADTVDRAFLIDRHPEYRSLLLAVGGSGNGAMQMSTIGGFITDALEGHLQKELKHALRWRPEIATERDWKDTQNRFGGPNKVMDFQKVGENEWTKIGDDKCRL

SEQ ID NO: 45 - protein, 446 aa, synthetic construct
MASSNLTLTSSILIVGAGTWGCSTALHLARRGYKNVTVLDPHPVPSPIAAGNDINKIMEHREVKASETDPWSIAFSTCTRAALKGWKTDPVFQPYFHETGAIVSGHTPSLIKHIEEHEIDSSDAEFVKLNTAEDFRKTMPPGILTGNFPGWKGWLNKTGAGWIHAKKAMFSAYTEAKRLGVTFITGSPEGDVVSLVYENGDVAGARTADGTIHRAEHTILSAGANSDRLLDFKKQLRPTAWTLCHIKMTPEEAKKYRNLPVLFNVAKGFFMEPDEDKHELKICDEHPGYCNFIPDPKHGGEVRSIPFAKHQIPLEAEARARDFLRDTMPHLADRPLSFARICWDADTVDRAFLIDRHPEYRSLLLAVGGSGNGAMQMSTIGGFITDALEGHLQKELKHALRWRPEIATERDWKDTQNRFGGPNKVMDFQKVGENEWTKIGDDKCRL

SEQ ID NO: 46 - protein, 446 aa, synthetic construct
MASSNLTLTSSILIVGAGTWGCSTALHLARRGYKNVTVLDPHPVPSPIAAGNDINKIMEHREVKASETDPWSIAFSTCTRAALKGWKTDPVFQPYFHETGAIVSGHTPSLIKHIEEHEIDSSDAEFVKLNTAEDFRKTMPPGILTGNFPGWKGWLNKTGAGWIHAKKAMFSAYTEAKRLGVTFITGSPEGDVVSLVYENGDVAGARTADGTIHRAEHTILSAGAQSDRLLDFKKQLRPTAWTLCHIKMTPEEAKKYRNLPVLFNVAKGFFMEPDEDKHELKICDEHPGYCNFIPDPKHGGEVRSIPFAKHQIPLEAEARARDFLRDTMPHLADRPLSFARICWDADTVDRAFLIDRHPEYRSLLLAVGGSGNGAMQMSTIGGFITDALEGHLQKELKHALRWRPEIATERDWKDTQNRFGGPNKVMDFQKVGENEWTKIGDDKCRL

SEQ ID NO: 47 - protein, 446 aa, synthetic construct
MASSNLTLTSSILIVGAGTWGCSTALHLARRGYKNVTVLDPHPVPSPIAAGNDINKIMEHREVKASETDPWSIAFSTCTRAALKGWKTDPVFQPYFHETGAIVSGHTPSLIKHIEEHEIDSSDAEFVKLNTAEDFRKTMPPGILTGNFPGWKGWLNKTGAGWIHAKKAMFSAYTEAKRLGVTFITGSPEGDVVSLVYENGDVAGARTADGTIHRAEHTILSAGASSDRLLDFKKQLRPTAWTLCHIKMTPEEAKKYRNLPVLFNVAKGFFMEPDEDKHELKICDEHPGYCNFIPDPKHGGEVRSIPFAKHQIPLEAEARARDFLRDTMPHLADRPLSFARICWDADTVDRAFLIDRHPEYRSLLLAVGGSGNGAMQMSTIGGFITDALEGHLQKELKHALRWRPEIATERDWKDTQNRFGGPNKVMDFQKVGENEWTKIGDDKCRL

SEQ ID NO: 48 - protein, 446 aa, synthetic construct
MASSNLTLTSSILIVGAGTWGCSTALHLARRGYKNVTVLDPHPVPSPIAAGNDINKIMEHREVKASETDPWSIAFSTCTRAALKGWKTDPVFQPYFHETGAIVSGHTPSLIKHIEEHEIDSSDAEFVKLNTAEDFRKTMPPGILTGNFPGWKGWLNKTGAGWIHAKKAMFSAYTEAKRLGVTFITGSPEGDVVSLVYENGDVAGARTADGTIHRAEHTILSAGATSDRLLDFKKQLRPTAWTLCHIKMTPEEAKKYRNLPVLFNVAKGFFMEPDEDKHELKICDEHPGYCNFIPDPKHGGEVRSIPFAKHQIPLEAEARARDFLRDTMPHLADRPLSFARICWDADTVDRAFLIDRHPEYRSLLLAVGGSGNGAMQMSTIGGFITDALEGHLQKELKHALRWRPEIATERDWKDTQNRFGGPNKVMDFQKVGENEWTKIGDDKCRL

SEQ ID NO: 49 - protein, 446 aa, synthetic construct
MASSNLTLTSSILIVGAGTWGCSTALHLARRGYKNVTVLDPHPVPSPIAAGNDINKIMEHREVKASETDPWSIAFSTCTRAALKGWKTDPVFQPYFHETGAIVSGHTPSLIKHIEEHEIDSSDAEFVKLNTAEDFRKTMPPGILTGNFPGWKGWLNKTGAGWIHAKKAMFSAYTEAKRLGVTFITGSPEGDVVSLVYENGDVAGARTADGTIHRAEHTILSAGAYSDRLLDFKKQLRPTAWTLCHIKMTPEEAKKYRNLPVLFNVAKGFFMEPDEDKHELKICDEHPGYCNFIPDPKHGGEVRSIPFAKHQIPLEAEARARDFLRDTMPHLADRPLSFARICWDADTVDRAFLIDRHPEYRSLLLAVGGSGNGAMQMSTIGGFITDALEGHLQKELKHALRWRPEIATERDWKDTQNRFGGPNKVMDFQKVGENEWTKIGDDKCRL

SEQ ID NO: 50 - protein, 446 aa, synthetic construct
MASSNLTLTSSILIVGAGTWGCSTALHLARRGYKNVTVLDPHPVPSPIAAGNDINKIMEHREVKASETDPWSIAFSTCTRAALKGWKTDPVFQPYFHETGAIVSGHTPSLIKHIEEHEIDSSDAEFVKLNTAEDFRKTMPPGILTGNFPGWKGWLNKTGAGWIHAKKAMFSAYTEAKRLGVTFITGSPEGDVVSLVYENGDVAGARTADGTIHRAEHTILSAGACSDRLLDFKKQLRPTAWTLCHIKMTPEEAKKYRNLPVLFNVAKGFFMEPDEDKHELKICDEHPGYCNFIPDPKHGGEVRSIPFAKHQIPLEAEARARDFLRDTMPHLADRPLSFARICWDADTVDRAFLIDRHPEYRSLLLAVGGSGNGAMQMSTIGGFITDALEGHLQKELKHALRWRPEIATERDWKDTQNRFGGPNKVMDFQKVGENEWTKIGDDKCRL

SEQ ID NO: 51 - protein, 446 aa, synthetic construct
MASSNLTLTSSILIVGAGTWGCSTALHLARRGYKNVTVLDPHPVPSPIAAGNDINKIMEHREVKASETDPWSIAFSTCTRAALKGWKTDPVFQPYFHETGAIVSGHTPSLIKHIEEHEIDSSDAEFVKLNTAEDFRKTMPPGILTGNFPGWKGWLNKTGAGWIHAKKAMFSAYTEAKRLGVTFITGSPEGDVVSLVYENGDVAGARTADGTIHRAEHTILSAGAASDRLLDFKKQLRPTAWTLCHIKMTPEEAKKYRNLPVLFNVAKGFFMEPDEDKHELKICDEHPGYCNFIPDPKHGGEVRSIPFAKHQIPLEAEARARDFLRDTMPHLADRPLSFARICWDADTVDRAFLIDRHPEYRSLLLAVGGSGNGAMQMSTIGGFITDALEGHLQKELKHALRWRPEIATERDWKDTQNRFGGPNKVMDFQKVGENEWTKIGDDKCRL

SEQ ID NO: 52 - protein, 446 aa, synthetic construct
MASSNLTLTSSILIVGAGTWGCSTALHLARRGYKNVTVLDPHPVPSPIAAGNDINKIMEHREVKASETDPWSIAFSTCTRAALKGWKTDPVFQPYFHETGAIVSGHTPSLIKHIEEHEIDSSDAEFVKLNTAEDFRKTMPPGILTGNFPGWKGWLNKTGAGWIHAKKAMFSAYTEAKRLGVTFITGSPEGDVVSLVYENGDVAGARTADGTIHRAEHTILSAGAVSDRLLDFKKQLRPTAWTLCHIKMTPEEAKKYRNLPVLFNVAKGFFMEPDEDKHELKICDEHPGYCNFIPDPKHGGEVRSIPFAKHQIPLEAEARARDFLRDTMPHLADRPLSFARICWDADTVDRAFLIDRHPEYRSLLLAVGGSGNGAMQMSTIGGFITDALEGHLQKELKHALRWRPEIATERDWKDTQNRFGGPNKVMDFQKVGENEWTKIGDDKCRL

SEQ ID NO: 53 - protein, 446 aa, synthetic construct
MASSNLTLTSSILIVGAGTWGCSTALHLARRGYKNVTVLDPHPVPSPIAAGNDINKIMEHREVKASETDPWSIAFSTCTRAALKGWKTDPVFQPYFHETGAIVSGHTPSLIKHIEEHEIDSSDAEFVKLNTAEDFRKTMPPGILTGNFPGWKGWLNKTGAGWIHAKKAMFSAYTEAKRLGVTFITGSPEGDVVSLVYENGDVAGARTADGTIHRAEHTILSAGAPSDRLLDFKKQLRPTAWTLCHIKMTPEEAKKYRNLPVLFNVAKGFFMEPDEDKHELKICDEHPGYCNFIPDPKHGGEVRSIPFAKHQIPLEAEARARDFLRDTMPHLADRPLSFARICWDADTVDRAFLIDRHPEYRSLLLAVGGSGNGAMQMSTIGGFITDALEGHLQKELKHALRWRPEIATERDWKDTQNRFGGPNKVMDFQKVGENEWTKIGDDKCRL

SEQ ID NO: 54 - protein, 446 aa, synthetic construct
MASSNLTLTSSILIVGAGTWGCSTALHLARRGYKNVTVLDPHPVPSPIAAGNDINKIMEHREVKASETDPWSIAFSTCTRAALKGWKTDPVFQPYFHETGAIVSGHTPSLIKHIEEHEIDSSDAEFVKLNTAEDFRKTMPPGILTGNFPGWKGWLNKTGAGWIHAKKAMFSAYTEAKRLGVTFITGSPEGDVVSLVYENGDVAGARTADGTIHRAEHTILSAGALSDRLLDFKKQLRPTAWTLCHIKMTPEEAKKYRNLPVLFNVAKGFFMEPDEDKHELKICDEHPGYCNFIPDPKHGGEVRSIPFAKHQIPLEAEARARDFLRDTMPHLADRPLSFARICWDADTVDRAFLIDRHPEYRSLLLAVGGSGNGAMQMSTIGGFITDALEGHLQKELKHALRWRPEIATERDWKDTQNRFGGPNKVMDFQKVGENEWTKIGDDKCRL

SEQ ID NO: 55 - protein, 446 aa, synthetic construct
MASSNLTLTSSILIVGAGTWGCSTALHLARRGYKNVTVLDPHPVPSPIAAGNDINKIMEHREVKASETDPWSIAFSTCTRAALKGWKTDPVFQPYFHETGAIVSGHTPSLIKHIEEHEIDSSDAEFVKLNTAEDFRKTMPPGILTGNFPGWKGWLNKTGAGWIHAKKAMFSAYTEAKRLGVTFITGSPEGDVVSLVYENGDVAGARTADGTIHRAEHTILSAGAISDRLLDFKKQLRPTAWTLCHIKMTPEEAKKYRNLPVLFNVAKGFFMEPDEDKHELKICDEHPGYCNFIPDPKHGGEVRSIPFAKHQIPLEAEARARDFLRDTMPHLADRPLSFARICWDADTVDRAFLIDRHPEYRSLLLAVGGSGNGAMQMSTIGGFITDALEGHLQKELKHALRWRPEIATERDWKDTQNRFGGPNKVMDFQKVGENEWTKIGDDKCRL

SEQ ID NO: 56 - protein, 446 aa, synthetic construct
MASSNLTLTSSILIVGAGTWGCSTALHLARRGYKNVTVLDPHPVPSPIAAGNDINKIMEHREVKASETDPWSIAFSTCTRAALKGWKTDPVFQPYFHETGAIVSGHTPSLIKHIEEHEIDSSDAEFVKLNTAEDFRKTMPPGILTGNFPGWKGWLNKTGAGWIHAKKAMFSAYTEAKRLGVTFITGSPEGDVVSLVYENGDVAGARTADGTIHRAEHTILSAGAFSDRLLDFKKQLRPTAWTLCHIKMTPEEAKKYRNLPVLFNVAKGFFMEPDEDKHELKICDEHPGYCNFIPDPKHGGEVRSIPFAKHQIPLEAEARARDFLRDTMPHLADRPLSFARICWDADTVDRAFLIDRHPEYRSLLLAVGGSGNGAMQMSTIGGFITDALEGHLQKELKHALRWRPEIATERDWKDTQNRFGGPNKVMDFQKVGENEWTKIGDDKCRL

SEQ ID NO: 57 - protein, 446 aa, synthetic construct
MASSNLTLTSSILIVGAGTWGCSTALHLARRGYKNVTVLDPHPVPSPIAAGNDINKIMEHREVKASETDPWSIAFSTCTRAALKGWKTDPVFQPYFHETGAIVSGHTPSLIKHIEEHEIDSSDAEFVKLNTAEDFRKTMPPGILTGNFPGWKGWLNKTGAGWIHAKKAMFSAYTEAKRLGVTFITGSPEGDVVSLVYENGDVAGARTADGTIHRAEHTILSAGAMSDRLLDFKKQLRPTAWTLCHIKMTPEEAKKYRNLPVLFNVAKGFFMEPDEDKHELKICDEHPGYCNFIPDPKHGGEVRSIPFAKHQIPLEAEARARDFLRDTMPHLADRPLSFARICWDADTVDRAFLIDRHPEYRSLLLAVGGSGNGAMQMSTIGGFITDALEGHLQKELKHALRWRPEIATERDWKDTQNRFGGPNKVMDFQKVGENEWTKIGDDKCRL

SEQ ID NO: 58 - protein, 446 aa, synthetic construct
MASSNLTLTSSILIVGAGTWGCSTALHLARRGYKNVTVLDPHPVPSPIAAGNDINKIMEHREVKASETDPWSIAFSTCTRAALKGWKTDPVFQPYFHETGAIVSGHTPSLIKHIEEHEIDSSDAEFVKLNTAEDFRKTMPPGILTGNFPGWKGWLNKTGAGWIHAKKAMFSAYTEAKRLGVTFITGSPEGDVVSLVYENGDVAGARTADGTIHRAEHTILSAGAWSDRLLDFKKQLRPTAWTLCHIKMTPEEAKKYRNLPVLFNVAKGFFMEPDEDKHELKICDEHPGYCNFIPDPKHGGEVRSIPFAKHQIPLEAEARARDFLRDTMPHLADRPLSFARICWDADTVDRAFLIDRHPEYRSLLLAVGGSGNGAMQMSTIGGFITDALEGHLQKELKHALRWRPEIATERDWKDTQNRFGGPNKVMDFQKVGENEWTKIGDDKCRL

SEQ ID NO: 59 - protein, 446 aa, synthetic construct
MASSNLTLTSSILIVGAGTWGCSTALHLARRGYKNVTVLDPHPVPSPIAAGNDINKIMEHREVKASETDPWSIAFSTCTRAALKGWKTDPVFQPYFHETGAIVSGHTPSLIKHIEEHEIDSSDAEFVKLNTAEDFRKTMPPGILTGNFPGWKGWLNKTGAGWIHAKKAMFSAYTEAKRLGVTFITGSPEGDVVSLVYENGDVAGARTADGTIHRAEHTILSAGAGSDRLLDFKKQLRPTAWTLCHIKMTPEEAKKYRNLPVLFNVAKGFFMEPDEDKHELKICDEHPGYCNFIPDPKHGGEVRSIPFAKHQIPLEAEARARDFLRDTMPHLADRPLSFARICWDADTVDRAFLIDRHPEYRSLLLAVGGSGNGAMQMSTIGGFITDALEGHLQKELKHALRWRPEIATERDWKDTQNRFGGPNKVMDFQKVGENEWTKIDDDKCRL

SEQ ID NO: 60 - protein, 446 aa, synthetic construct
MASSNLTLTSSILIVGAGTWGCSTALHLARRGYKNVTVLDPHPVPSPIAAGNDINKIMEHREVKASETDPWSIAFSTCTRAALKGWKTDPVFQPYFHETGAIVSGHTPSLIKHIEEHEIDSSDAEFVKLNTAEDFRKTMPPGILTGNFPGWKGWLNKTGAGWIHAKKAMFSAYTEAKRLGVTFITGSPEGDVVSLVYENGDVAGARTADGTIHRAEHTILSAGAGSDRLLDFKKQLRPTAWTLCHIKMTPEEAKKYRNLPVLFNVAKGFFMEPDEDKHELKICDEHPGYCNFIPDPKHGGEVRSIPFAKHQIPLEAEARARDFLRDTMPHLADRPLSFARICWDADTVDRAFLIDRHPEYRSLLLAVGGSGNGAMQMSTIGGFITDALEGHLQKELKHALRWRPEIATERDWKDTQNRFGGPNKVMDFQKVGENEWTKIEDDKCRL

SEQ ID NO: 61 - protein, 446 aa, synthetic construct
MASSNLTLTSSILIVGAGTWGCSTALHLARRGYKNVTVLDPHPVPSPIAAGNDINKIMEHREVKASETDPWSIAFSTCTRAALKGWKTDPVFQPYFHETGAIVSGHTPSLIKHIEEHEIDSSDAEFVKLNTAEDFRKTMPPGILTGNFPGWKGWLNKTGAGWIHAKKAMFSAYTEAKRLGVTFITGSPEGDVVSLVYENGDVAGARTADGTIHRAEHTILSAGAGSDRLLDFKKQLRPTAWTLCHIKMTPEEAKKYRNLPVLFNVAKGFFMEPDEDKHELKICDEHPGYCNFIPDPKHGGEVRSIPFAKHQIPLEAEARARDFLRDTMPHLADRPLSFARICWDADTVDRAFLIDRHPEYRSLLLAVGGSGNGAMQMSTIGGFITDALEGHLQKELKHALRWRPEIATERDWKDTQNRFGGPNKVMDFQKVGENEWTKIKDDKCRL

SEQ ID NO: 62 - protein, 446 aa, synthetic construct
MASSNLTLTSSILIVGAGTWGCSTALHLARRGYKNVTVLDPHPVPSPIAAGNDINKIMEHREVKASETDPWSIAFSTCTRAALKGWKTDPVFQPYFHETGAIVSGHTPSLIKHIEEHEIDSSDAEFVKLNTAEDFRKTMPPGILTGNFPGWKGWLNKTGAGWIHAKKAMFSAYTEAKRLGVTFITGSPEGDVVSLVYENGDVAGARTADGTIHRAEHTILSAGAGSDRLLDFKKQLRPTAWTLCHIKMTPEEAKKYRNLPVLFNVAKGFFMEPDEDKHELKICDEHPGYCNFIPDPKHGGEVRSIPFAKHQIPLEAEARARDFLRDTMPHLADRPLSFARICWDADTVDRAFLIDRHPEYRSLLLAVGGSGNGAMQMSTIGGFITDALEGHLQKELKHALRWRPEIATERDWKDTQNRFGGPNKVMDFQKVGENEWTKIRDDKCRL

SEQ ID NO: 63 - protein, 446 aa, synthetic construct
MASSNLTLTSSILIVGAGTWGCSTALHLARRGYKNVTVLDPHPVPSPIAAGNDINKIMEHREVKASETDPWSIAFSTCTRAALKGWKTDPVFQPYFHETGAIVSGHTPSLIKHIEEHEIDSSDAEFVKLNTAEDFRKTMPPGILTGNFPGWKGWLNKTGAGWIHAKKAMFSAYTEAKRLGVTFITGSPEGDVVSLVYENGDVAGARTADGTIHRAEHTILSAGAGSDRLLDFKKQLRPTAWTLCHIKMTPEEAKKYRNLPVLFNVAKGFFMEPDEDKHELKICDEHPGYCNFIPDPKHGGEVRSIPFAKHQIPLEAEARARDFLRDTMPHLADRPLSFARICWDADTVDRAFLIDRHPEYRSLLLAVGGSGNGAMQMSTIGGFITDALEGHLQKELKHALRWRPEIATERDWKDTQNRFGGPNKVMDFQKVGENEWTKIHDDKCRL

SEQ ID NO: 64 - protein, 446 aa, synthetic construct
MASSNLTLTSSILIVGAGTWGCSTALHLARRGYKNVTVLDPHPVPSPIAAGNDINKIMEHREVKASETDPWSIAFSTCTRAALKGWKTDPVFQPYFHETGAIVSGHTPSLIKHIEEHEIDSSDAEFVKLNTAEDFRKTMPPGILTGNFPGWKGWLNKTGAGWIHAKKAMFSAYTEAKRLGVTFITGSPEGDVVSLVYENGDVAGARTADGTIHRAEHTILSAGAGSDRLLDFKKQLRPTAWTLCHIKMTPEEAKKYRNLPVLFNVAKGFFMEPDEDKHELKICDEHPGYCNFIPDPKHGGEVRSIPFAKHQIPLEAEARARDFLRDTMPHLADRPLSFARICWDADTVDRAFLIDRHPEYRSLLLAVGGSGNGAMQMSTIGGFITDALEGHLQKELKHALRWRPEIATERDWKDTQNRFGGPNKVMDFQKVGENEWTKINDDKCRL

SEQ ID NO: 65 - protein, 446 aa, synthetic construct
MASSNLTLTSSILIVGAGTWGCSTALHLARRGYKNVTVLDPHPVPSPIAAGNDINKIMEHREVKASETDPWSIAFSTCTRAALKGWKTDPVFQPYFHETGAIVSGHTPSLIKHIEEHEIDSSDAEFVKLNTAEDFRKTMPPGILTGNFPGWKGWLNKTGAGWIHAKKAMFSAYTEAKRLGVTFITGSPEGDVVSLVYENGDVAGARTADGTIHRAEHTILSAGAGSDRLLDFKKQLRPTAWTLCHIKMTPEEAKKYRNLPVLFNVAKGFFMEPDEDKHELKICDEHPGYCNFIPDPKHGGEVRSIPFAKHQIPLEAEARARDFLRDTMPHLADRPLSFARICWDADTVDRAFLIDRHPEYRSLLLAVGGSGNGAMQMSTIGGFITDALEGHLQKELKHALRWRPEIATERDWKDTQNRFGGPNKVMDFQKVGENEWTKIQDDKCRL

SEQ ID NO: 66 - protein, 446 aa, synthetic construct
MASSNLTLTSSILIVGAGTWGCSTALHLARRGYKNVTVLDPHPVPSPIAAGNDINKIMEHREVKASETDPWSIAFSTCTRAALKGWKTDPVFQPYFHETGAIVSGHTPSLIKHIEEHEIDSSDAEFVKLNTAEDFRKTMPPGILTGNFPGWKGWLNKTGAGWIHAKKAMFSAYTEAKRLGVTFITGSPEGDVVSLVYENGDVAGARTADGTIHRAEHTILSAGAGSDRLLDFKKQLRPTAWTLCHIKMTPEEAKKYRNLPVLFNVAKGFFMEPDEDKHELKICDEHPGYCNFIPDPKHGGEVRSIPFAKHQIPLEAEARARDFLRDTMPHLADRPLSFARICWDADTVDRAFLIDRHPEYRSLLLAVGGSGNGAMQMSTIGGFITDALEGHLQKELKHALRWRPEIATERDWKDTQNRFGGPNKVMDFQKVGENEWTKISDDKCRL

SEQ ID NO: 67 - protein, 446 aa, synthetic construct
MASSNLTLTSSILIVGAGTWGCSTALHLARRGYKNVTVLDPHPVPSPIAAGNDINKIMEHREVKASETDPWSIAFSTCTRAALKGWKTDPVFQPYFHETGAIVSGHTPSLIKHIEEHEIDSSDAEFVKLNTAEDFRKTMPPGILTGNFPGWKGWLNKTGAGWIHAKKAMFSAYTEAKRLGVTFITGSPEGDVVSLVYENGDVAGARTADGTIHRAEHTILSAGAGSDRLLDFKKQLRPTAWTLCHIKMTPEEAKKYRNLPVLFNVAKGFFMEPDEDKHELKICDEHPGYCNFIPDPKHGGEVRSIPFAKHQIPLEAEARARDFLRDTMPHLADRPLSFARICWDADTVDRAFLIDRHPEYRSLLLAVGGSGNGAMQMSTIGGFITDALEGHLQKELKHALRWRPEIATERDWKDTQNRFGGPNKVMDFQKVGENEWTKITDDKCRL

SEQ ID NO: 68 - protein, 446 aa, synthetic construct
MASSNLTLTSSILIVGAGTWGCSTALHLARRGYKNVTVLDPHPVPSPIAAGNDINKIMEHREVKASETDPWSIAFSTCTRAALKGWKTDPVFQPYFHETGAIVSGHTPSLIKHIEEHEIDSSDAEFVKLNTAEDFRKTMPPGILTGNFPGWKGWLNKTGAGWIHAKKAMFSAYTEAKRLGVTFITGSPEGDVVSLVYENGDVAGARTADGTIHRAEHTILSAGAGSDRLLDFKKQLRPTAWTLCHIKMTPEEAKKYRNLPVLFNVAKGFFMEPDEDKHELKICDEHPGYCNFIPDPKHGGEVRSIPFAKHQIPLEAEARARDFLRDTMPHLADRPLSFARICWDADTVDRAFLIDRHPEYRSLLLAVGGSGNGAMQMSTIGGFITDALEGHLQKELKHALRWRPEIATERDWKDTQNRFGGPNKVMDFQKVGENEWTKIYDDKCRL

SEQ ID NO: 69 - protein, 446 aa, synthetic construct
MASSNLTLTSSILIVGAGTWGCSTALHLARRGYKNVTVLDPHPVPSPIAAGNDINKIMEHREVKASETDPWSIAFSTCTRAALKGWKTDPVFQPYFHETGAIVSGHTPSLIKHIEEHEIDSSDAEFVKLNTAEDFRKTMPPGILTGNFPGWKGWLNKTGAGWIHAKKAMFSAYTEAKRLGVTFITGSPEGDVVSLVYENGDVAGARTADGTIHRAEHTILSAGAGSDRLLDFKKQLRPTAWTLCHIKMTPEEAKKYRNLPVLFNVAKGFFMEPDEDKHELKICDEHPGYCNFIPDPKHGGEVRSIPFAKHQIPLEAEARARDFLRDTMPHLADRPLSFARICWDADTVDRAFLIDRHPEYRSLLLAVGGSGNGAMQMSTIGGFITDALEGHLQKELKHALRWRPEIATERDWKDTQNRFGGPNKVMDFQKVGENEWTKICDDKCRL

SEQ ID NO: 70 - protein, 446 aa, synthetic construct
MASSNLTLTSSILIVGAGTWGCSTALHLARRGYKNVTVLDPHPVPSPIAAGNDINKIMEHREVKASETDPWSIAFSTCTRAALKGWKTDPVFQPYFHETGAIVSGHTPSLIKHIEEHEIDSSDAEFVKLNTAEDFRKTMPPGILTGNFPGWKGWLNKTGAGWIHAKKAMFSAYTEAKRLGVTFITGSPEGDVVSLVYENGDVAGARTADGTIHRAEHTILSAGAGSDRLLDFKKQLRPTAWTLCHIKMTPEEAKKYRNLPVLFNVAKGFFMEPDEDKHELKICDEHPGYCNFIPDPKHGGEVRSIPFAKHQIPLEAEARARDFLRDTMPHLADRPLSFARICWDADTVDRAFLIDRHPEYRSLLLAVGGSGNGAMQMSTIGGFITDALEGHLQKELKHALRWRPEIATERDWKDTQNRFGGPNKVMDFQKVGENEWTKIADDKCRL

SEQ ID NO: 71 - protein, 446 aa, synthetic construct
MASSNLTLTSSILIVGAGTWGCSTALHLARRGYKNVTVLDPHPVPSPIAAGNDINKIMEHREVKASETDPWSIAFSTCTRAALKGWKTDPVFQPYFHETGAIVSGHTPSLIKHIEEHEIDSSDAEFVKLNTAEDFRKTMPPGILTGNFPGWKGWLNKTGAGWIHAKKAMFSAYTEAKRLGVTFITGSPEGDVVSLVYENGDVAGARTADGTIHRAEHTILSAGAGSDRLLDFKKQLRPTAWTLCHIKMTPEEAKKYRNLPVLFNVAKGFFMEPDEDKHELKICDEHPGYCNFIPDPKHGGEVRSIPFAKHQIPLEAEARARDFLRDTMPHLADRPLSFARICWDADTVDRAFLIDRHPEYRSLLLAVGGSGNGAMQMSTIGGFITDALEGHLQKELKHALRWRPEIATERDWKDTQNRFGGPNKVMDFQKVGENEWTKIVDDKCRL

SEQ ID NO: 72 - protein, 446 aa, synthetic construct
MASSNLTLTSSILIVGAGTWGCSTALHLARRGYKNVTVLDPHPVPSPIAAGNDINKIMEHREVKASETDPWSIAFSTCTRAALKGWKTDPVFQPYFHETGAIVSGHTPSLIKHIEEHEIDSSDAEFVKLNTAEDFRKTMPPGILTGNFPGWKGWLNKTGAGWIHAKKAMFSAYTEAKRLGVTFITGSPEGDVVSLVYENGDVAGARTADGTIHRAEHTILSAGAGSDRLLDFKKQLRPTAWTLCHIKMTPEEAKKYRNLPVLFNVAKGFFMEPDEDKHELKICDEHPGYCNFIPDPKHGGEVRSIPFAKHQIPLEAEARARDFLRDTMPHLADRPLSFARICWDADTVDRAFLIDRHPEYRSLLLAVGGSGNGAMQMSTIGGFITDALEGHLQKELKHALRWRPEIATERDWKDTQNRFGGPNKVMDFQKVGENEWTKIPDDKCRL

SEQ ID NO: 73 - protein, 446 aa, synthetic construct
MASSNLTLTSSILIVGAGTWGCSTALHLARRGYKNVTVLDPHPVPSPIAAGNDINKIMEHREVKASETDPWSIAFSTCTRAALKGWKTDPVFQPYFHETGAIVSGHTPSLIKHIEEHEIDSSDAEFVKLNTAEDFRKTMPPGILTGNFPGWKGWLNKTGAGWIHAKKAMFSAYTEAKRLGVTFITGSPEGDVVSLVYENGDVAGARTADGTIHRAEHTILSAGAGSDRLLDFKKQLRPTAWTLCHIKMTPEEAKKYRNLPVLFNVAKGFFMEPDEDKHELKICDEHPGYCNFIPDPKHGGEVRSIPFAKHQIPLEAEARARDFLRDTMPHLADRPLSFARICWDADTVDRAFLIDRHPEYRSLLLAVGGSGNGAMQMSTIGGFITDALEGHLQKELKHALRWRPEIATERDWKDTQNRFGGPNKVMDFQKVGENEWTKILDDKCRL

SEQ ID NO: 74 - protein, 446 aa, synthetic construct
MASSNLTLTSSILIVGAGTWGCSTALHLARRGYKNVTVLDPHPVPSPIAAGNDINKIMEHREVKASETDPWSIAFSTCTRAALKGWKTDPVFQPYFHETGAIVSGHTPSLIKHIEEHEIDSSDAEFVKLNTAEDFRKTMPPGILTGNFPGWKGWLNKTGAGWIHAKKAMFSAYTEAKRLGVTFITGSPEGDVVSLVYENGDVAGARTADGTIHRAEHTILSAGAGSDRLLDFKKQLRPTAWTLCHIKMTPEEAKKYRNLPVLFNVAKGFFMEPDEDKHELKICDEHPGYCNFIPDPKHGGEVRSIPFAKHQIPLEAEARARDFLRDTMPHLADRPLSFARICWDADTVDRAFLIDRHPEYRSLLLAVGGSGNGAMQMSTIGGFITDALEGHLQKELKHALRWRPEIATERDWKDTQNRFGGPNKVMDFQKVGENEWTKIIDDKCRL

SEQ ID NO: 75 - protein, 446 aa, synthetic construct
MASSNLTLTSSILIVGAGTWGCSTALHLARRGYKNVTVLDPHPVPSPIAAGNDINKIMEHREVKASETDPWSIAFSTCTRAALKGWKTDPVFQPYFHETGAIVSGHTPSLIKHIEEHEIDSSDAEFVKLNTAEDFRKTMPPGILTGNFPGWKGWLNKTGAGWIHAKKAMFSAYTEAKRLGVTFITGSPEGDVVSLVYENGDVAGARTADGTIHRAEHTILSAGAGSDRLLDFKKQLRPTAWTLCHIKMTPEEAKKYRNLPVLFNVAKGFFMEPDEDKHELKICDEHPGYCNFIPDPKHGGEVRSIPFAKHQIPLEAEARARDFLRDTMPHLADRPLSFARICWDADTVDRAFLIDRHPEYRSLLLAVGGSGNGAMQMSTIGGFITDALEGHLQKELKHALRWRPEIATERDWKDTQNRFGGPNKVMDFQKVGENEWTKIFDDKCRL

SEQ ID NO: 76 - protein, 446 aa, synthetic construct
MASSNLTLTSSILIVGAGTWGCSTALHLARRGYKNVTVLDPHPVPSPIAAGNDINKIMEHREVKASETDPWSIAFSTCTRAALKGWKTDPVFQPYFHETGAIVSGHTPSLIKHIEEHEIDSSDAEFVKLNTAEDFRKTMPPGILTGNFPGWKGWLNKTGAGWIHAKKAMFSAYTEAKRLGVTFITGSPEGDVVSLVYENGDVAGARTADGTIHRAEHTILSAGAGSDRLLDFKKQLRPTAWTLCHIKMTPEEAKKYRNLPVLFNVAKGFFMEPDEDKHELKICDEHPGYCNFIPDPKHGGEVRSIPFAKHQIPLEAEARARDFLRDTMPHLADRPLSFARICWDADTVDRAFLIDRHPEYRSLLLAVGGSGNGAMQMSTIGGFITDALEGHLQKELKHALRWRPEIATERDWKDTQNRFGGPNKVMDFQKVGENEWTKIMDDKCRL

SEQ ID NO: 77 - protein, 446 aa, synthetic construct
MASSNLTLTSSILIVGAGTWGCSTALHLARRGYKNVTVLDPHPVPSPIAAGNDINKIMEHREVKASETDPWSIAFSTCTRAALKGWKTDPVFQPYFHETGAIVSGHTPSLIKHIEEHEIDSSDAEFVKLNTAEDFRKTMPPGILTGNFPGWKGWLNKTGAGWIHAKKAMFSAYTEAKRLGVTFITGSPEGDVVSLVYENGDVAGARTADGTIHRAEHTILSAGAGSDRLLDFKKQLRPTAWTLCHIKMTPEEAKKYRNLPVLFNVAKGFFMEPDEDKHELKICDEHPGYCNFIPDPKHGGEVRSIPFAKHQIPLEAEARARDFLRDTMPHLADRPLSFARICWDADTVDRAFLIDRHPEYRSLLLAVGGSGNGAMQMSTIGGFITDALEGHLQKELKHALRWRPEIATERDWKDTQNRFGGPNKVMDFQKVGENEWTKIWDDKCRL

SEQ ID NO: 78 - protein, 446 aa, synthetic construct
MASSNLTLTSSILIVGAGTWGCSTALHLARRGYKNVTVLDPHPVPSPIAAGNDINKIMDHREVKASETDPWSIAFSTCTRAALKGWKTDPVFQPYFHETGAIVSGHTPSLIKHIEEHEIDSSDAEFVKLNTAEDFRKTMPPGILTGNFPGWKGWLNKTGAGWIHAKKAMFSAYTEAKRLGVTFITGSPEGDVVSLVYENGDVAGARTADGTIHRAEHTILSAGAGSDRLLDFKKQLRPTAWTLCHIKMTPEEAKKYRNLPVLFNVAKGFFMEPDEDKHELKICDEHPGYCNFIPDPKHGGEVRSIPFAKHQIPLEAEARARDFLRDTMPHLADRPLSFARICWDADTVDRAFLIDRHPEYRSLLLAVGGSGNGAMQMSTIGGFITDALEGHLQKELKHALRWRPEIATERDWKDTQNRFGGPNKVMDFQKVGENEWTKIGDDKCRL

SEQ ID NO: 79 - protein, 446 aa, synthetic construct
MASSNLTLTSSILIVGAGTWGCSTALHLARRGYKNVTVLDPHPVPSPIAAGNDINKIMKHREVKASETDPWSIAFSTCTRAALKGWKTDPVFQPYFHETGAIVSGHTPSLIKHIEEHEIDSSDAEFVKLNTAEDFRKTMPPGILTGNFPGWKGWLNKTGAGWIHAKKAMFSAYTEAKRLGVTFITGSPEGDVVSLVYENGDVAGARTADGTIHRAEHTILSAGAGSDRLLDFKKQLRPTAWTLCHIKMTPEEAKKYRNLPVLFNVAKGFFMEPDEDKHELKICDEHPGYCNFIPDPKHGGEVRSIPFAKHQIPLEAEARARDFLRDTMPHLADRPLSFARICWDADTVDRAFLIDRHPEYRSLLLAVGGSGNGAMQMSTIGGFITDALEGHLQKELKHALRWRPEIATERDWKDTQNRFGGPNKVMDFQKVGENEWTKIGDDKCRL

SEQ ID NO: 80 - protein, 446 aa, synthetic construct
MASSNLTLTSSILIVGAGTWGCSTALHLARRGYKNVTVLDPHPVPSPIAAGNDINKIMRHREVKASETDPWSIAFSTCTRAALKGWKTDPVFQPYFHETGAIVSGHTPSLIKHIEEHEIDSSDAEFVKLNTAEDFRKTMPPGILTGNFPGWKGWLNKTGAGWIHAKKAMFSAYTEAKRLGVTFITGSPEGDVVSLVYENGDVAGARTADGTIHRAEHTILSAGAGSDRLLDFKKQLRPTAWTLCHIKMTPEEAKKYRNLPVLFNVAKGFFMEPDEDKHELKICDEHPGYCNFIPDPKHGGEVRSIPFAKHQIPLEAEARARDFLRDTMPHLADRPLSFARICWDADTVDRAFLIDRHPEYRSLLLAVGGSGNGAMQMSTIGGFITDALEGHLQKELKHALRWRPEIATERDWKDTQNRFGGPNKVMDFQKVGENEWTKIGDDKCRL

SEQ ID NO: 81 - protein, 446 aa, synthetic construct
MASSNLTLTSSILIVGAGTWGCSTALHLARRGYKNVTVLDPHPVPSPIAAGNDINKIMHHREVKASETDPWSIAFSTCTRAALKGWKTDPVFQPYFHETGAIVSGHTPSLIKHIEEHEIDSSDAEFVKLNTAEDFRKTMPPGILTGNFPGWKGWLNKTGAGWIHAKKAMFSAYTEAKRLGVTFITGSPEGDVVSLVYENGDVAGARTADGTIHRAEHTILSAGAGSDRLLDFKKQLRPTAWTLCHIKMTPEEAKKYRNLPVLFNVAKGFFMEPDEDKHELKICDEHPGYCNFIPDPKHGGEVRSIPFAKHQIPLEAEARARDFLRDTMPHLADRPLSFARICWDADTVDRAFLIDRHPEYRSLLLAVGGSGNGAMQMSTIGGFITDALEGHLQKELKHALRWRPEIATERDWKDTQNRFGGPNKVMDFQKVGENEWTKIGDDKCRL

SEQ ID NO: 82 - protein, 446 aa, synthetic construct
MASSNLTLTSSILIVGAGTWGCSTALHLARRGYKNVTVLDPHPVPSPIAAGNDINKIMNHREVKASETDPWSIAFSTCTRAALKGWKTDPVFQPYFHETGAIVSGHTPSLIKHIEEHEIDSSDAEFVKLNTAEDFRKTMPPGILTGNFPGWKGWLNKTGAGWIHAKKAMFSAYTEAKRLGVTFITGSPEGDVVSLVYENGDVAGARTADGTIHRAEHTILSAGAGSDRLLDFKKQLRPTAWTLCHIKMTPEEAKKYRNLPVLFNVAKGFFMEPDEDKHELKICDEHPGYCNFIPDPKHGGEVRSIPFAKHQIPLEAEARARDFLRDTMPHLADRPLSFARICWDADTVDRAFLIDRHPEYRSLLLAVGGSGNGAMQMSTIGGFITDALEGHLQKELKHALRWRPEIATERDWKDTQNRFGGPNKVMDFQKVGENEWTKIGDDKCRL

SEQ ID NO: 83 - protein, 446 aa, synthetic construct
MASSNLTLTSSILIVGAGTWGCSTALHLARRGYKNVTVLDPHPVPSPIAAGNDINKIMQHREVKASETDPWSIAFSTCTRAALKGWKTDPVFQPYFHETGAIVSGHTPSLIKHIEEHEIDSSDAEFVKLNTAEDFRKTMPPGILTGNFPGWKGWLNKTGAGWIHAKKAMFSAYTEAKRLGVTFITGSPEGDVVSLVYENGDVAGARTADGTIHRAEHTILSAGAGSDRLLDFKKQLRPTAWTLCHIKMTPEEAKKYRNLPVLFNVAKGFFMEPDEDKHELKICDEHPGYCNFIPDPKHGGEVRSIPFAKHQIPLEAEARARDFLRDTMPHLADRPLSFARICWDADTVDRAFLIDRHPEYRSLLLAVGGSGNGAMQMSTIGGFITDALEGHLQKELKHALRWRPEIATERDWKDTQNRFGGPNKVMDFQKVGENEWTKIGDDKCRL

SEQ ID NO: 84 - protein, 446 aa, synthetic construct
MASSNLTLTSSILIVGAGTWGCSTALHLARRGYKNVTVLDPHPVPSPIAAGNDINKIMSHREVKASETDPWSIAFSTCTRAALKGWKTDPVFQPYFHETGAIVSGHTPSLIKHIEEHEIDSSDAEFVKLNTAEDFRKTMPPGILTGNFPGWKGWLNKTGAGWIHAKKAMFSAYTEAKRLGVTFITGSPEGDVVSLVYENGDVAGARTADGTIHRAEHTILSAGAGSDRLLDFKKQLRPTAWTLCHIKMTPEEAKKYRNLPVLFNVAKGFFMEPDEDKHELKICDEHPGYCNFIPDPKHGGEVRSIPFAKHQIPLEAEARARDFLRDTMPHLADRPLSFARICWDADTVDRAFLIDRHPEYRSLLLAVGGSGNGAMQMSTIGGFITDALEGHLQKELKHALRWRPEIATERDWKDTQNRFGGPNKVMDFQKVGENEWTKIGDDKCRL

SEQ ID NO: 85 - protein, 446 aa, synthetic construct
MASSNLTLTSSILIVGAGTWGCSTALHLARRGYKNVTVLDPHPVPSPIAAGNDINKIMTHREVKASETDPWSIAFSTCTRAALKGWKTDPVFQPYFHETGAIVSGHTPSLIKHIEEHEIDSSDAEFVKLNTAEDFRKTMPPGILTGNFPGWKGWLNKTGAGWIHAKKAMFSAYTEAKRLGVTFITGSPEGDVVSLVYENGDVAGARTADGTIHRAEHTILSAGAGSDRLLDFKKQLRPTAWTLCHIKMTPEEAKKYRNLPVLFNVAKGFFMEPDEDKHELKICDEHPGYCNFIPDPKHGGEVRSIPFAKHQIPLEAEARARDFLRDTMPHLADRPLSFARICWDADTVDRAFLIDRHPEYRSLLLAVGGSGNGAMQMSTIGGFITDALEGHLQKELKHALRWRPEIATERDWKDTQNRFGGPNKVMDFQKVGENEWTKIGDDKCRL

SEQ ID NO: 86 - protein, 446 aa, synthetic construct
MASSNLTLTSSILIVGAGTWGCSTALHLARRGYKNVTVLDPHPVPSPIAAGNDINKIMYHREVKASETDPWSIAFSTCTRAALKGWKTDPVFQPYFHETGAIVSGHTPSLIKHIEEHEIDSSDAEFVKLNTAEDFRKTMPPGILTGNFPGWKGWLNKTGAGWIHAKKAMFSAYTEAKRLGVTFITGSPEGDVVSLVYENGDVAGARTADGTIHRAEHTILSAGAGSDRLLDFKKQLRPTAWTLCHIKMTPEEAKKYRNLPVLFNVAKGFFMEPDEDKHELKICDEHPGYCNFIPDPKHGGEVRSIPFAKHQIPLEAEARARDFLRDTMPHLADRPLSFARICWDADTVDRAFLIDRHPEYRSLLLAVGGSGNGAMQMSTIGGFITDALEGHLQKELKHALRWRPEIATERDWKDTQNRFGGPNKVMDFQKVGENEWTKIGDDKCRL

SEQ ID NO: 87 - protein, 446 aa, synthetic construct
MASSNLTLTSSILIVGAGTWGCSTALHLARRGYKNVTVLDPHPVPSPIAAGNDINKIMCHREVKASETDPWSIAFSTCTRAALKGWKTDPVFQPYFHETGAIVSGHTPSLIKHIEEHEIDSSDAEFVKLNTAEDFRKTMPPGILTGNFPGWKGWLNKTGAGWIHAKKAMFSAYTEAKRLGVTFITGSPEGDVVSLVYENGDVAGARTADGTIHRAEHTILSAGAGSDRLLDFKKQLRPTAWTLCHIKMTPEEAKKYRNLPVLFNVAKGFFMEPDEDKHELKICDEHPGYCNFIPDPKHGGEVRSIPFAKHQIPLEAEARARDFLRDTMPHLADRPLSFARICWDADTVDRAFLIDRHPEYRSLLLAVGGSGNGAMQMSTIGGFITDALEGHLQKELKHALRWRPEIATERDWKDTQNRFGGPNKVMDFQKVGENEWTKIGDDKCRL

SEQ ID NO: 88 - protein, 446 aa, synthetic construct
MASSNLTLTSSILIVGAGTWGCSTALHLARRGYKNVTVLDPHPVPSPIAAGNDINKIMGHREVKASETDPWSIAFSTCTRAALKGWKTDPVFQPYFHETGAIVSGHTPSLIKHIEEHEIDSSDAEFVKLNTAEDFRKTMPPGILTGNFPGWKGWLNKTGAGWIHAKKAMFSAYTEAKRLGVTFITGSPEGDVVSLVYENGDVAGARTADGTIHRAEHTILSAGAGSDRLLDFKKQLRPTAWTLCHIKMTPEEAKKYRNLPVLFNVAKGFFMEPDEDKHELKICDEHPGYCNFIPDPKHGGEVRSIPFAKHQIPLEAEARARDFLRDTMPHLADRPLSFARICWDADTVDRAFLIDRHPEYRSLLLAVGGSGNGAMQMSTIGGFITDALEGHLQKELKHALRWRPEIATERDWKDTQNRFGGPNKVMDFQKVGENEWTKIGDDKCRL

SEQ ID NO: 89 - protein, 446 aa, synthetic construct
MASSNLTLTSSILIVGAGTWGCSTALHLARRGYKNVTVLDPHPVPSPIAAGNDINKIMAHREVKASETDPWSIAFSTCTRAALKGWKTDPVFQPYFHETGAIVSGHTPSLIKHIEEHEIDSSDAEFVKLNTAEDFRKTMPPGILTGNFPGWKGWLNKTGAGWIHAKKAMFSAYTEAKRLGVTFITGSPEGDVVSLVYENGDVAGARTADGTIHRAEHTILSAGAGSDRLLDFKKQLRPTAWTLCHIKMTPEEAKKYRNLPVLFNVAKGFFMEPDEDKHELKICDEHPGYCNFIPDPKHGGEVRSIPFAKHQIPLEAEARARDFLRDTMPHLADRPLSFARICWDADTVDRAFLIDRHPEYRSLLLAVGGSGNGAMQMSTIGGFITDALEGHLQKELKHALRWRPEIATERDWKDTQNRFGGPNKVMDFQKVGENEWTKIGDDKCRL

SEQ ID NO: 90 - protein, 446 aa, synthetic construct
MASSNLTLTSSILIVGAGTWGCSTALHLARRGYKNVTVLDPHPVPSPIAAGNDINKIMVHREVKASETDPWSIAFSTCTRAALKGWKTDPVFQPYFHETGAIVSGHTPSLIKHIEEHEIDSSDAEFVKLNTAEDFRKTMPPGILTGNFPGWKGWLNKTGAGWIHAKKAMFSAYTEAKRLGVTFITGSPEGDVVSLVYENGDVAGARTADGTIHRAEHTILSAGAGSDRLLDFKKQLRPTAWTLCHIKMTPEEAKKYRNLPVLFNVAKGFFMEPDEDKHELKICDEHPGYCNFIPDPKHGGEVRSIPFAKHQIPLEAEARARDFLRDTMPHLADRPLSFARICWDADTVDRAFLIDRHPEYRSLLLAVGGSGNGAMQMSTIGGFITDALEGHLQKELKHALRWRPEIATERDWKDTQNRFGGPNKVMDFQKVGENEWTKIGDDKCRL

SEQ ID NO: 91 - protein, 446 aa, synthetic construct
MASSNLTLTSSILIVGAGTWGCSTALHLARRGYKNVTVLDPHPVPSPIAAGNDINKIMPHREVKASETDPWSIAFSTCTRAALKGWKTDPVFQPYFHETGAIVSGHTPSLIKHIEEHEIDSSDAEFVKLNTAEDFRKTMPPGILTGNFPGWKGWLNKTGAGWIHAKKAMFSAYTEAKRLGVTFITGSPEGDVVSLVYENGDVAGARTADGTIHRAEHTILSAGAGSDRLLDFKKQLRPTAWTLCHIKMTPEEAKKYRNLPVLFNVAKGFFMEPDEDKHELKICDEHPGYCNFIPDPKHGGEVRSIPFAKHQIPLEAEARARDFLRDTMPHLADRPLSFARICWDADTVDRAFLIDRHPEYRSLLLAVGGSGNGAMQMSTIGGFITDALEGHLQKELKHALRWRPEIATERDWKDTQNRFGGPNKVMDFQKVGENEWTKIGDDKCRL

SEQ ID NO: 92 - protein, 446 aa, synthetic construct
MASSNLTLTSSILIVGAGTWGCSTALHLARRGYKNVTVLDPHPVPSPIAAGNDINKIMLHREVKASETDPWSIAFSTCTRAALKGWKTDPVFQPYFHETGAIVSGHTPSLIKHIEEHEIDSSDAEFVKLNTAEDFRKTMPPGILTGNFPGWKGWLNKTGAGWIHAKKAMFSAYTEAKRLGVTFITGSPEGDVVSLVYENGDVAGARTADGTIHRAEHTILSAGAGSDRLLDFKKQLRPTAWTLCHIKMTPEEAKKYRNLPVLFNVAKGFFMEPDEDKHELKICDEHPGYCNFIPDPKHGGEVRSIPFAKHQIPLEAEARARDFLRDTMPHLADRPLSFARICWDADTVDRAFLIDRHPEYRSLLLAVGGSGNGAMQMSTIGGFITDALEGHLQKELKHALRWRPEIATERDWKDTQNRFGGPNKVMDFQKVGENEWTKIGDDKCRL

SEQ ID NO: 93 - protein, 446 aa, synthetic construct
MASSNLTLTSSILIVGAGTWGCSTALHLARRGYKNVTVLDPHPVPSPIAAGNDINKIMIHREVKASETDPWSIAFSTCTRAALKGWKTDPVFQPYFHETGAIVSGHTPSLIKHIEEHEIDSSDAEFVKLNTAEDFRKTMPPGILTGNFPGWKGWLNKTGAGWIHAKKAMFSAYTEAKRLGVTFITGSPEGDVVSLVYENGDVAGARTADGTIHRAEHTILSAGAGSDRLLDFKKQLRPTAWTLCHIKMTPEEAKKYRNLPVLFNVAKGFFMEPDEDKHELKICDEHPGYCNFIPDPKHGGEVRSIPFAKHQIPLEAEARARDFLRDTMPHLADRPLSFARICWDADTVDRAFLIDRHPEYRSLLLAVGGSGNGAMQMSTIGGFITDALEGHLQKELKHALRWRPEIATERDWKDTQNRFGGPNKVMDFQKVGENEWTKIGDDKCRL

SEQ ID NO: 94 - protein, 446 aa, synthetic construct
MASSNLTLTSSILIVGAGTWGCSTALHLARRGYKNVTVLDPHPVPSPIAAGNDINKIMFHREVKASETDPWSIAFSTCTRAALKGWKTDPVFQPYFHETGAIVSGHTPSLIKHIEEHEIDSSDAEFVKLNTAEDFRKTMPPGILTGNFPGWKGWLNKTGAGWIHAKKAMFSAYTEAKRLGVTFITGSPEGDVVSLVYENGDVAGARTADGTIHRAEHTILSAGAGSDRLLDFKKQLRPTAWTLCHIKMTPEEAKKYRNLPVLFNVAKGFFMEPDEDKHELKICDEHPGYCNFIPDPKHGGEVRSIPFAKHQIPLEAEARARDFLRDTMPHLADRPLSFARICWDADTVDRAFLIDRHPEYRSLLLAVGGSGNGAMQMSTIGGFITDALEGHLQKELKHALRWRPEIATERDWKDTQNRFGGPNKVMDFQKVGENEWTKIGDDKCRL

SEQ ID NO: 95 - protein, 446 aa, synthetic construct
MASSNLTLTSSILIVGAGTWGCSTALHLARRGYKNVTVLDPHPVPSPIAAGNDINKIMMHREVKASETDPWSIAFSTCTRAALKGWKTDPVFQPYFHETGAIVSGHTPSLIKHIEEHEIDSSDAEFVKLNTAEDFRKTMPPGILTGNFPGWKGWLNKTGAGWIHAKKAMFSAYTEAKRLGVTFITGSPEGDVVSLVYENGDVAGARTADGTIHRAEHTILSAGAGSDRLLDFKKQLRPTAWTLCHIKMTPEEAKKYRNLPVLFNVAKGFFMEPDEDKHELKICDEHPGYCNFIPDPKHGGEVRSIPFAKHQIPLEAEARARDFLRDTMPHLADRPLSFARICWDADTVDRAFLIDRHPEYRSLLLAVGGSGNGAMQMSTIGGFITDALEGHLQKELKHALRWRPEIATERDWKDTQNRFGGPNKVMDFQKVGENEWTKIGDDKCRL

SEQ ID NO: 96 - protein, 446 aa, synthetic construct
MASSNLTLTSSILIVGAGTWGCSTALHLARRGYKNVTVLDPHPVPSPIAAGNDINKIMWHREVKASETDPWSIAFSTCTRAALKGWKTDPVFQPYFHETGAIVSGHTPSLIKHIEEHEIDSSDAEFVKLNTAEDFRKTMPPGILTGNFPGWKGWLNKTGAGWIHAKKAMFSAYTEAKRLGVTFITGSPEGDVVSLVYENGDVAGARTADGTIHRAEHTILSAGAGSDRLLDFKKQLRPTAWTLCHIKMTPEEAKKYRNLPVLFNVAKGFFMEPDEDKHELKICDEHPGYCNFIPDPKHGGEVRSIPFAKHQIPLEAEARARDFLRDTMPHLADRPLSFARICWDADTVDRAFLIDRHPEYRSLLLAVGGSGNGAMQMSTIGGFITDALEGHLQKELKHALRWRPEIATERDWKDTQNRFGGPNKVMDFQKVGENEWTKIGDDKCRL

SEQ ID NO: 97 - protein, 446 aa, synthetic construct
MASSNLTLTSSILIVGAGTWGCSTALHLARRGYKNVTVLDPHPVPSPIAAGNDINKIMEHREVKASETDPWSIAFSTCTRAALKGWKTDPVFQPYFHDTGAIVSGHTPSLIKHIEEHEIDSSDAEFVKLNTAEDFRKTMPPGILTGNFPGWKGWLNKTGAGWIHAKKAMFSAYTEAKRLGVTFITGSPEGDVVSLVYENGDVAGARTADGTIHRAEHTILSAGAGSDRLLDFKKQLRPTAWTLCHIKMTPEEAKKYRNLPVLFNVAKGFFMEPDEDKHELKICDEHPGYCNFIPDPKHGGEVRSIPFAKHQIPLEAEARARDFLRDTMPHLADRPLSFARICWDADTVDRAFLIDRHPEYRSLLLAVGGSGNGAMQMSTIGGFITDALEGHLQKELKHALRWRPEIATERDWKDTQNRFGGPNKVMDFQKVGENEWTKIGDDKCRL

SEQ ID NO: 98 - protein, 446 aa, synthetic construct
MASSNLTLTSSILIVGAGTWGCSTALHLARRGYKNVTVLDPHPVPSPIAAGNDINKIMEHREVKASETDPWSIAFSTCTRAALKGWKTDPVFQPYFHKTGAIVSGHTPSLIKHIEEHEIDSSDAEFVKLNTAEDFRKTMPPGILTGNFPGWKGWLNKTGAGWIHAKKAMFSAYTEAKRLGVTFITGSPEGDVVSLVYENGDVAGARTADGTIHRAEHTILSAGAGSDRLLDFKKQLRPTAWTLCHIKMTPEEAKKYRNLPVLFNVAKGFFMEPDEDKHELKICDEHPGYCNFIPDPKHGGEVRSIPFAKHQIPLEAEARARDFLRDTMPHLADRPLSFARICWDADTVDRAFLIDRHPEYRSLLLAVGGSGNGAMQMSTIGGFITDALEGHLQKELKHALRWRPEIATERDWKDTQNRFGGPNKVMDFQKVGENEWTKIGDDKCRL

SEQ ID NO: 99 - protein, 446 aa, synthetic construct
MASSNLTLTSSILIVGAGTWGCSTALHLARRGYKNVTVLDPHPVPSPIAAGNDINKIMEHREVKASETDPWSIAFSTCTRAALKGWKTDPVFQPYFHRTGAIVSGHTPSLIKHIEEHEIDSSDAEFVKLNTAEDFRKTMPPGILTGNFPGWKGWLNKTGAGWIHAKKAMFSAYTEAKRLGVTFITGSPEGDVVSLVYENGDVAGARTADGTIHRAEHTILSAGAGSDRLLDFKKQLRPTAWTLCHIKMTPEEAKKYRNLPVLFNVAKGFFMEPDEDKHELKICDEHPGYCNFIPDPKHGGEVRSIPFAKHQIPLEAEARARDFLRDTMPHLADRPLSFARICWDADTVDRAFLIDRHPEYRSLLLAVGGSGNGAMQMSTIGGFITDALEGHLQKELKHALRWRPEIATERDWKDTQNRFGGPNKVMDFQKVGENEWTKIGDDKCRL

SEQ ID NO: 100 - protein, 446 aa, synthetic construct
MASSNLTLTSSILIVGAGTWGCSTALHLARRGYKNVTVLDPHPVPSPIAAGNDINKIMEHREVKASETDPWSIAFSTCTRAALKGWKTDPVFQPYFHHTGAIVSGHTPSLIKHIEEHEIDSSDAEFVKLNTAEDFRKTMPPGILTGNFPGWKGWLNKTGAGWIHAKKAMFSAYTEAKRLGVTFITGSPEGDVVSLVYENGDVAGARTADGTIHRAEHTILSAGAGSDRLLDFKKQLRPTAWTLCHIKMTPEEAKKYRNLPVLFNVAKGFFMEPDEDKHELKICDEHPGYCNFIPDPKHGGEVRSIPFAKHQIPLEAEARARDFLRDTMPHLADRPLSFARICWDADTVDRAFLIDRHPEYRSLLLAVGGSGNGAMQMSTIGGFITDALEGHLQKELKHALRWRPEIATERDWKDTQNRFGGPNKVMDFQKVGENEWTKIGDDKCRL

SEQ ID NO: 101 - protein, 446 aa, synthetic construct
MASSNLTLTSSILIVGAGTWGCSTALHLARRGYKNVTVLDPHPVPSPIAAGNDINKIMEHREVKASETDPWSIAFSTCTRAALKGWKTDPVFQPYFHNTGAIVSGHTPSLIKHIEEHEIDSSDAEFVKLNTAEDFRKTMPPGILTGNFPGWKGWLNKTGAGWIHAKKAMFSAYTEAKRLGVTFITGSPEGDVVSLVYENGDVAGARTADGTIHRAEHTILSAGAGSDRLLDFKKQLRPTAWTLCHIKMTPEEAKKYRNLPVLFNVAKGFFMEPDEDKHELKICDEHPGYCNFIPDPKHGGEVRSIPFAKHQIPLEAEARARDFLRDTMPHLADRPLSFARICWDADTVDRAFLIDRHPEYRSLLLAVGGSGNGAMQMSTIGGFITDALEGHLQKELKHALRWRPEIATERDWKDTQNRFGGPNKVMDFQKVGENEWTKIGDDKCRL

SEQ ID NO: 102 - protein, 446 aa, synthetic construct
MASSNLTLTSSILIVGAGTWGCSTALHLARRGYKNVTVLDPHPVPSPIAAGNDINKIMEHREVKASETDPWSIAFSTCTRAALKGWKTDPVFQPYFHQTGAIVSGHTPSLIKHIEEHEIDSSDAEFVKLNTAEDFRKTMPPGILTGNFPGWKGWLNKTGAGWIHAKKAMFSAYTEAKRLGVTFITGSPEGDVVSLVYENGDVAGARTADGTIHRAEHTILSAGAGSDRLLDFKKQLRPTAWTLCHIKMTPEEAKKYRNLPVLFNVAKGFFMEPDEDKHELKICDEHPGYCNFIPDPKHGGEVRSIPFAKHQIPLEAEARARDFLRDTMPHLADRPLSFARICWDADTVDRAFLIDRHPEYRSLLLAVGGSGNGAMQMSTIGGFITDALEGHLQKELKHALRWRPEIATERDWKDTQNRFGGPNKVMDFQKVGENEWTKIGDDKCRL

SEQ ID NO: 103 - protein, 446 aa, synthetic construct
MASSNLTLTSSILIVGAGTWGCSTALHLARRGYKNVTVLDPHPVPSPIAAGNDINKIMEHREVKASETDPWSIAFSTCTRAALKGWKTDPVFQPYFHSTGAIVSGHTPSLIKHIEEHEIDSSDAEFVKLNTAEDFRKTMPPGILTGNFPGWKGWLNKTGAGWIHAKKAMFSAYTEAKRLGVTFITGSPEGDVVSLVYENGDVAGARTADGTIHRAEHTILSAGAGSDRLLDFKKQLRPTAWTLCHIKMTPEEAKKYRNLPVLFNVAKGFFMEPDEDKHELKICDEHPGYCNFIPDPKHGGEVRSIPFAKHQIPLEAEARARDFLRDTMPHLADRPLSFARICWDADTVDRAFLIDRHPEYRSLLLAVGGSGNGAMQMSTIGGFITDALEGHLQKELKHALRWRPEIATERDWKDTQNRFGGPNKVMDFQKVGENEWTKIGDDKCRL

SEQ ID NO: 104 - protein, 446 aa, synthetic construct
MASSNLTLTSSILIVGAGTWGCSTALHLARRGYKNVTVLDPHPVPSPIAAGNDINKIMEHREVKASETDPWSIAFSTCTRAALKGWKTDPVFQPYFHTTGAIVSGHTPSLIKHIEEHEIDSSDAEFVKLNTAEDFRKTMPPGILTGNFPGWKGWLNKTGAGWIHAKKAMFSAYTEAKRLGVTFITGSPEGDVVSLVYENGDVAGARTADGTIHRAEHTILSAGAGSDRLLDFKKQLRPTAWTLCHIKMTPEEAKKYRNLPVLFNVAKGFFMEPDEDKHELKICDEHPGYCNFIPDPKHGGEVRSIPFAKHQIPLEAEARARDFLRDTMPHLADRPLSFARICWDADTVDRAFLIDRHPEYRSLLLAVGGSGNGAMQMSTIGGFITDALEGHLQKELKHALRWRPEIATERDWKDTQNRFGGPNKVMDFQKVGENEWTKIGDDKCRL

SEQ ID NO: 105 - protein, 446 aa, synthetic construct
MASSNLTLTSSILIVGAGTWGCSTALHLARRGYKNVTVLDPHPVPSPIAAGNDINKIMEHREVKASETDPWSIAFSTCTRAALKGWKTDPVFQPYFHYTGAIVSGHTPSLIKHIEEHEIDSSDAEFVKLNTAEDFRKTMPPGILTGNFPGWKGWLNKTGAGWIHAKKAMFSAYTEAKRLGVTFITGSPEGDVVSLVYENGDVAGARTADGTIHRAEHTILSAGAGSDRLLDFKKQLRPTAWTLCHIKMTPEEAKKYRNLPVLFNVAKGFFMEPDEDKHELKICDEHPGYCNFIPDPKHGGEVRSIPFAKHQIPLEAEARARDFLRDTMPHLADRPLSFARICWDADTVDRAFLIDRHPEYRSLLLAVGGSGNGAMQMSTIGGFITDALEGHLQKELKHALRWRPEIATERDWKDTQNRFGGPNKVMDFQKVGENEWTKIGDDKCRL

SEQ ID NO: 106 - protein, 446 aa, synthetic construct
MASSNLTLTSSILIVGAGTWGCSTALHLARRGYKNVTVLDPHPVPSPIAAGNDINKIMEHREVKASETDPWSIAFSTCTRAALKGWKTDPVFQPYFHCTGAIVSGHTPSLIKHIEEHEIDSSDAEFVKLNTAEDFRKTMPPGILTGNFPGWKGWLNKTGAGWIHAKKAMFSAYTEAKRLGVTFITGSPEGDVVSLVYENGDVAGARTADGTIHRAEHTILSAGAGSDRLLDFKKQLRPTAWTLCHIKMTPEEAKKYRNLPVLFNVAKGFFMEPDEDKHELKICDEHPGYCNFIPDPKHGGEVRSIPFAKHQIPLEAEARARDFLRDTMPHLADRPLSFARICWDADTVDRAFLIDRHPEYRSLLLAVGGSGNGAMQMSTIGGFITDALEGHLQKELKHALRWRPEIATERDWKDTQNRFGGPNKVMDFQKVGENEWTKIGDDKCRL

SEQ ID NO: 107 - protein, 446 aa, synthetic construct
MASSNLTLTSSILIVGAGTWGCSTALHLARRGYKNVTVLDPHPVPSPIAAGNDINKIMEHREVKASETDPWSIAFSTCTRAALKGWKTDPVFQPYFHGTGAIVSGHTPSLIKHIEEHEIDSSDAEFVKLNTAEDFRKTMPPGILTGNFPGWKGWLNKTGAGWIHAKKAMFSAYTEAKRLGVTFITGSPEGDVVSLVYENGDVAGARTADGTIHRAEHTILSAGAGSDRLLDFKKQLRPTAWTLCHIKMTPEEAKKYRNLPVLFNVAKGFFMEPDEDKHELKICDEHPGYCNFIPDPKHGGEVRSIPFAKHQIPLEAEARARDFLRDTMPHLADRPLSFARICWDADTVDRAFLIDRHPEYRSLLLAVGGSGNGAMQMSTIGGFITDALEGHLQKELKHALRWRPEIATERDWKDTQNRFGGPNKVMDFQKVGENEWTKIGDDKCRL

SEQ ID NO: 108 - protein, 446 aa, synthetic construct
MASSNLTLTSSILIVGAGTWGCSTALHLARRGYKNVTVLDPHPVPSPIAAGNDINKIMEHREVKASETDPWSIAFSTCTRAALKGWKTDPVFQPYFHATGAIVSGHTPSLIKHIEEHEIDSSDAEFVKLNTAEDFRKTMPPGILTGNFPGWKGWLNKTGAGWIHAKKAMFSAYTEAKRLGVTFITGSPEGDVVSLVYENGDVAGARTADGTIHRAEHTILSAGAGSDRLLDFKKQLRPTAWTLCHIKMTPEEAKKYRNLPVLFNVAKGFFMEPDEDKHELKICDEHPGYCNFIPDPKHGGEVRSIPFAKHQIPLEAEARARDFLRDTMPHLADRPLSFARICWDADTVDRAFLIDRHPEYRSLLLAVGGSGNGAMQMSTIGGFITDALEGHLQKELKHALRWRPEIATERDWKDTQNRFGGPNKVMDFQKVGENEWTKIGDDKCRL

SEQ ID NO: 109 - protein, 446 aa, synthetic construct
MASSNLTLTSSILIVGAGTWGCSTALHLARRGYKNVTVLDPHPVPSPIAAGNDINKIMEHREVKASETDPWSIAFSTCTRAALKGWKTDPVFQPYFHVTGAIVSGHTPSLIKHIEEHEIDSSDAEFVKLNTAEDFRKTMPPGILTGNFPGWKGWLNKTGAGWIHAKKAMFSAYTEAKRLGVTFITGSPEGDVVSLVYENGDVAGARTADGTIHRAEHTILSAGAGSDRLLDFKKQLRPTAWTLCHIKMTPEEAKKYRNLPVLFNVAKGFFMEPDEDKHELKICDEHPGYCNFIPDPKHGGEVRSIPFAKHQIPLEAEARARDFLRDTMPHLADRPLSFARICWDADTVDRAFLIDRHPEYRSLLLAVGGSGNGAMQMSTIGGFITDALEGHLQKELKHALRWRPEIATERDWKDTQNRFGGPNKVMDFQKVGENEWTKIGDDKCRL

SEQ ID NO: 110 - protein, 446 aa, synthetic construct
MASSNLTLTSSILIVGAGTWGCSTALHLARRGYKNVTVLDPHPVPSPIAAGNDINKIMEHREVKASETDPWSIAFSTCTRAALKGWKTDPVFQPYFHPTGAIVSGHTPSLIKHIEEHEIDSSDAEFVKLNTAEDFRKTMPPGILTGNFPGWKGWLNKTGAGWIHAKKAMFSAYTEAKRLGVTFITGSPEGDVVSLVYENGDVAGARTADGTIHRAEHTILSAGAGSDRLLDFKKQLRPTAWTLCHIKMTPEEAKKYRNLPVLFNVAKGFFMEPDEDKHELKICDEHPGYCNFIPDPKHGGEVRSIPFAKHQIPLEAEARARDFLRDTMPHLADRPLSFARICWDADTVDRAFLIDRHPEYRSLLLAVGGSGNGAMQMSTIGGFITDALEGHLQKELKHALRWRPEIATERDWKDTQNRFGGPNKVMDFQKVGENEWTKIGDDKCRL

SEQ ID NO: 111 - protein, 446 aa, synthetic construct
MASSNLTLTSSILIVGAGTWGCSTALHLARRGYKNVTVLDPHPVPSPIAAGNDINKIMEHREVKASETDPWSIAFSTCTRAALKGWKTDPVFQPYFHLTGAIVSGHTPSLIKHIEEHEIDSSDAEFVKLNTAEDFRKTMPPGILTGNFPGWKGWLNKTGAGWIHAKKAMFSAYTEAKRLGVTFITGSPEGDVVSLVYENGDVAGARTADGTIHRAEHTILSAGAGSDRLLDFKKQLRPTAWTLCHIKMTPEEAKKYRNLPVLFNVAKGFFMEPDEDKHELKICDEHPGYCNFIPDPKHGGEVRSIPFAKHQIPLEAEARARDFLRDTMPHLADRPLSFARICWDADTVDRAFLIDRHPEYRSLLLAVGGSGNGAMQMSTIGGFITDALEGHLQKELKHALRWRPEIATERDWKDTQNRFGGPNKVMDFQKVGENEWTKIGDDKCRL

SEQ ID NO: 112 - protein, 446 aa, synthetic construct
MASSNLTLTSSILIVGAGTWGCSTALHLARRGYKNVTVLDPHPVPSPIAAGNDINKIMEHREVKASETDPWSIAFSTCTRAALKGWKTDPVFQPYFHITGAIVSGHTPSLIKHIEEHEIDSSDAEFVKLNTAEDFRKTMPPGILTGNFPGWKGWLNKTGAGWIHAKKAMFSAYTEAKRLGVTFITGSPEGDVVSLVYENGDVAGARTADGTIHRAEHTILSAGAGSDRLLDFKKQLRPTAWTLCHIKMTPEEAKKYRNLPVLFNVAKGFFMEPDEDKHELKICDEHPGYCNFIPDPKHGGEVRSIPFAKHQIPLEAEARARDFLRDTMPHLADRPLSFARICWDADTVDRAFLIDRHPEYRSLLLAVGGSGNGAMQMSTIGGFITDALEGHLQKELKHALRWRPEIATERDWKDTQNRFGGPNKVMDFQKVGENEWTKIGDDKCRL

SEQ ID NO: 113 - protein, 446 aa, synthetic construct
MASSNLTLTSSILIVGAGTWGCSTALHLARRGYKNVTVLDPHPVPSPIAAGNDINKIMEHREVKASETDPWSIAFSTCTRAALKGWKTDPVFQPYFHFTGAIVSGHTPSLIKHIEEHEIDSSDAEFVKLNTAEDFRKTMPPGILTGNFPGWKGWLNKTGAGWIHAKKAMFSAYTEAKRLGVTFITGSPEGDVVSLVYENGDVAGARTADGTIHRAEHTILSAGAGSDRLLDFKKQLRPTAWTLCHIKMTPEEAKKYRNLPVLFNVAKGFFMEPDEDKHELKICDEHPGYCNFIPDPKHGGEVRSIPFAKHQIPLEAEARARDFLRDTMPHLADRPLSFARICWDADTVDRAFLIDRHPEYRSLLLAVGGSGNGAMQMSTIGGFITDALEGHLQKELKHALRWRPEIATERDWKDTQNRFGGPNKVMDFQKVGENEWTKIGDDKCRL

SEQ ID NO: 114 - protein, 446 aa, synthetic construct
MASSNLTLTSSILIVGAGTWGCSTALHLARRGYKNVTVLDPHPVPSPIAAGNDINKIMEHREVKASETDPWSIAFSTCTRAALKGWKTDPVFQPYFHMTGAIVSGHTPSLIKHIEEHEIDSSDAEFVKLNTAEDFRKTMPPGILTGNFPGWKGWLNKTGAGWIHAKKAMFSAYTEAKRLGVTFITGSPEGDVVSLVYENGDVAGARTADGTIHRAEHTILSAGAGSDRLLDFKKQLRPTAWTLCHIKMTPEEAKKYRNLPVLFNVAKGFFMEPDEDKHELKICDEHPGYCNFIPDPKHGGEVRSIPFAKHQIPLEAEARARDFLRDTMPHLADRPLSFARICWDADTVDRAFLIDRHPEYRSLLLAVGGSGNGAMQMSTIGGFITDALEGHLQKELKHALRWRPEIATERDWKDTQNRFGGPNKVMDFQKVGENEWTKIGDDKCRL

SEQ ID NO: 115 - protein, 446 aa, synthetic construct
MASSNLTLTSSILIVGAGTWGCSTALHLARRGYKNVTVLDPHPVPSPIAAGNDINKIMEHREVKASETDPWSIAFSTCTRAALKGWKTDPVFQPYFHWTGAIVSGHTPSLIKHIEEHEIDSSDAEFVKLNTAEDFRKTMPPGILTGNFPGWKGWLNKTGAGWIHAKKAMFSAYTEAKRLGVTFITGSPEGDVVSLVYENGDVAGARTADGTIHRAEHTILSAGAGSDRLLDFKKQLRPTAWTLCHIKMTPEEAKKYRNLPVLFNVAKGFFMEPDEDKHELKICDEHPGYCNFIPDPKHGGEVRSIPFAKHQIPLEAEARARDFLRDTMPHLADRPLSFARICWDADTVDRAFLIDRHPEYRSLLLAVGGSGNGAMQMSTIGGFITDALEGHLQKELKHALRWRPEIATERDWKDTQNRFGGPNKVMDFQKVGENEWTKIGDDKCRL

SEQ ID NO: 116 - protein, 446 aa, synthetic construct
MASSNLTLTSSILIVGAGTWGCSTALHLARRGYKNVTVLDPHPVPSPIAAGNDINKIMEHREVKASETDPWSIAFSTCTRAALKGWKTDPVFQPYFHETGAIVSGHTPSLIKHIEEHEIDSSDAEFVKLNTAEDFRKTMPPGILTGNFPGWKGWLNKTGAGWIHAKKAMFSAYTEAKRLGVTFITGSPEGDVVSLVYENGDVAGARTADGTIHRAEHTILSAGAGSDRLLDFKKQLRPTAWTLCHIKMTPEEAKKYRNLPVLFNVAKGFFMEPDEDDHELKICDEHPGYCNFIPDPKHGGEVRSIPFAKHQIPLEAEARARDFLRDTMPHLADRPLSFARICWDADTVDRAFLIDRHPEYRSLLLAVGGSGNGAMQMSTIGGFITDALEGHLQKELKHALRWRPEIATERDWKDTQNRFGGPNKVMDFQKVGENEWTKIGDDKCRL

SEQ ID NO: 117 - protein, 446 aa, synthetic construct
MASSNLTLTSSILIVGAGTWGCSTALHLARRGYKNVTVLDPHPVPSPIAAGNDINKIMEHREVKASETDPWSIAFSTCTRAALKGWKTDPVFQPYFHETGAIVSGHTPSLIKHIEEHEIDSSDAEFVKLNTAEDFRKTMPPGILTGNFPGWKGWLNKTGAGWIHAKKAMFSAYTEAKRLGVTFITGSPEGDVVSLVYENGDVAGARTADGTIHRAEHTILSAGAGSDRLLDFKKQLRPTAWTLCHIKMTPEEAKKYRNLPVLFNVAKGFFMEPDEDEHELKICDEHPGYCNFIPDPKHGGEVRSIPFAKHQIPLEAEARARDFLRDTMPHLADRPLSFARICWDADTVDRAFLIDRHPEYRSLLLAVGGSGNGAMQMSTIGGFITDALEGHLQKELKHALRWRPEIATERDWKDTQNRFGGPNKVMDFQKVGENEWTKIGDDKCRL

SEQ ID NO: 118 - protein, 446 aa, synthetic construct
MASSNLTLTSSILIVGAGTWGCSTALHLARRGYKNVTVLDPHPVPSPIAAGNDINKIMEHREVKASETDPWSIAFSTCTRAALKGWKTDPVFQPYFHETGAIVSGHTPSLIKHIEEHEIDSSDAEFVKLNTAEDFRKTMPPGILTGNFPGWKGWLNKTGAGWIHAKKAMFSAYTEAKRLGVTFITGSPEGDVVSLVYENGDVAGARTADGTIHRAEHTILSAGAGSDRLLDFKKQLRPTAWTLCHIKMTPEEAKKYRNLPVLFNVAKGFFMEPDEDRHELKICDEHPGYCNFIPDPKHGGEVRSIPFAKHQIPLEAEARARDFLRDTMPHLADRPLSFARICWDADTVDRAFLIDRHPEYRSLLLAVGGSGNGAMQMSTIGGFITDALEGHLQKELKHALRWRPEIATERDWKDTQNRFGGPNKVMDFQKVGENEWTKIGDDKCRL

SEQ ID NO: 119 - protein, 446 aa, synthetic construct
MASSNLTLTSSILIVGAGTWGCSTALHLARRGYKNVTVLDPHPVPSPIAAGNDINKIMEHREVKASETDPWSIAFSTCTRAALKGWKTDPVFQPYFHETGAIVSGHTPSLIKHIEEHEIDSSDAEFVKLNTAEDFRKTMPPGILTGNFPGWKGWLNKTGAGWIHAKKAMFSAYTEAKRLGVTFITGSPEGDVVSLVYENGDVAGARTADGTIHRAEHTILSAGAGSDRLLDFKKQLRPTAWTLCHIKMTPEEAKKYRNLPVLFNVAKGFFMEPDEDHHELKICDEHPGYCNFIPDPKHGGEVRSIPFAKHQIPLEAEARARDFLRDTMPHLADRPLSFARICWDADTVDRAFLIDRHPEYRSLLLAVGGSGNGAMQMSTIGGFITDALEGHLQKELKHALRWRPEIATERDWKDTQNRFGGPNKVMDFQKVGENEWTKIGDDKCRL

SEQ ID NO: 120 - protein, 446 aa, synthetic construct
MASSNLTLTSSILIVGAGTWGCSTALHLARRGYKNVTVLDPHPVPSPIAAGNDINKIMEHREVKASETDPWSIAFSTCTRAALKGWKTDPVFQPYFHETGAIVSGHTPSLIKHIEEHEIDSSDAEFVKLNTAEDFRKTMPPGILTGNFPGWKGWLNKTGAGWIHAKKAMFSAYTEAKRLGVTFITGSPEGDVVSLVYENGDVAGARTADGTIHRAEHTILSAGAGSDRLLDFKKQLRPTAWTLCHIKMTPEEAKKYRNLPVLFNVAKGFFMEPDEDNHELKICDEHPGYCNFIPDPKHGGEVRSIPFAKHQIPLEAEARARDFLRDTMPHLADRPLSFARICWDADTVDRAFLIDRHPEYRSLLLAVGGSGNGAMQMSTIGGFITDALEGHLQKELKHALRWRPEIATERDWKDTQNRFGGPNKVMDFQKVGENEWTKIGDDKCRL

SEQ ID NO: 121 - protein, 446 aa, synthetic construct
MASSNLTLTSSILIVGAGTWGCSTALHLARRGYKNVTVLDPHPVPSPIAAGNDINKIMEHREVKASETDPWSIAFSTCTRAALKGWKTDPVFQPYFHETGAIVSGHTPSLIKHIEEHEIDSSDAEFVKLNTAEDFRKTMPPGILTGNFPGWKGWLNKTGAGWIHAKKAMFSAYTEAKRLGVTFITGSPEGDVVSLVYENGDVAGARTADGTIHRAEHTILSAGAGSDRLLDFKKQLRPTAWTLCHIKMTPEEAKKYRNLPVLFNVAKGFFMEPDEDQHELKICDEHPGYCNFIPDPKHGGEVRSIPFAKHQIPLEAEARARDFLRDTMPHLADRPLSFARICWDADTVDRAFLIDRHPEYRSLLLAVGGSGNGAMQMSTIGGFITDALEGHLQKELKHALRWRPEIATERDWKDTQNRFGGPNKVMDFQKVGENEWTKIGDDKCRL

SEQ ID NO: 122 - protein, 446 aa, synthetic construct
MASSNLTLTSSILIVGAGTWGCSTALHLARRGYKNVTVLDPHPVPSPIAAGNDINKIMEHREVKASETDPWSIAFSTCTRAALKGWKTDPVFQPYFHETGAIVSGHTPSLIKHIEEHEIDSSDAEFVKLNTAEDFRKTMPPGILTGNFPGWKGWLNKTGAGWIHAKKAMFSAYTEAKRLGVTFITGSPEGDVVSLVYENGDVAGARTADGTIHRAEHTILSAGAGSDRLLDFKKQLRPTAWTLCHIKMTPEEAKKYRNLPVLFNVAKGFFMEPDEDSHELKICDEHPGYCNFIPDPKHGGEVRSIPFAKHQIPLEAEARARDFLRDTMPHLADRPLSFARICWDADTVDRAFLIDRHPEYRSLLLAVGGSGNGAMQMSTIGGFITDALEGHLQKELKHALRWRPEIATERDWKDTQNRFGGPNKVMDFQKVGENEWTKIGDDKCRL

SEQ ID NO: 123 - protein, 446 aa, synthetic construct
MASSNLTLTSSILIVGAGTWGCSTALHLARRGYKNVTVLDPHPVPSPIAAGNDINKIMEHREVKASETDPWSIAFSTCTRAALKGWKTDPVFQPYFHETGAIVSGHTPSLIKHIEEHEIDSSDAEFVKLNTAEDFRKTMPPGILTGNFPGWKGWLNKTGAGWIHAKKAMFSAYTEAKRLGVTFITGSPEGDVVSLVYENGDVAGARTADGTIHRAEHTILSAGAGSDRLLDFKKQLRPTAWTLCHIKMTPEEAKKYRNLPVLFNVAKGFFMEPDEDTHELKICDEHPGYCNFIPDPKHGGEVRSIPFAKHQIPLEAEARARDFLRDTMPHLADRPLSFARICWDADTVDRAFLIDRHPEYRSLLLAVGGSGNGAMQMSTIGGFITDALEGHLQKELKHALRWRPEIATERDWKDTQNRFGGPNKVMDFQKVGENEWTKIGDDKCRL

SEQ ID NO: 124 - protein, 446 aa, synthetic construct
MASSNLTLTSSILIVGAGTWGCSTALHLARRGYKNVTVLDPHPVPSPIAAGNDINKIMEHREVKASETDPWSIAFSTCTRAALKGWKTDPVFQPYFHETGAIVSGHTPSLIKHIEEHEIDSSDAEFVKLNTAEDFRKTMPPGILTGNFPGWKGWLNKTGAGWIHAKKAMFSAYTEAKRLGVTFITGSPEGDVVSLVYENGDVAGARTADGTIHRAEHTILSAGAGSDRLLDFKKQLRPTAWTLCHIKMTPEEAKKYRNLPVLFNVAKGFFMEPDEDYHELKICDEHPGYCNFIPDPKHGGEVRSIPFAKHQIPLEAEARARDFLRDTMPHLADRPLSFARICWDADTVDRAFLIDRHPEYRSLLLAVGGSGNGAMQMSTIGGFITDALEGHLQKELKHALRWRPEIATERDWKDTQNRFGGPNKVMDFQKVGENEWTKIGDDKCRL

SEQ ID NO: 125 - protein, 446 aa, synthetic construct
MASSNLTLTSSILIVGAGTWGCSTALHLARRGYKNVTVLDPHPVPSPIAAGNDINKIMEHREVKASETDPWSIAFSTCTRAALKGWKTDPVFQPYFHETGAIVSGHTPSLIKHIEEHEIDSSDAEFVKLNTAEDFRKTMPPGILTGNFPGWKGWLNKTGAGWIHAKKAMFSAYTEAKRLGVTFITGSPEGDVVSLVYENGDVAGARTADGTIHRAEHTILSAGAGSDRLLDFKKQLRPTAWTLCHIKMTPEEAKKYRNLPVLFNVAKGFFMEPDEDCHELKICDEHPGYCNFIPDPKHGGEVRSIPFAKHQIPLEAEARARDFLRDTMPHLADRPLSFARICWDADTVDRAFLIDRHPEYRSLLLAVGGSGNGAMQMSTIGGFITDALEGHLQKELKHALRWRPEIATERDWKDTQNRFGGPNKVMDFQKVGENEWTKIGDDKCRL

SEQ ID NO: 126 - protein, 446 aa, synthetic construct
MASSNLTLTSSILIVGAGTWGCSTALHLARRGYKNVTVLDPHPVPSPIAAGNDINKIMEHREVKASETDPWSIAFSTCTRAALKGWKTDPVFQPYFHETGAIVSGHTPSLIKHIEEHEIDSSDAEFVKLNTAEDFRKTMPPGILTGNFPGWKGWLNKTGAGWIHAKKAMFSAYTEAKRLGVTFITGSPEGDVVSLVYENGDVAGARTADGTIHRAEHTILSAGAGSDRLLDFKKQLRPTAWTLCHIKMTPEEAKKYRNLPVLFNVAKGFFMEPDEDGHELKICDEHPGYCNFIPDPKHGGEVRSIPFAKHQIPLEAEARARDFLRDTMPHLADRPLSFARICWDADTVDRAFLIDRHPEYRSLLLAVGGSGNGAMQMSTIGGFITDALEGHLQKELKHALRWRPEIATERDWKDTQNRFGGPNKVMDFQKVGENEWTKIGDDKCRL

SEQ ID NO: 127 - protein, 446 aa, synthetic construct
MASSNLTLTSSILIVGAGTWGCSTALHLARRGYKNVTVLDPHPVPSPIAAGNDINKIMEHREVKASETDPWSIAFSTCTRAALKGWKTDPVFQPYFHETGAIVSGHTPSLIKHIEEHEIDSSDAEFVKLNTAEDFRKTMPPGILTGNFPGWKGWLNKTGAGWIHAKKAMFSAYTEAKRLGVTFITGSPEGDVVSLVYENGDVAGARTADGTIHRAEHTILSAGAGSDRLLDFKKQLRPTAWTLCHIKMTPEEAKKYRNLPVLFNVAKGFFMEPDEDAHELKICDEHPGYCNFIPDPKHGGEVRSIPFAKHQIPLEAEARARDFLRDTMPHLADRPLSFARICWDADTVDRAFLIDRHPEYRSLLLAVGGSGNGAMQMSTIGGFITDALEGHLQKELKHALRWRPEIATERDWKDTQNRFGGPNKVMDFQKVGENEWTKIGDDKCRL

SEQ ID NO: 128 - protein, 446 aa, synthetic construct
MASSNLTLTSSILIVGAGTWGCSTALHLARRGYKNVTVLDPHPVPSPIAAGNDINKIMEHREVKASETDPWSIAFSTCTRAALKGWKTDPVFQPYFHETGAIVSGHTPSLIKHIEEHEIDSSDAEFVKLNTAEDFRKTMPPGILTGNFPGWKGWLNKTGAGWIHAKKAMFSAYTEAKRLGVTFITGSPEGDVVSLVYENGDVAGARTADGTIHRAEHTILSAGAGSDRLLDFKKQLRPTAWTLCHIKMTPEEAKKYRNLPVLFNVAKGFFMEPDEDVHELKICDEHPGYCNFIPDPKHGGEVRSIPFAKHQIPLEAEARARDFLRDTMPHLADRPLSFARICWDADTVDRAFLIDRHPEYRSLLLAVGGSGNGAMQMSTIGGFITDALEGHLQKELKHALRWRPEIATERDWKDTQNRFGGPNKVMDFQKVGENEWTKIGDDKCRL

SEQ ID NO: 129 - protein, 446 aa, synthetic construct
MASSNLTLTSSILIVGAGTWGCSTALHLARRGYKNVTVLDPHPVPSPIAAGNDINKIMEHREVKASETDPWSIAFSTCTRAALKGWKTDPVFQPYFHETGAIVSGHTPSLIKHIEEHEIDSSDAEFVKLNTAEDFRKTMPPGILTGNFPGWKGWLNKTGAGWIHAKKAMFSAYTEAKRLGVTFITGSPEGDVVSLVYENGDVAGARTADGTIHRAEHTILSAGAGSDRLLDFKKQLRPTAWTLCHIKMTPEEAKKYRNLPVLFNVAKGFFMEPDEDPHELKICDEHPGYCNFIPDPKHGGEVRSIPFAKHQIPLEAEARARDFLRDTMPHLADRPLSFARICWDADTVDRAFLIDRHPEYRSLLLAVGGSGNGAMQMSTIGGFITDALEGHLQKELKHALRWRPEIATERDWKDTQNRFGGPNKVMDFQKVGENEWTKIGDDKCRL

SEQ ID NO: 130 - protein, 446 aa, synthetic construct
MASSNLTLTSSILIVGAGTWGCSTALHLARRGYKNVTVLDPHPVPSPIAAGNDINKIMEHREVKASETDPWSIAFSTCTRAALKGWKTDPVFQPYFHETGAIVSGHTPSLIKHIEEHEIDSSDAEFVKLNTAEDFRKTMPPGILTGNFPGWKGWLNKTGAGWIHAKKAMFSAYTEAKRLGVTFITGSPEGDVVSLVYENGDVAGARTADGTIHRAEHTILSAGAGSDRLLDFKKQLRPTAWTLCHIKMTPEEAKKYRNLPVLFNVAKGFFMEPDEDLHELKICDEHPGYCNFIPDPKHGGEVRSIPFAKHQIPLEAEARARDFLRDTMPHLADRPLSFARICWDADTVDRAFLIDRHPEYRSLLLAVGGSGNGAMQMSTIGGFITDALEGHLQKELKHALRWRPEIATERDWKDTQNRFGGPNKVMDFQKVGENEWTKIGDDKCRL

SEQ ID NO: 131 - protein, 446 aa, synthetic construct
MASSNLTLTSSILIVGAGTWGCSTALHLARRGYKNVTVLDPHPVPSPIAAGNDINKIMEHREVKASETDPWSIAFSTCTRAALKGWKTDPVFQPYFHETGAIVSGHTPSLIKHIEEHEIDSSDAEFVKLNTAEDFRKTMPPGILTGNFPGWKGWLNKTGAGWIHAKKAMFSAYTEAKRLGVTFITGSPEGDVVSLVYENGDVAGARTADGTIHRAEHTILSAGAGSDRLLDFKKQLRPTAWTLCHIKMTPEEAKKYRNLPVLFNVAKGFFMEPDEDIHELKICDEHPGYCNFIPDPKHGGEVRSIPFAKHQIPLEAEARARDFLRDTMPHLADRPLSFARICWDADTVDRAFLIDRHPEYRSLLLAVGGSGNGAMQMSTIGGFITDALEGHLQKELKHALRWRPEIATERDWKDTQNRFGGPNKVMDFQKVGENEWTKIGDDKCRL

SEQ ID NO: 132 - protein, 446 aa, synthetic construct
MASSNLTLTSSILIVGAGTWGCSTALHLARRGYKNVTVLDPHPVPSPIAAGNDINKIMEHREVKASETDPWSIAFSTCTRAALKGWKTDPVFQPYFHETGAIVSGHTPSLIKHIEEHEIDSSDAEFVKLNTAEDFRKTMPPGILTGNFPGWKGWLNKTGAGWIHAKKAMFSAYTEAKRLGVTFITGSPEGDVVSLVYENGDVAGARTADGTIHRAEHTILSAGAGSDRLLDFKKQLRPTAWTLCHIKMTPEEAKKYRNLPVLFNVAKGFFMEPDEDFHELKICDEHPGYCNFIPDPKHGGEVRSIPFAKHQIPLEAEARARDFLRDTMPHLADRPLSFARICWDADTVDRAFLIDRHPEYRSLLLAVGGSGNGAMQMSTIGGFITDALEGHLQKELKHALRWRPEIATERDWKDTQNRFGGPNKVMDFQKVGENEWTKIGDDKCRL

SEQ ID NO: 133 - protein, 446 aa, synthetic construct
MASSNLTLTSSILIVGAGTWGCSTALHLARRGYKNVTVLDPHPVPSPIAAGNDINKIMEHREVKASETDPWSIAFSTCTRAALKGWKTDPVFQPYFHETGAIVSGHTPSLIKHIEEHEIDSSDAEFVKLNTAEDFRKTMPPGILTGNFPGWKGWLNKTGAGWIHAKKAMFSAYTEAKRLGVTFITGSPEGDVVSLVYENGDVAGARTADGTIHRAEHTILSAGAGSDRLLDFKKQLRPTAWTLCHIKMTPEEAKKYRNLPVLFNVAKGFFMEPDEDMHELKICDEHPGYCNFIPDPKHGGEVRSIPFAKHQIPLEAEARARDFLRDTMPHLADRPLSFARICWDADTVDRAFLIDRHPEYRSLLLAVGGSGNGAMQMSTIGGFITDALEGHLQKELKHALRWRPEIATERDWKDTQNRFGGPNKVMDFQKVGENEWTKIGDDKCRL

SEQ ID NO: 134 - protein, 446 aa, synthetic construct
MASSNLTLTSSILIVGAGTWGCSTALHLARRGYKNVTVLDPHPVPSPIAAGNDINKIMEHREVKASETDPWSIAFSTCTRAALKGWKTDPVFQPYFHETGAIVSGHTPSLIKHIEEHEIDSSDAEFVKLNTAEDFRKTMPPGILTGNFPGWKGWLNKTGAGWIHAKKAMFSAYTEAKRLGVTFITGSPEGDVVSLVYENGDVAGARTADGTIHRAEHTILSAGAGSDRLLDFKKQLRPTAWTLCHIKMTPEEAKKYRNLPVLFNVAKGFFMEPDEDWHELKICDEHPGYCNFIPDPKHGGEVRSIPFAKHQIPLEAEARARDFLRDTMPHLADRPLSFARICWDADTVDRAFLIDRHPEYRSLLLAVGGSGNGAMQMSTIGGFITDALEGHLQKELKHALRWRPEIATERDWKDTQNRFGGPNKVMDFQKVGENEWTKIGDDKCRL

SEQ ID NO: 135 - protein, 446 aa, synthetic construct
MASSNLTLTSSILIVGAGTWGCSTALHLARRGYKNVTVLDPHPVPSPIAAGNDINKIMEHREVKASETDPWSIAFSTCTRAALKGWKTDPVFQPYFHETGAIVSGHTPSLIKHIEEHEIDSSDAEFVKLNTAEDFRKTMPPGILTGNFPGWKGWLNKTGAGWIHAKKAMFSAYTEAKRLGVTFITGSPEGDVVSLVYENGDVAGARTADGTIHRAEHTILSAGAGSDRLLDFKKQLRPTAWTLCHIKMTPEEAKKYRNLPVLFNVAKGFFMEPDEDKHELKICDDHPGYCNFIPDPKHGGEVRSIPFAKHQIPLEAEARARDFLRDTMPHLADRPLSFARICWDADTVDRAFLIDRHPEYRSLLLAVGGSGNGAMQMSTIGGFITDALEGHLQKELKHALRWRPEIATERDWKDTQNRFGGPNKVMDFQKVGENEWTKIGDDKCRL

SEQ ID NO: 136 - protein, 446 aa, synthetic construct
MASSNLTLTSSILIVGAGTWGCSTALHLARRGYKNVTVLDPHPVPSPIAAGNDINKIMEHREVKASETDPWSIAFSTCTRAALKGWKTDPVFQPYFHETGAIVSGHTPSLIKHIEEHEIDSSDAEFVKLNTAEDFRKTMPPGILTGNFPGWKGWLNKTGAGWIHAKKAMFSAYTEAKRLGVTFITGSPEGDVVSLVYENGDVAGARTADGTIHRAEHTILSAGAGSDRLLDFKKQLRPTAWTLCHIKMTPEEAKKYRNLPVLFNVAKGFFMEPDEDKHELKICDKHPGYCNFIPDPKHGGEVRSIPFAKHQIPLEAEARARDFLRDTMPHLADRPLSFARICWDADTVDRAFLIDRHPEYRSLLLAVGGSGNGAMQMSTIGGFITDALEGHLQKELKHALRWRPEIATERDWKDTQNRFGGPNKVMDFQKVGENEWTKIGDDKCRL

SEQ ID NO: 137 - protein, 446 aa, synthetic construct
MASSNLTLTSSILIVGAGTWGCSTALHLARRGYKNVTVLDPHPVPSPIAAGNDINKIMEHREVKASETDPWSIAFSTCTRAALKGWKTDPVFQPYFHETGAIVSGHTPSLIKHIEEHEIDSSDAEFVKLNTAEDFRKTMPPGILTGNFPGWKGWLNKTGAGWIHAKKAMFSAYTEAKRLGVTFITGSPEGDVVSLVYENGDVAGARTADGTIHRAEHTILSAGAGSDRLLDFKKQLRPTAWTLCHIKMTPEEAKKYRNLPVLFNVAKGFFMEPDEDKHELKICDRHPGYCNFIPDPKHGGEVRSIPFAKHQIPLEAEARARDFLRDTMPHLADRPLSFARICWDADTVDRAFLIDRHPEYRSLLLAVGGSGNGAMQMSTIGGFITDALEGHLQKELKHALRWRPEIATERDWKDTQNRFGGPNKVMDFQKVGENEWTKIGDDKCRL

SEQ ID NO: 138 - protein, 446 aa, synthetic construct
MASSNLTLTSSILIVGAGTWGCSTALHLARRGYKNVTVLDPHPVPSPIAAGNDINKIMEHREVKASETDPWSIAFSTCTRAALKGWKTDPVFQPYFHETGAIVSGHTPSLIKHIEEHEIDSSDAEFVKLNTAEDFRKTMPPGILTGNFPGWKGWLNKTGAGWIHAKKAMFSAYTEAKRLGVTFITGSPEGDVVSLVYENGDVAGARTADGTIHRAEHTILSAGAGSDRLLDFKKQLRPTAWTLCHIKMTPEEAKKYRNLPVLFNVAKGFFMEPDEDKHELKICDHHPGYCNFIPDPKHGGEVRSIPFAKHQIPLEAEARARDFLRDTMPHLADRPLSFARICWDADTVDRAFLIDRHPEYRSLLLAVGGSGNGAMQMSTIGGFITDALEGHLQKELKHALRWRPEIATERDWKDTQNRFGGPNKVMDFQKVGENEWTKIGDDKCRL

SEQ ID NO: 139 - protein, 446 aa, synthetic construct
MASSNLTLTSSILIVGAGTWGCSTALHLARRGYKNVTVLDPHPVPSPIAAGNDINKIMEHREVKASETDPWSIAFSTCTRAALKGWKTDPVFQPYFHETGAIVSGHTPSLIKHIEEHEIDSSDAEFVKLNTAEDFRKTMPPGILTGNFPGWKGWLNKTGAGWIHAKKAMFSAYTEAKRLGVTFITGSPEGDVVSLVYENGDVAGARTADGTIHRAEHTILSAGAGSDRLLDFKKQLRPTAWTLCHIKMTPEEAKKYRNLPVLFNVAKGFFMEPDEDKHELKICDNHPGYCNFIPDPKHGGEVRSIPFAKHQIPLEAEARARDFLRDTMPHLADRPLSFARICWDADTVDRAFLIDRHPEYRSLLLAVGGSGNGAMQMSTIGGFITDALEGHLQKELKHALRWRPEIATERDWKDTQNRFGGPNKVMDFQKVGENEWTKIGDDKCRL

SEQ ID NO: 140 - protein, 446 aa, synthetic construct
MASSNLTLTSSILIVGAGTWGCSTALHLARRGYKNVTVLDPHPVPSPIAAGNDINKIMEHREVKASETDPWSIAFSTCTRAALKGWKTDPVFQPYFHETGAIVSGHTPSLIKHIEEHEIDSSDAEFVKLNTAEDFRKTMPPGILTGNFPGWKGWLNKTGAGWIHAKKAMFSAYTEAKRLGVTFITGSPEGDVVSLVYENGDVAGARTADGTIHRAEHTILSAGAGSDRLLDFKKQLRPTAWTLCHIKMTPEEAKKYRNLPVLFNVAKGFFMEPDEDKHELKICDQHPGYCNFIPDPKHGGEVRSIPFAKHQIPLEAEARARDFLRDTMPHLADRPLSFARICWDADTVDRAFLIDRHPEYRSLLLAVGGSGNGAMQMSTIGGFITDALEGHLQKELKHALRWRPEIATERDWKDTQNRFGGPNKVMDFQKVGENEWTKIGDDKCRL

SEQ ID NO: 141 - protein, 446 aa, synthetic construct
MASSNLTLTSSILIVGAGTWGCSTALHLARRGYKNVTVLDPHPVPSPIAAGNDINKIMEHREVKASETDPWSIAFSTCTRAALKGWKTDPVFQPYFHETGAIVSGHTPSLIKHIEEHEIDSSDAEFVKLNTAEDFRKTMPPGILTGNFPGWKGWLNKTGAGWIHAKKAMFSAYTEAKRLGVTFITGSPEGDVVSLVYENGDVAGARTADGTIHRAEHTILSAGAGSDRLLDFKKQLRPTAWTLCHIKMTPEEAKKYRNLPVLFNVAKGFFMEPDEDKHELKICDSHPGYCNFIPDPKHGGEVRSIPFAKHQIPLEAEARARDFLRDTMPHLADRPLSFARICWDADTVDRAFLIDRHPEYRSLLLAVGGSGNGAMQMSTIGGFITDALEGHLQKELKHALRWRPEIATERDWKDTQNRFGGPNKVMDFQKVGENEWTKIGDDKCRL

SEQ ID NO: 142 - protein, 446 aa, synthetic construct
MASSNLTLTSSILIVGAGTWGCSTALHLARRGYKNVTVLDPHPVPSPIAAGNDINKIMEHREVKASETDPWSIAFSTCTRAALKGWKTDPVFQPYFHETGAIVSGHTPSLIKHIEEHEIDSSDAEFVKLNTAEDFRKTMPPGILTGNFPGWKGWLNKTGAGWIHAKKAMFSAYTEAKRLGVTFITGSPEGDVVSLVYENGDVAGARTADGTIHRAEHTILSAGAGSDRLLDFKKQLRPTAWTLCHIKMTPEEAKKYRNLPVLFNVAKGFFMEPDEDKHELKICDTHPGYCNFIPDPKHGGEVRSIPFAKHQIPLEAEARARDFLRDTMPHLADRPLSFARICWDADTVDRAFLIDRHPEYRSLLLAVGGSGNGAMQMSTIGGFITDALEGHLQKELKHALRWRPEIATERDWKDTQNRFGGPNKVMDFQKVGENEWTKIGDDKCRL

SEQ ID NO: 143 - protein, 446 aa, synthetic construct
MASSNLTLTSSILIVGAGTWGCSTALHLARRGYKNVTVLDPHPVPSPIAAGNDINKIMEHREVKASETDPWSIAFSTCTRAALKGWKTDPVFQPYFHETGAIVSGHTPSLIKHIEEHEIDSSDAEFVKLNTAEDFRKTMPPGILTGNFPGWKGWLNKTGAGWIHAKKAMFSAYTEAKRLGVTFITGSPEGDVVSLVYENGDVAGARTADGTIHRAEHTILSAGAGSDRLLDFKKQLRPTAWTLCHIKMTPEEAKKYRNLPVLFNVAKGFFMEPDEDKHELKICDYHPGYCNFIPDPKHGGEVRSIPFAKHQIPLEAEARARDFLRDTMPHLADRPLSFARICWDADTVDRAFLIDRHPEYRSLLLAVGGSGNGAMQMSTIGGFITDALEGHLQKELKHALRWRPEIATERDWKDTQNRFGGPNKVMDFQKVGENEWTKIGDDKCRL

SEQ ID NO: 144 - protein, 446 aa, synthetic construct
MASSNLTLTSSILIVGAGTWGCSTALHLARRGYKNVTVLDPHPVPSPIAAGNDINKIMEHREVKASETDPWSIAFSTCTRAALKGWKTDPVFQPYFHETGAIVSGHTPSLIKHIEEHEIDSSDAEFVKLNTAEDFRKTMPPGILTGNFPGWKGWLNKTGAGWIHAKKAMFSAYTEAKRLGVTFITGSPEGDVVSLVYENGDVAGARTADGTIHRAEHTILSAGAGSDRLLDFKKQLRPTAWTLCHIKMTPEEAKKYRNLPVLFNVAKGFFMEPDEDKHELKICDCHPGYCNFIPDPKHGGEVRSIPFAKHQIPLEAEARARDFLRDTMPHLADRPLSFARICWDADTVDRAFLIDRHPEYRSLLLAVGGSGNGAMQMSTIGGFITDALEGHLQKELKHALRWRPEIATERDWKDTQNRFGGPNKVMDFQKVGENEWTKIGDDKCRL

SEQ ID NO: 145 - protein, 446 aa, synthetic construct
MASSNLTLTSSILIVGAGTWGCSTALHLARRGYKNVTVLDPHPVPSPIAAGNDINKIMEHREVKASETDPWSIAFSTCTRAALKGWKTDPVFQPYFHETGAIVSGHTPSLIKHIEEHEIDSSDAEFVKLNTAEDFRKTMPPGILTGNFPGWKGWLNKTGAGWIHAKKAMFSAYTEAKRLGVTFITGSPEGDVVSLVYENGDVAGARTADGTIHRAEHTILSAGAGSDRLLDFKKQLRPTAWTLCHIKMTPEEAKKYRNLPVLFNVAKGFFMEPDEDKHELKICDGHPGYCNFIPDPKHGGEVRSIPFAKHQIPLEAEARARDFLRDTMPHLADRPLSFARICWDADTVDRAFLIDRHPEYRSLLLAVGGSGNGAMQMSTIGGFITDALEGHLQKELKHALRWRPEIATERDWKDTQNRFGGPNKVMDFQKVGENEWTKIGDDKCRL

SEQ ID NO: 146 - protein, 446 aa, synthetic construct
MASSNLTLTSSILIVGAGTWGCSTALHLARRGYKNVTVLDPHPVPSPIAAGNDINKIMEHREVKASETDPWSIAFSTCTRAALKGWKTDPVFQPYFHETGAIVSGHTPSLIKHIEEHEIDSSDAEFVKLNTAEDFRKTMPPGILTGNFPGWKGWLNKTGAGWIHAKKAMFSAYTEAKRLGVTFITGSPEGDVVSLVYENGDVAGARTADGTIHRAEHTILSAGAGSDRLLDFKKQLRPTAWTLCHIKMTPEEAKKYRNLPVLFNVAKGFFMEPDEDKHELKICDAHPGYCNFIPDPKHGGEVRSIPFAKHQIPLEAEARARDFLRDTMPHLADRPLSFARICWDADTVDRAFLIDRHPEYRSLLLAVGGSGNGAMQMSTIGGFITDALEGHLQKELKHALRWRPEIATERDWKDTQNRFGGPNKVMDFQKVGENEWTKIGDDKCRL

SEQ ID NO: 147 - protein, 446 aa, synthetic construct
MASSNLTLTSSILIVGAGTWGCSTALHLARRGYKNVTVLDPHPVPSPIAAGNDINKIMEHREVKASETDPWSIAFSTCTRAALKGWKTDPVFQPYFHETGAIVSGHTPSLIKHIEEHEIDSSDAEFVKLNTAEDFRKTMPPGILTGNFPGWKGWLNKTGAGWIHAKKAMFSAYTEAKRLGVTFITGSPEGDVVSLVYENGDVAGARTADGTIHRAEHTILSAGAGSDRLLDFKKQLRPTAWTLCHIKMTPEEAKKYRNLPVLFNVAKGFFMEPDEDKHELKICDVHPGYCNFIPDPKHGGEVRSIPFAKHQIPLEAEARARDFLRDTMPHLADRPLSFARICWDADTVDRAFLIDRHPEYRSLLLAVGGSGNGAMQMSTIGGFITDALEGHLQKELKHALRWRPEIATERDWKDTQNRFGGPNKVMDFQKVGENEWTKIGDDKCRL

SEQ ID NO: 148 - protein, 446 aa, synthetic construct
MASSNLTLTSSILIVGAGTWGCSTALHLARRGYKNVTVLDPHPVPSPIAAGNDINKIMEHREVKASETDPWSIAFSTCTRAALKGWKTDPVFQPYFHETGAIVSGHTPSLIKHIEEHEIDSSDAEFVKLNTAEDFRKTMPPGILTGNFPGWKGWLNKTGAGWIHAKKAMFSAYTEAKRLGVTFITGSPEGDVVSLVYENGDVAGARTADGTIHRAEHTILSAGAGSDRLLDFKKQLRPTAWTLCHIKMTPEEAKKYRNLPVLFNVAKGFFMEPDEDKHELKICDPHPGYCNFIPDPKHGGEVRSIPFAKHQIPLEAEARARDFLRDTMPHLADRPLSFARICWDADTVDRAFLIDRHPEYRSLLLAVGGSGNGAMQMSTIGGFITDALEGHLQKELKHALRWRPEIATERDWKDTQNRFGGPNKVMDFQKVGENEWTKIGDDKCRL

SEQ ID NO: 149 - protein, 446 aa, synthetic construct
MASSNLTLTSSILIVGAGTWGCSTALHLARRGYKNVTVLDPHPVPSPIAAGNDINKIMEHREVKASETDPWSIAFSTCTRAALKGWKTDPVFQPYFHETGAIVSGHTPSLIKHIEEHEIDSSDAEFVKLNTAEDFRKTMPPGILTGNFPGWKGWLNKTGAGWIHAKKAMFSAYTEAKRLGVTFITGSPEGDVVSLVYENGDVAGARTADGTIHRAEHTILSAGAGSDRLLDFKKQLRPTAWTLCHIKMTPEEAKKYRNLPVLFNVAKGFFMEPDEDKHELKICDLHPGYCNFIPDPKHGGEVRSIPFAKHQIPLEAEARARDFLRDTMPHLADRPLSFARICWDADTVDRAFLIDRHPEYRSLLLAVGGSGNGAMQMSTIGGFITDALEGHLQKELKHALRWRPEIATERDWKDTQNRFGGPNKVMDFQKVGENEWTKIGDDKCRL

SEQ ID NO: 150 - protein, 446 aa, synthetic construct
MASSNLTLTSSILIVGAGTWGCSTALHLARRGYKNVTVLDPHPVPSPIAAGNDINKIMEHREVKASETDPWSIAFSTCTRAALKGWKTDPVFQPYFHETGAIVSGHTPSLIKHIEEHEIDSSDAEFVKLNTAEDFRKTMPPGILTGNFPGWKGWLNKTGAGWIHAKKAMFSAYTEAKRLGVTFITGSPEGDVVSLVYENGDVAGARTADGTIHRAEHTILSAGAGSDRLLDFKKQLRPTAWTLCHIKMTPEEAKKYRNLPVLFNVAKGFFMEPDEDKHELKICDIHPGYCNFIPDPKHGGEVRSIPFAKHQIPLEAEARARDFLRDTMPHLADRPLSFARICWDADTVDRAFLIDRHPEYRSLLLAVGGSGNGAMQMSTIGGFITDALEGHLQKELKHALRWRPEIATERDWKDTQNRFGGPNKVMDFQKVGENEWTKIGDDKCRL

SEQ ID NO: 151 - protein, 446 aa, synthetic construct
MASSNLTLTSSILIVGAGTWGCSTALHLARRGYKNVTVLDPHPVPSPIAAGNDINKIMEHREVKASETDPWSIAFSTCTRAALKGWKTDPVFQPYFHETGAIVSGHTPSLIKHIEEHEIDSSDAEFVKLNTAEDFRKTMPPGILTGNFPGWKGWLNKTGAGWIHAKKAMFSAYTEAKRLGVTFITGSPEGDVVSLVYENGDVAGARTADGTIHRAEHTILSAGAGSDRLLDFKKQLRPTAWTLCHIKMTPEEAKKYRNLPVLFNVAKGFFMEPDEDKHELKICDFHPGYCNFIPDPKHGGEVRSIPFAKHQIPLEAEARARDFLRDTMPHLADRPLSFARICWDADTVDRAFLIDRHPEYRSLLLAVGGSGNGAMQMSTIGGFITDALEGHLQKELKHALRWRPEIATERDWKDTQNRFGGPNKVMDFQKVGENEWTKIGDDKCRL

SEQ ID NO: 152 - protein, 446 aa, synthetic construct; identical to SEQ ID NO: 148

SEQ ID NO: 153 - protein, 446 aa, synthetic construct
MASSNLTLTSSILIVGAGTWGCSTALHLARRGYKNVTVLDPHPVPSPIAAGNDINKIMEHREVKASETDPWSIAFSTCTRAALKGWKTDPVFQPYFHETGAIVSGHTPSLIKHIEEHEIDSSDAEFVKLNTAEDFRKTMPPGILTGNFPGWKGWLNKTGAGWIHAKKAMFSAYTEAKRLGVTFITGSPEGDVVSLVYENGDVAGARTADGTIHRAEHTILSAGAGSDRLLDFKKQLRPTAWTLCHIKMTPEEAKKYRNLPVLFNVAKGFFMEPDEDKHELKICDWHPGYCNFIPDPKHGGEVRSIPFAKHQIPLEAEARARDFLRDTMPHLADRPLSFARICWDADTVDRAFLIDRHPEYRSLLLAVGGSGNGAMQMSTIGGFITDALEGHLQKELKHALRWRPEIATERDWKDTQNRFGGPNKVMDFQKVGENEWTKIGDDKCRL

SEQ ID NO: 154 - protein, 446 aa, synthetic construct
MASSNLTLTSSILIVGAGTWGCSTALHLARRGYKNVTVLDPHPVPSPIAAGNDINKIMEHREVKASETDPWSIAFSTCTRAALKGWKTDPVFQPYFHETGAIVSGHTPSLIKHIEEHEIDSSDAEFVKLNTAEDFRKTMPPGILTGNFPGWKGWLNKTGAGWIHAKKAMFSAYTEAKRLGVTFITGSPEGDVVSLVYENGDVAGARTADGTIHRAEHTILSAGAGSDRLLDFKKQLRPTAWTLCHIKMTPEEAKKYRNLPVLFNVAKGFFMEPDEDKHELKICDEHPGYCNFIPDPKHGGEVRSIPFAKHQIPLEAEARARDFLRDTMPHLADRPLSFARICWDADTVDRAFLIERHPEYRSLLLAVGGSGNGAMQMSTIGGFITDALEGHLQKELKHALRWRPEIATERDWKDTQNRFGGPNKVMDFQKVGENEWTKIGDDKCRL

SEQ ID NO: 155 - protein, 446 aa, synthetic construct
MASSNLTLTSSILIVGAGTWGCSTALHLARRGYKNVTVLDPHPVPSPIAAGNDINKIMEHREVKASETDPWSIAFSTCTRAALKGWKTDPVFQPYFHETGAIVSGHTPSLIKHIEEHEIDSSDAEFVKLNTAEDFRKTMPPGILTGNFPGWKGWLNKTGAGWIHAKKAMFSAYTEAKRLGVTFITGSPEGDVVSLVYENGDVAGARTADGTIHRAEHTILSAGAGSDRLLDFKKQLRPTAWTLCHIKMTPEEAKKYRNLPVLFNVAKGFFMEPDEDKHELKICDEHPGYCNFIPDPKHGGEVRSIPFAKHQIPLEAEARARDFLRDTMPHLADRPLSFARICWDADTVDRAFLIKRHPEYRSLLLAVGGSGNGAMQMSTIGGFITDALEGHLQKELKHALRWRPEIATERDWKDTQNRFGGPNKVMDFQKVGENEWTKIGDDKCRL

SEQ ID NO: 156 - protein, 446 aa, synthetic construct
MASSNLTLTSSILIVGAGTWGCSTALHLARRGYKNVTVLDPHPVPSPIAAGNDINKIMEHREVKASETDPWSIAFSTCTRAALKGWKTDPVFQPYFHETGAIVSGHTPSLIKHIEEHEIDSSDAEFVKLNTAEDFRKTMPPGILTGNFPGWKGWLNKTGAGWIHAKKAMFSAYTEAKRLGVTFITGSPEGDVVSLVYENGDVAGARTADGTIHRAEHTILSAGAGSDRLLDFKKQLRPTAWTLCHIKMTPEEAKKYRNLPVLFNVAKGFFMEPDEDKHELKICDEHPGYCNFIPDPKHGGEVRSIPFAKHQIPLEAEARARDFLRDTMPHLADRPLSFARICWDADTVDRAFLIRRHPEYRSLLLAVGGSGNGAMQMSTIGGFITDALEGHLQKELKHALRWRPEIATERDWKDTQNRFGGPNKVMDFQKVGENEWTKIGDDKCRL

SEQ ID NO: 157 - protein, 446 aa, synthetic construct
MASSNLTLTSSILIVGAGTWGCSTALHLARRGYKNVTVLDPHPVPSPIAAGNDINKIMEHREVKASETDPWSIAFSTCTRAALKGWKTDPVFQPYFHETGAIVSGHTPSLIKHIEEHEIDSSDAEFVKLNTAEDFRKTMPPGILTGNFPGWKGWLNKTGAGWIHAKKAMFSAYTEAKRLGVTFITGSPEGDVVSLVYENGDVAGARTADGTIHRAEHTILSAGAGSDRLLDFKKQLRPTAWTLCHIKMTPEEAKKYRNLPVLFNVAKGFFMEPDEDKHELKICDEHPGYCNFIPDPKHGGEVRSIPFAKHQIPLEAEARARDFLRDTMPHLADRPLSFARICWDADTVDRAFLIHRHPEYRSLLLAVGGSGNGAMQMSTIGGFITDALEGHLQKELKHALRWRPEIATERDWKDTQNRFGGPNKVMDFQKVGENEWTKIGDDKCRL

SEQ ID NO: 158 - protein, 446 aa, synthetic construct
MASSNLTLTSSILIVGAGTWGCSTALHLARRGYKNVTVLDPHPVPSPIAAGNDINKIMEHREVKASETDPWSIAFSTCTRAALKGWKTDPVFQPYFHETGAIVSGHTPSLIKHIEEHEIDSSDAEFVKLNTAEDFRKTMPPGILTGNFPGWKGWLNKTGAGWIHAKKAMFSAYTEAKRLGVTFITGSPEGDVVSLVYENGDVAGARTADGTIHRAEHTILSAGAGSDRLLDFKKQLRPTAWTLCHIKMTPEEAKKYRNLPVLFNVAKGFFMEPDEDKHELKICDEHPGYCNFIPDPKHGGEVRSIPFAKHQIPLEAEARARDFLRDTMPHLADRPLSFARICWDADTVDRAFLINRHPEYRSLLLAVGGSGNGAMQMSTIGGFITDALEGHLQKELKHALRWRPEIATERDWKDTQNRFGGPNKVMDFQKVGENEWTKIGDDKCRL

SEQ ID NO: 159 - protein, 446 aa, synthetic construct
MASSNLTLTSSILIVGAGTWGCSTALHLARRGYKNVTVLDPHPVPSPIAAGNDINKIMEHREVKASETDPWSIAFSTCTRAALKGWKTDPVFQPYFHETGAIVSGHTPSLIKHIEEHEIDSSDAEFVKLNTAEDFRKTMPPGILTGNFPGWKGWLNKTGAGWIHAKKAMFSAYTEAKRLGVTFITGSPEGDVVSLVYENGDVAGARTADGTIHRAEHTILSAGAGSDRLLDFKKQLRPTAWTLCHIKMTPEEAKKYRNLPVLFNVAKGFFMEPDEDKHELKICDEHPGYCNFIPDPKHGGEVRSIPFAKHQIPLEAEARARDFLRDTMPHLADRPLSFARICWDADTVDRAFLIQRHPEYRSLLLAVGGSGNGAMQMSTIGGFITDALEGHLQKELKHALRWRPEIATERDWKDTQNRFGGPNKVMDFQKVGENEWTKIGDDKCRL

SEQ ID NO: 160 - protein, 446 aa, synthetic construct
MASSNLTLTSSILIVGAGTWGCSTALHLARRGYKNVTVLDPHPVPSPIAAGNDINKIMEHREVKASETDPWSIAFSTCTRAALKGWKTDPVFQPYFHETGAIVSGHTPSLIKHIEEHEIDSSDAEFVKLNTAEDFRKTMPPGILTGNFPGWKGWLNKTGAGWIHAKKAMFSAYTEAKRLGVTFITGSPEGDVVSLVYENGDVAGARTADGTIHRAEHTILSAGAGSDRLLDFKKQLRPTAWTLCHIKMTPEEAKKYRNLPVLFNVAKGFFMEPDEDKHELKICDEHPGYCNFIPDPKHGGEVRSIPFAKHQIPLEAEARARDFLRDTMPHLADRPLSFARICWDADTVDRAFLISRHPEYRSLLLAVGGSGNGAMQMSTIGGFITDALEGHLQKELKHALRWRPEIATERDWKDTQNRFGGPNKVMDFQKVGENEWTKIGDDKCRL

SEQ ID NO: 161 - protein, 446 aa, synthetic construct
MASSNLTLTSSILIVGAGTWGCSTALHLARRGYKNVTVLDPHPVPSPIAAGNDINKIMEHREVKASETDPWSIAFSTCTRAALKGWKTDPVFQPYFHETGAIVSGHTPSLIKHIEEHEIDSSDAEFVKLNTAEDFRKTMPPGILTGNFPGWKGWLNKTGAGWIHAKKAMFSAYTEAKRLGVTFITGSPEGDVVSLVYENGDVAGARTADGTIHRAEHTILSAGAGSDRLLDFKKQLRPTAWTLCHIKMTPEEAKKYRNLPVLFNVAKGFFMEPDEDKHELKICDEHPGYCNFIPDPKHGGEVRSIPFAKHQIPLEAEARARDFLRDTMPHLADRPLSFARICWDADTVDRAFLITRHPEYRSLLLAVGGSGNGAMQMSTIGGFITDALEGHLQKELKHALRWRPEIATERDWKDTQNRFGGPNKVMDFQKVGENEWTKIGDDKCRL

SEQ ID NO: 162 - protein, 446 aa, synthetic construct
MASSNLTLTSSILIVGAGTWGCSTALHLARRGYKNVTVLDPHPVPSPIAAGNDINKIMEHREVKASETDPWSIAFSTCTRAALKGWKTDPVFQPYFHETGAIVSGHTPSLIKHIEEHEIDSSDAEFVKLNTAEDFRKTMPPGILTGNFPGWKGWLNKTGAGWIHAKKAMFSAYTEAKRLGVTFITGSPEGDVVSLVYENGDVAGARTADGTIHRAEHTILSAGAGSDRLLDFKKQLRPTAWTLCHIKMTPEEAKKYRNLPVLFNVAKGFFMEPDEDKHELKICDEHPGYCNFIPDPKHGGEVRSIPFAKHQIPLEAEARARDFLRDTMPHLADRPLSFARICWDADTVDRAFLIYRHPEYRSLLLAVGGSGNGAMQMSTIGGFITDALEGHLQKELKHALRWRPEIATERDWKDTQNRFGGPNKVMDFQKVGENEWTKIGDDKCRL

SEQ ID NO: 163 - protein, 446 aa, synthetic construct
MASSNLTLTSSILIVGAGTWGCSTALHLARRGYKNVTVLDPHPVPSPIAAGNDINKIMEHREVKASETDPWSIAFSTCTRAALKGWKTDPVFQPYFHETGAIVSGHTPSLIKHIEEHEIDSSDAEFVKLNTAEDFRKTMPPGILTGNFPGWKGWLNKTGAGWIHAKKAMFSAYTEAKRLGVTFITGSPEGDVVSLVYENGDVAGARTADGTIHRAEHTILSAGAGSDRLLDFKKQLRPTAWTLCHIKMTPEEAKKYRNLPVLFNVAKGFFMEPDEDKHELKICDEHPGYCNFIPDPKHGGEVRSIPFAKHQIPLEAEARARDFLRDTMPHLADRPLSFARICWDADTVDRAFLICRHPEYRSLLLAVGGSGNGAMQMSTIGGFITDALEGHLQKELKHALRWRPEIATERDWKDTQNRFGGPNKVMDFQKVGENEWTKIGDDKCRL

SEQ ID NO: 164 - protein, 446 aa, synthetic construct
MASSNLTLTSSILIVGAGTWGCSTALHLARRGYKNVTVLDPHPVPSPIAAGNDINKIMEHREVKASETDPWSIAFSTCTRAALKGWKTDPVFQPYFHETGAIVSGHTPSLIKHIEEHEIDSSDAEFVKLNTAEDFRKTMPPGILTGNFPGWKGWLNKTGAGWIHAKKAMFSAYTEAKRLGVTFITGSPEGDVVSLVYENGDVAGARTADGTIHRAEHTILSAGAGSDRLLDFKKQLRPTAWTLCHIKMTPEEAKKYRNLPVLFNVAKGFFMEPDEDKHELKICDEHPGYCNFIPDPKHGGEVRSIPFAKHQIPLEAEARARDFLRDTMPHLADRPLSFARICWDADTVDRAFLIGRHPEYRSLLLAVGGSGNGAMQMSTIGGFITDALEGHLQKELKHALRWRPEIATERDWKDTQNRFGGPNKVMDFQKVGENEWTKIGDDKCRL

SEQ ID NO: 165 - protein, 446 aa, synthetic construct
MASSNLTLTSSILIVGAGTWGCSTALHLARRGYKNVTVLDPHPVPSPIAAGNDINKIMEHREVKASETDPWSIAFSTCTRAALKGWKTDPVFQPYFHETGAIVSGHTPSLIKHIEEHEIDSSDAEFVKLNTAEDFRKTMPPGILTGNFPGWKGWLNKTGAGWIHAKKAMFSAYTEAKRLGVTFITGSPEGDVVSLVYENGDVAGARTADGTIHRAEHTILSAGAGSDRLLDFKKQLRPTAWTLCHIKMTPEEAKKYRNLPVLFNVAKGFFMEPDEDKHELKICDEHPGYCNFIPDPKHGGEVRSIPFAKHQIPLEAEARARDFLRDTMPHLADRPLSFARICWDADTVDRAFLIARHPEYRSLLLAVGGSGNGAMQMSTIGGFITDALEGHLQKELKHALRWRPEIATERDWKDTQNRFGGPNKVMDFQKVGENEWTKIGDDKCRL

SEQ ID NO: 166 - protein, 446 aa, synthetic construct
MASSNLTLTSSILIVGAGTWGCSTALHLARRGYKNVTVLDPHPVPSPIAAGNDINKIMEHREVKASETDPWSIAFSTCTRAALKGWKTDPVFQPYFHETGAIVSGHTPSLIKHIEEHEIDSSDAEFVKLNTAEDFRKTMPPGILTGNFPGWKGWLNKTGAGWIHAKKAMFSAYTEAKRLGVTFITGSPEGDVVSLVYENGDVAGARTADGTIHRAEHTILSAGAGSDRLLDFKKQLRPTAWTLCHIKMTPEEAKKYRNLPVLFNVAKGFFMEPDEDKHELKICDEHPGYCNFIPDPKHGGEVRSIPFAKHQIPLEAEARARDFLRDTMPHLADRPLSFARICWDADTVDRAFLIVRHPEYRSLLLAVGGSGNGAMQMSTIGGFITDALEGHLQKELKHALRWRPEIATERDWKDTQNRFGGPNKVMDFQKVGENEWTKIGDDKCRL

SEQ ID NO: 167 - protein, 446 aa, synthetic construct
MASSNLTLTSSILIVGAGTWGCSTALHLARRGYKNVTVLDPHPVPSPIAAGNDINKIMEHREVKASETDPWSIAFSTCTRAALKGWKTDPVFQPYFHETGAIVSGHTPSLIKHIEEHEIDSSDAEFVKLNTAEDFRKTMPPGILTGNFPGWKGWLNKTGAGWIHAKKAMFSAYTEAKRLGVTFITGSPEGDVVSLVYENGDVAGARTADGTIHRAEHTILSAGAGSDRLLDFKKQLRPTAWTLCHIKMTPEEAKKYRNLPVLFNVAKGFFMEPDEDKHELKICDEHPGYCNFIPDPKHGGEVRSIPFAKHQIPLEAEARARDFLRDTMPHLADRPLSFARICWDADTVDRAFLIPRHPEYRSLLLAVGGSGNGAMQMSTIGGFITDALEGHLQKELKHALRWRPEIATERDWKDTQNRFGGPNKVMDFQKVGENEWTKIGDDKCRL

SEQ ID NO: 168 - protein, 446 aa, synthetic construct
MASSNLTLTSSILIVGAGTWGCSTALHLARRGYKNVTVLDPHPVPSPIAAGNDINKIMEHREVKASETDPWSIAFSTCTRAALKGWKTDPVFQPYFHETGAIVSGHTPSLIKHIEEHEIDSSDAEFVKLNTAEDFRKTMPPGILTGNFPGWKGWLNKTGAGWIHAKKAMFSAYTEAKRLGVTFITGSPEGDVVSLVYENGDVAGARTADGTIHRAEHTILSAGAGSDRLLDFKKQLRPTAWTLCHIKMTPEEAKKYRNLPVLFNVAKGFFMEPDEDKHELKICDEHPGYCNFIPDPKHGGEVRSIPFAKHQIPLEAEARARDFLRDTMPHLADRPLSFARICWDADTVDRAFLILRHPEYRSLLLAVGGSGNGAMQMSTIGGFITDALEGHLQKELKHALRWRPEIATERDWKDTQNRFGGPNKVMDFQKVGENEWTKIGDDKCRL

SEQ ID NO: 169 - protein, 446 aa, synthetic construct
MASSNLTLTSSILIVGAGTWGCSTALHLARRGYKNVTVLDPHPVPSPIAAGNDINKIMEHREVKASETDPWSIAFSTCTRAALKGWKTDPVFQPYFHETGAIVSGHTPSLIKHIEEHEIDSSDAEFVKLNTAEDFRKTMPPGILTGNFPGWKGWLNKTGAGWIHAKKAMFSAYTEAKRLGVTFITGSPEGDVVSLVYENGDVAGARTADGTIHRAEHTILSAGAGSDRLLDFKKQLRPTAWTLCHIKMTPEEAKKYRNLPVLFNVAKGFFMEPDEDKHELKICDEHPGYCNFIPDPKHGGEVRSIPFAKHQIPLEAEARARDFLRDTMPHLADRPLSFARICWDADTVDRAFLIIRHPEYRSLLLAVGGSGNGAMQMSTIGGFITDALEGHLQKELKHALRWRPEIATERDWKDTQNRFGGPNKVMDFQKVGENEWTKIGDDKCRL

SEQ ID NO: 170 - protein, 446 aa, synthetic construct
MASSNLTLTSSILIVGAGTWGCSTALHLARRGYKNVTVLDPHPVPSPIAAGNDINKIMEHREVKASETDPWSIAFSTCTRAALKGWKTDPVFQPYFHETGAIVSGHTPSLIKHIEEHEIDSSDAEFVKLNTAEDFRKTMPPGILTGNFPGWKGWLNKTGAGWIHAKKAMFSAYTEAKRLGVTFITGSPEGDVVSLVYENGDVAGARTADGTIHRAEHTILSAGAGSDRLLDFKKQLRPTAWTLCHIKMTPEEAKKYRNLPVLFNVAKGFFMEPDEDKHELKICDEHPGYCNFIPDPKHGGEVRSIPFAKHQIPLEAEARARDFLRDTMPHLADRPLSFARICWDADTVDRAFLIFRHPEYRSLLLAVGGSGNGAMQMSTIGGFITDALEGHLQKELKHALRWRPEIATERDWKDTQNRFGGPNKVMDFQKVGENEWTKIGDDKCRL

SEQ ID NO: 171 - protein, 446 aa, synthetic construct
MASSNLTLTSSILIVGAGTWGCSTALHLARRGYKNVTVLDPHPVPSPIAAGNDINKIMEHREVKASETDPWSIAFSTCTRAALKGWKTDPVFQPYFHETGAIVSGHTPSLIKHIEEHEIDSSDAEFVKLNTAEDFRKTMPPGILTGNFPGWKGWLNKTGAGWIHAKKAMFSAYTEAKRLGVTFITGSPEGDVVSLVYENGDVAGARTADGTIHRAEHTILSAGAGSDRLLDFKKQLRPTAWTLCHIKMTPEEAKKYRNLPVLFNVAKGFFMEPDEDKHELKICDEHPGYCNFIPDPKHGGEVRSIPFAKHQIPLEAEARARDFLRDTMPHLADRPLSFARICWDADTVDRAFLIMRHPEYRSLLLAVGGSGNGAMQMSTIGGFITDALEGHLQKELKHALRWRPEIATERDWKDTQNRFGGPNKVMDFQKVGENEWTKIGDDKCRL

SEQ ID NO: 172 - protein, 446 aa, synthetic construct
MASSNLTLTSSILIVGAGTWGCSTALHLARRGYKNVTVLDPHPVPSPIAAGNDINKIMEHREVKASETDPWSIAFSTCTRAALKGWKTDPVFQPYFHETGAIVSGHTPSLIKHIEEHEIDSSDAEFVKLNTAEDFRKTMPPGILTGNFPGWKGWLNKTGAGWIHAKKAMFSAYTEAKRLGVTFITGSPEGDVVSLVYENGDVAGARTADGTIHRAEHTILSAGAGSDRLLDFKKQLRPTAWTLCHIKMTPEEAKKYRNLPVLFNVAKGFFMEPDEDKHELKICDEHPGYCNFIPDPKHGGEVRSIPFAKHQIPLEAEARARDFLRDTMPHLADRPLSFARICWDADTVDRAFLIWRHPEYRSLLLAVGGSGNGAMQMSTIGGFITDALEGHLQKELKHALRWRPEIATERDWKDTQNRFGGPNKVMDFQKVGENEWTKIGDDKCRL

SEQ ID NO: 173 - protein, 446 aa, synthetic construct
MASSSLTLTSSILIVGAGTWGCSTALHLARRGYKNVTVLDPHPVPSPIAAGNDINKIFEHREVKASETDPWSIAFSTCTRAALKGWKTDPVFQPYFHETGAIVSGHTPSLIKHIEEHEIDSSDAEFVKLNTAEDFRKTMPPGILTGNFPGWKGWLNKTGAGWIHAKKAMFSAYTEAKRLGVTFITGSPEGDVVSLVYENGDVAGARTADGTIHRAEHTILSAGAGSDRLLDFKKQLRPTAWTLCHIKMTPEEAKKYRNLPVLFNVAKGFFMEPDEDKHELKICDEHPGYCNFIPDPKHGGEVRSIPFAKHQIPLEAEARARDFLRDTMPHLADRPLSFARICWDADTVDRAFLIDRHPEYRSLLLAVGGSGNGAMQMSTIGGFITDALEGHLQKELKHALRWRPEIATERDWKDTQNRFGGPNKVMDFQKVGENEWTKIGDDKCRL

SEQ ID NO: 174 - protein, 446 aa, synthetic construct
MASSSLTLTSSILIVGAGTWGCSTALHLARRGYKNVTVLDPHPVPSPIAAGNDINKIMEHREVKASETDPWSIAFSTCTRAALKGWKTDPVFQPYFHETGAIVSGHTPSLIKHIEEHEIDSSDAEFVKLNTAEDFRKTMPPGILTGNFPGWKGWLNKTGAGWIHAKKAMFSAYTEAKRLGVTFITGSPEGDVVSLVYENGDVAGARTADGTIHRAEHTILSAGANSDRLLDFKKQLRPTAWTLCHIKMTPEEAKKYRNLPVLFNVAKGFFMEPDEDKHELKICDEHPGYCNFIPDPKHGGEVRSIPFAKHQIPLEAEARARDFLRDTMPHLADRPLSFARICWDADTVDRAFLIDRHPEYRSLLLAVGGSGNGAMQMSTIGGFITDALEGHLQKELKHALRWRPEIATERDWKDTQNRFGGPNKVMDFQKVGENEWTKIGDDKCRL

SEQ ID NO: 175 - protein, 446 aa, synthetic construct
MASSSLTLTSSILIVGAGTWGCSTALHLARRGYKNVTVLDPHPVPSPIAAGNDINKIMEHREVKASETDPWSIAFSTCTRAALKGWKTDPVFQPYFHETGAIVSGHTPSLIKHIEEHEIDSSDAEFVKLNTAEDFRKTMPPGILTGNFPGWKGWLNKTGAGWIHAKKAMFSAYTEAKRLGVTFITGSPEGDVVSLVYENGDVAGARTADGTIHRAEHTILSAGAASDRLLDFKKQLRPTAWTLCHIKMTPEEAKKYRNLPVLFNVAKGFFMEPDEDKHELKICDEHPGYCNFIPDPKHGGEVRSIPFAKHQIPLEAEARARDFLRDTMPHLADRPLSFARICWDADTVDRAFLIDRHPEYRSLLLAVGGSGNGAMQMSTIGGFITDALEGHLQKELKHALRWRPEIATERDWKDTQNRFGGPNKVMDFQKVGENEWTKIGDDKCRL

SEQ ID NO: 176 - protein, 446 aa, synthetic construct
MASSSLTLTSSILIVGAGTWGCSTALHLARRGYKNVTVLDPHPVPSPIAAGNDINKIMEHREVKASETDPWSIAFSTCTRAALKGWKTDPVFQPYFHETGAIVSGHTPSLIKHIEEHEIDSSDAEFVKLNTAEDFRKTMPPGILTGNFPGWKGWLNKTGAGWIHAKKAMFSAYTEAKRLGVTFITGSPEGDVVSLVYENGDVAGARTADGTIHRAEHTILSAGAGSDRLLDFKKQLRPTAWTLCHIKMTPEEAKKYRNLPVLFNVAKGFFMEPDEDKHELKICDEHPGYCNFIPDPKHGGEVRSIPFAKHQIPLEAEARARDFLRDTMPHLADRPLSFARICWDADTVDRAFLIDRHPEYRSLLLAVGGSGNGAMQMSTIGGFITDALEGHLQKELKHALRWRPEIATERDWKDTQNRFGGPNKVMDFQKVGENEWTKIADDKCRL

SEQ ID NO: 177 - protein, 446 aa, synthetic construct
MASSSLTLTSSILIVGAGTWGCSTALHLARRGYKNVTVLDPHPVPSPIAAGNDINKIMEHREVKASETDPWSIAFSTCTRAALKGWKTDPVFQPYFHETGAIVSGHTPSLIKHIEEHEIDSSDAEFVKLNTAEDFRKTMPPGILTGNFPGWKGWLNKTGAGWIHAKKAMFSAYTEAKRLGVTFITGSPEGDVVSLVYENGDVAGARTADGTIHRAEHTILSAGAGSDRLLDFKKQLRPTAWTLCHIKMTPEEAKKYRNLPVLFNVAKGFFMEPDEDKHELKICDEHPGYCNFIPDPKHGGEVRSIPFAKHQIPLEAEARARDFLRDTMPHLADRPLSFARICWDADTVDRAFLIDRHPEYRSLLLAVGGSGNGAMQMSTIGGFITDALEGHLQKELKHALRWRPEIATERDWKDTQNRFGGPNKVMDFQKVGENEWTKIMDDKCRL

SEQ ID NO: 178 - protein, 446 aa, synthetic construct
MASSLLTLTSSILIVGAGTWGCSTALHLARRGYKNVTVLDPHPVPSPIAAGNDINKIFEHREVKASETDPWSIAFSTCTRAALKGWKTDPVFQPYFHETGAIVSGHTPSLIKHIEEHEIDSSDAEFVKLNTAEDFRKTMPPGILTGNFPGWKGWLNKTGAGWIHAKKAMFSAYTEAKRLGVTFITGSPEGDVVSLVYENGDVAGARTADGTIHRAEHTILSAGAGSDRLLDFKKQLRPTAWTLCHIKMTPEEAKKYRNLPVLFNVAKGFFMEPDEDKHELKICDEHPGYCNFIPDPKHGGEVRSIPFAKHQIPLEAEARARDFLRDTMPHLADRPLSFARICWDADTVDRAFLIDRHPEYRSLLLAVGGSGNGAMQMSTIGGFITDALEGHLQKELKHALRWRPEIATERDWKDTQNRFGGPNKVMDFQKVGENEWTKIGDDKCRL

SEQ ID NO: 179 - protein, 446 aa, synthetic construct
MASSLLTLTSSILIVGAGTWGCSTALHLARRGYKNVTVLDPHPVPSPIAAGNDINKIMEHREVKASETDPWSIAFSTCTRAALKGWKTDPVFQPYFHETGAIVSGHTPSLIKHIEEHEIDSSDAEFVKLNTAEDFRKTMPPGILTGNFPGWKGWLNKTGAGWIHAKKAMFSAYTEAKRLGVTFITGSPEGDVVSLVYENGDVAGARTADGTIHRAEHTILSAGANSDRLLDFKKQLRPTAWTLCHIKMTPEEAKKYRNLPVLFNVAKGFFMEPDEDKHELKICDEHPGYCNFIPDPKHGGEVRSIPFAKHQIPLEAEARARDFLRDTMPHLADRPLSFARICWDADTVDRAFLIDRHPEYRSLLLAVGGSGNGAMQMSTIGGFITDALEGHLQKELKHALRWRPEIATERDWKDTQNRFGGPNKVMDFQKVGENEWTKIGDDKCRL

SEQ ID NO: 180 - protein, 446 aa, synthetic construct
MASSLLTLTSSILIVGAGTWGCSTALHLARRGYKNVTVLDPHPVPSPIAAGNDINKIMEHREVKASETDPWSIAFSTCTRAALKGWKTDPVFQPYFHETGAIVSGHTPSLIKHIEEHEIDSSDAEFVKLNTAEDFRKTMPPGILTGNFPGWKGWLNKTGAGWIHAKKAMFSAYTEAKRLGVTFITGSPEGDVVSLVYENGDVAGARTADGTIHRAEHTILSAGAASDRLLDFKKQLRPTAWTLCHIKMTPEEAKKYRNLPVLFNVAKGFFMEPDEDKHELKICDEHPGYCNFIPDPKHGGEVRSIPFAKHQIPLEAEARARDFLRDTMPHLADRPLSFARICWDADTVDRAFLIDRHPEYRSLLLAVGGSGNGAMQMSTIGGFITDALEGHLQKELKHALRWRPEIATERDWKDTQNRFGGPNKVMDFQKVGENEWTKIGDDKCRL

SEQ ID NO: 181 - protein, 446 aa, synthetic construct; identical to SEQ ID NO: 16

SEQ ID NO: 182 - protein, 446 aa, synthetic construct
MASSLLTLTSSILIVGAGTWGCSTALHLARRGYKNVTVLDPHPVPSPIAAGNDINKIMEHREVKASETDPWSIAFSTCTRAALKGWKTDPVFQPYFHETGAIVSGHTPSLIKHIEEHEIDSSDAEFVKLNTAEDFRKTMPPGILTGNFPGWKGWLNKTGAGWIHAKKAMFSAYTEAKRLGVTFITGSPEGDVVSLVYENGDVAGARTADGTIHRAEHTILSAGAGSDRLLDFKKQLRPTAWTLCHIKMTPEEAKKYRNLPVLFNVAKGFFMEPDEDKHELKICDEHPGYCNFIPDPKHGGEVRSIPFAKHQIPLEAEARARDFLRDTMPHLADRPLSFARICWDADTVDRAFLIDRHPEYRSLLLAVGGSGNGAMQMSTIGGFITDALEGHLQKELKHALRWRPEIATERDWKDTQNRFGGPNKVMDFQKVGENEWTKIDDDKCRL

SEQ ID NO: 183 - protein, 446 aa, synthetic construct
MASSLLTLTSSILIVGAGTWGCSTALHLARRGYKNVTVLDPHPVPSPIAAGNDINKIMEHREVKASETDPWSIAFSTCTRAALKGWKTDPVFQPYFHETGAIVSGHTPSLIKHIEEHEIDSSDAEFVKLNTAEDFRKTMPPGILTGNFPGWKGWLNKTGAGWIHAKKAMFSAYTEAKRLGVTFITGSPEGDVVSLVYENGDVAGARTADGTIHRAEHTILSAGAGSDRLLDFKKQLRPTAWTLCHIKMTPEEAKKYRNLPVLFNVAKGFFMEPDEDKHELKICDEHPGYCNFIPDPKHGGEVRSIPFAKHQIPLEAEARARDFLRDTMPHLADRPLSFARICWDADTVDRAFLIDRHPEYRSLLLAVGGSGNGAMQMSTIGGFITDALEGHLQKELKHALRWRPEIATERDWKDTQNRFGGPNKVMDFQKVGENEWTKIADDKCRL

SEQ ID NO: 184 - protein, 446 aa, synthetic construct
MASSLLTLTSSILIVGAGTWGCSTALHLARRGYKNVTVLDPHPVPSPIAAGNDINKIMEHREVKASETDPWSIAFSTCTRAALKGWKTDPVFQPYFHETGAIVSGHTPSLIKHIEEHEIDSSDAEFVKLNTAEDFRKTMPPGILTGNFPGWKGWLNKTGAGWIHAKKAMFSAYTEAKRLGVTFITGSPEGDVVSLVYENGDVAGARTADGTIHRAEHTILSAGAGSDRLLDFKKQLRPTAWTLCHIKMTPEEAKKYRNLPVLFNVAKGFFMEPDEDKHELKICDEHPGYCNFIPDPKHGGEVRSIPFAKHQIPLEAEARARDFLRDTMPHLADRPLSFARICWDADTVDRAFLIDRHPEYRSLLLAVGGSGNGAMQMSTIGGFITDALEGHLQKELKHALRWRPEIATERDWKDTQNRFGGPNKVMDFQKVGENEWTKIMDDKCRL

SEQ ID NO: 185 - protein, 446 aa, synthetic construct
MASSNLTLTSSILIVGAGTWGCSTALHLARRGYKNVTVLDPHPVPSPIAAGNDINKIFEHREVKASETDPWSIAFSTCTRAALKGWKTDPVFQPYFHETGAIVSGHTPSLIKHIEEHEIDSSDAEFVKLNTAEDFRKTMPPGILTGNFPGWKGWLNKTGAGWIHAKKAMFSAYTEAKRLGVTFITGSPEGDVVSLVYENGDVAGARTADGTIHRAEHTILSAGANSDRLLDFKKQLRPTAWTLCHIKMTPEEAKKYRNLPVLFNVAKGFFMEPDEDKHELKICDEHPGYCNFIPDPKHGGEVRSIPFAKHQIPLEAEARARDFLRDTMPHLADRPLSFARICWDADTVDRAFLIDRHPEYRSLLLAVGGSGNGAMQMSTIGGFITDALEGHLQKELKHALRWRPEIATERDWKDTQNRFGGPNKVMDFQKVGENEWTKIGDDKCRL

SEQ ID NO: 186 - protein, 446 aa, synthetic construct
MASSNLTLTSSILIVGAGTWGCSTALHLARRGYKNVTVLDPHPVPSPIAAGNDINKIFEHREVKASETDPWSIAFSTCTRAALKGWKTDPVFQPYFHETGAIVSGHTPSLIKHIEEHEIDSSDAEFVKLNTAEDFRKTMPPGILTGNFPGWKGWLNKTGAGWIHAKKAMFSAYTEAKRLGVTFITGSPEGDVVSLVYENGDVAGARTADGTIHRAEHTILSAGAASDRLLDFKKQLRPTAWTLCHIKMTPEEAKKYRNLPVLFNVAKGFFMEPDEDKHELKICDEHPGYCNFIPDPKHGGEVRSIPFAKHQIPLEAEARARDFLRDTMPHLADRPLSFARICWDADTVDRAFLIDRHPEYRSLLLAVGGSGNGAMQMSTIGGFITDALEGHLQKELKHALRWRPEIATERDWKDTQNRFGGPNKVMDFQKVGENEWTKIGDDKCRL

SEQ ID NO: 187 - protein, 446 aa, synthetic construct; identical to SEQ ID NO: 38

SEQ ID NO: 188 - protein, 446 aa, synthetic construct
MASSNLTLTSSILIVGAGTWGCSTALHLARRGYKNVTVLDPHPVPSPIAAGNDINKIFEHREVKASETDPWSIAFSTCTRAALKGWKTDPVFQPYFHETGAIVSGHTPSLIKHIEEHEIDSSDAEFVKLNTAEDFRKTMPPGILTGNFPGWKGWLNKTGAGWIHAKKAMFSAYTEAKRLGVTFITGSPEGDVVSLVYENGDVAGARTADGTIHRAEHTILSAGAGSDRLLDFKKQLRPTAWTLCHIKMTPEEAKKYRNLPVLFNVAKGFFMEPDEDKHELKICDEHPGYCNFIPDPKHGGEVRSIPFAKHQIPLEAEARARDFLRDTMPHLADRPLSFARICWDADTVDRAFLIDRHPEYRSLLLAVGGSGNGAMQMSTIGGFITDALEGHLQKELKHALRWRPEIATERDWKDTQNRFGGPNKVMDFQKVGENEWTKIDDDKCRL

SEQ ID NO: 189 - protein, 446 aa, synthetic construct
MASSNLTLTSSILIVGAGTWGCSTALHLARRGYKNVTVLDPHPVPSPIAAGNDINKIFEHREVKASETDPWSIAFSTCTRAALKGWKTDPVFQPYFHETGAIVSGHTPSLIKHIEEHEIDSSDAEFVKLNTAEDFRKTMPPGILTGNFPGWKGWLNKTGAGWIHAKKAMFSAYTEAKRLGVTFITGSPEGDVVSLVYENGDVAGARTADGTIHRAEHTILSAGAGSDRLLDFKKQLRPTAWTLCHIKMTPEEAKKYRNLPVLFNVAKGFFMEPDEDKHELKICDEHPGYCNFIPDPKHGGEVRSIPFAKHQIPLEAEARARDFLRDTMPHLADRPLSFARICWDADTVDRAFLIDRHPEYRSLLLAVGGSGNGAMQMSTIGGFITDALEGHLQKELKHALRWRPEIATERDWKDTQNRFGGPNKVMDFQKVGENEWTKIADDKCRL

SEQ ID NO: 190 - protein, 446 aa, synthetic construct
MASSNLTLTSSILIVGAGTWGCSTALHLARRGYKNVTVLDPHPVPSPIAAGNDINKIFEHREVKASETDPWSIAFSTCTRAALKGWKTDPVFQPYFHETGAIVSGHTPSLIKHIEEHEIDSSDAEFVKLNTAEDFRKTMPPGILTGNFPGWKGWLNKTGAGWIHAKKAMFSAYTEAKRLGVTFITGSPEGDVVSLVYENGDVAGARTADGTIHRAEHTILSAGAGSDRLLDFKKQLRPTAWTLCHIKMTPEEAKKYRNLPVLFNVAKGFFMEPDEDKHELKICDEHPGYCNFIPDPKHGGEVRSIPFAKHQIPLEAEARARDFLRDTMPHLADRPLSFARICWDADTVDRAFLIDRHPEYRSLLLAVGGSGNGAMQMSTIGGFITDALEGHLQKELKHALRWRPEIATERDWKDTQNRFGGPNKVMDFQKVGENEWTKIMDDKCRL

SEQ ID NO: 191 - protein, 446 aa, synthetic construct
MASSNLTLTSSILIVGAGTWGCSTALHLARRGYKNVTVLDPHPVPSPIAAGNDINKIMEHREVKASETDPWSIAFSTCTRAALKGWKTDPVFQPYFHETGAIVSGHTPSLIKHIEEHEIDSSDAEFVKLNTAEDFRKTMPPGILTGNFPGWKGWLNKTGAGWIHAKKAMFSAYTEAKRLGVTFITGSPEGDVVSLVYENGDVAGARTADGTIHRAEHTILSAGANSDRLLDFKKQLRPTAWTLCHIKMTPEEAKKYRNLPVLFNVAKGFFMEPDEDKHELKICDEHPGYCNFIPDPKHGGEVRSIPFAKHQIPLEAEARARDFLRDTMPHLADRPLSFARICWDADTVDRAFLIDRHPEYRSLLLAVGGSGNGAMQMSTIGGFITDALEGHLQKELKHALRWRPEIATERDWKDTQNRFGGPNKVMDFQKVGENEWTKIADDKCRL

SEQ ID NO: 192 - protein, 446 aa, synthetic construct
MASSNLTLTSSILIVGAGTWGCSTALHLARRGYKNVTVLDPHPVPSPIAAGNDINKIMEHREVKASETDPWSIAFSTCTRAALKGWKTDPVFQPYFHETGAIVSGHTPSLIKHIEEHEIDSSDAEFVKLNTAEDFRKTMPPGILTGNFPGWKGWLNKTGAGWIHAKKAMFSAYTEAKRLGVTFITGSPEGDVVSLVYENGDVAGARTADGTIHRAEHTILSAGANSDRLLDFKKQLRPTAWTLCHIKMTPEEAKKYRNLPVLFNVAKGFFMEPDEDKHELKICDEHPGYCNFIPDPKHGGEVRSIPFAKHQIPLEAEARARDFLRDTMPHLADRPLSFARICWDADTVDRAFLIDRHPEYRSLLLAVGGSGNGAMQMSTIGGFITDALEGHLQKELKHALRWRPEIATERDWKDTQNRFGGPNKVMDFQKVGENEWTKIMDDKCRL

SEQ ID NO: 193 - protein, 446 aa, synthetic construct
MASSNLTLTSSILIVGAGTWGCSTALHLARRGYKNVTVLDPHPVPSPIAAGNDINKIMEHREVKASETDPWSIAFSTCTRAALKGWKTDPVFQPYFHETGAIVSGHTPSLIKHIEEHEIDSSDAEFVKLNTAEDFRKTMPPGILTGNFPGWKGWLNKTGAGWIHAKKAMFSAYTEAKRLGVTFITGSPEGDVVSLVYENGDVAGARTADGTIHRAEHTILSAGANSDRLLDFKKQLRPTAWTLCHIKMTPEEAKKYRNLPVLFNVAKGFFMEPDEDYHELKICDEHPGYCNFIPDPKHGGEVRSIPFAKHQIPLEAEARARDFLRDTMPHLADRPLSFARICWDADTVDRAFLIDRHPEYRSLLLAVGGSGNGAMQMSTIGGFITDALEGHLQKELKHALRWRPEIATERDWKDTQNRFGGPNKVMDFQKVGENEWTKIGDDKCRL

SEQ ID NO: 194 - protein, 446 aa, synthetic construct
MASSNLTLTSSILIVGAGTWGCSTALHLARRGYKNVTVLDPHPVPSPIAAGNDINKIMEHREVKASETDPWSIAFSTCTRAALKGWKTDPVFQPYFHETGAIVSGHTPSLIKHIEEHEIDSSDAEFVKLNTAEDFRKTMPPGILTGNFPGWKGWLNKTGAGWIHAKKAMFSAYTEAKRLGVTFITGSPEGDVVSLVYENGDVAGARTADGTIHRAEHTILSAGANSDRLLDFKKQLRPTAWTLCHIKMTPEEAKKYRNLPVLFNVAKGFFMEPDEDKHELKICDEHPGYCNFIPDPKHGGEVRSIPFAKHQIPLEAEARARDFLRDTMPHLADRPLSFARICWDADTVDRAFLIDRHPEYRSLLLAVGGSGNGAMQMSTIGGFITDALEGHLQKELKHALRWRPEIATERDWKDTQNRFGGPNKVMDFQKVGENEWTKIDDDKCRL

SEQ ID NO: 195 - protein, 446 aa, synthetic construct
MASSNLTLTSSILIVGAGTWGCSTALHLARRGYKNVTVLDPHPVPSPIAAGNDINKIMEHREVKASETDPWSIAFSTCTRAALKGWKTDPVFQPYFHETGAIVSGHTPSLIKHIEEHEIDSSDAEFVKLNTAEDFRKTMPPGILTGNFPGWKGWLNKTGAGWIHAKKAMFSAYTEAKRLGVTFITGSPEGDVVSLVYENGDVAGARTADGTIHRAEHTILSAGAASDRLLDFKKQLRPTAWTLCHIKMTPEEAKKYRNLPVLFNVAKGFFMEPDEDKHELKICDEHPGYCNFIPDPKHGGEVRSIPFAKHQIPLEAEARARDFLRDTMPHLADRPLSFARICWDADTVDRAFLIDRHPEYRSLLLAVGGSGNGAMQMSTIGGFITDALEGHLQKELKHALRWRPEIATERDWKDTQNRFGGPNKVMDFQKVGENEWTKIADDKCRL

SEQ ID NO: 196 - protein, 446 aa, synthetic construct
MASSNLTLTSSILIVGAGTWGCSTALHLARRGYKNVTVLDPHPVPSPIAAGNDINKIMEHREVKASETDPWSIAFSTCTRAALKGWKTDPVFQPYFHETGAIVSGHTPSLIKHIEEHEIDSSDAEFVKLNTAEDFRKTMPPGILTGNFPGWKGWLNKTGAGWIHAKKAMFSAYTEAKRLGVTFITGSPEGDVVSLVYENGDVAGARTADGTIHRAEHTILSAGAASDRLLDFKKQLRPTAWTLCHIKMTPEEAKKYRNLPVLFNVAKGFFMEPDEDKHELKICDEHPGYCNFIPDPKHGGEVRSIPFAKHQIPLEAEARARDFLRDTMPHLADRPLSFARICWDADTVDRAFLIDRHPEYRSLLLAVGGSGNGAMQMSTIGGFITDALEGHLQKELKHALRWRPEIATERDWKDTQNRFGGPNKVMDFQKVGENEWTKIMDDKCRL

SEQ ID NO: 197 - protein, 446 aa, synthetic construct
MASSNLTLTSSILIVGAGTWGCSTALHLARRGYKNVTVLDPHPVPSPIAAGNDINKIMEHREVKASETDPWSIAFSTCTRAALKGWKTDPVFQPYFHETGAIVSGHTPSLIKHIEEHEIDSSDAEFVKLNTAEDFRKTMPPGILTGNFPGWKGWLNKTGAGWIHAKKAMFSAYTEAKRLGVTFITGSPEGDVVSLVYENGDVAGARTADGTIHRAEHTILSAGAGSDRLLDFKKQLRPTAWTLCHIKMTPEEAKKYRNLPVLFNVAKGFFMEPDEDYHELKICDEHPGYCNFIPDPKHGGEVRSIPFAKHQIPLEAEARARDFLRDTMPHLADRPLSFARICWDADTVDRAFLIDRHPEYRSLLLAVGGSGNGAMQMSTIGGFITDALEGHLQKELKHALRWRPEIATERDWKDTQNRFGGPNKVMDFQKVGENEWTKIDDDKCRL

SEQ ID NO: 198 - protein, 446 aa, synthetic construct; identical to SEQ ID NO: 179

SEQ ID NO: 199 - protein, 445 aa, Aspergillus fumigatus
MAPSILSTESSIIVIGAGTWGCSTALHLARRGYKDVTVLDPHPVPSPIAAGNDINKIMEHSELKDGSSDPRSAAFSTFTRAALKAWKTDPVFQPYFHETGFIISGHTPALIDHIRKDEVEPSETNFVKLETAEDFRRTMPPGVLTGDFPGWKGWLHKSGAGWIHAKKAMISAFNEAKRLGVRFVTGSPEGNVVSLVYEDGDVVGARTADGRVHKAHRTILSAGAGSDSLLDFKKQLRPTAWTLCHIQMGPEEVKQYRNLPVLFNIAKGFFMEPDEDKHELKICDEHPGYCNFLPDPNRPGQEKSVPFAKHQIPLEAEARARDFLHDTMPHLADRPLSFARICWDADTPDRAFLIDRHPEHPSLLVAVGGSGNGAMQMPTIGGFIADALESKLQKEVKDIVRWRPETAVDRDWRATQNRFGGPDRIMDFQQVGEDQWTKIGESRGP

SEQ ID NO: 200 - protein, 445 aa, synthetic construct
MAPSILSTESSIIVIGAGTWGCSTALHLARRGYKDVTVLDPHPVPSPIAAGNDINKIDEHSELKDGSSDPRSAAFSTFTRAALKAWKTDPVFQPYFHETGFIISGHTPALIDHIRKDEVEPSETNFVKLETAEDFRRTMPPGVLTGDFPGWKGWLHKSGAGWIHAKKAMISAFNEAKRLGVRFVTGSPEGNVVSLVYEDGDVVGARTADGRVHKAHRTILSAGAGSDSLLDFKKQLRPTAWTLCHIQMGPEEVKQYRNLPVLFNIAKGFFMEPDEDKHELKICDEHPGYCNFLPDPNRPGQEKSVPFAKHQIPLEAEARARDFLHDTMPHLADRPLSFARICWDADTPDRAFLIDRHPEHPSLLVAVGGSGNGAMQMPTIGGFIADALESKLQKEVKDIVRWRPETAVDRDWRATQNRFGGPDRIMDFQQVGEDQWTKIGESRGP

SEQ ID NO: 201 - protein, 445 aa, synthetic construct
MAPSILSTESSIIVIGAGTWGCSTALHLARRGYKDVTVLDPHPVPSPIAAGNDINKIEEHSELKDGSSDPRSAAFSTFTRAALKAWKTDPVFQPYFHETGFIISGHTPALIDHIRKDEVEPSETNFVKLETAEDFRRTMPPGVLTGDFPGWKGWLHKSGAGWIHAKKAMISAFNEAKRLGVRFVTGSPEGNVVSLVYEDGDVVGARTADGRVHKAHRTILSAGAGSDSLLDFKKQLRPTAWTLCHIQMGPEEVKQYRNLPVLFNIAKGFFMEPDEDKHELKICDEHPGYCNFLPDPNRPGQEKSVPFAKHQIPLEAEARARDFLHDTMPHLADRPLSFARICWDADTPDRAFLIDRHPEHPSLLVAVGGSGNGAMQMPTIGGFIADALESKLQKEVKDIVRWRPETAVDRDWRATQNRFGGPDRIMDFQQVGEDQWTKIGESRGP

SEQ ID NO: 202 - protein, 445 aa, synthetic construct
MAPSILSTESSIIVIGAGTWGCSTALHLARRGYKDVTVLDPHPVPSPIAAGNDINKIKEHSELKDGSSDPRSAAFSTFTRAALKAWKTDPVFQPYFHETGFIISGHTPALIDHIRKDEVEPSETNFVKLETAEDFRRTMPPGVLTGDFPGWKGWLHKSGAGWIHAKKAMISAFNEAKRLGVRFVTGSPEGNVVSLVYEDGDVVGARTADGRVHKAHRTILSAGAGSDSLLDFKKQLRPTAWTLCHIQMGPEEVKQYRNLPVLFNIAKGFFMEPDEDKHELKICDEHPGYCNFLPDPNRPGQEKSVPFAKHQIPLEAEARARDFLHDTMPHLADRPLSFARICWDADTPDRAFLIDRHPEHPSLLVAVGGSGNGAMQMPTIGGFIADALESKLQKEVKDIVRWRPETAVDRDWRATQNRFGGPDRIMDFQQVGEDQWTKIGESRGP

SEQ ID NO: 203 - protein, 445 aa, synthetic construct
MAPSILSTESSIIVIGAGTWGCSTALHLARRGYKDVTVLDPHPVPSPIAAGNDINKIREHSELKDGSSDPRSAAFSTFTRAALKAWKTDPVFQPYFHETGFIISGHTPALIDHIRKDEVEPSETNFVKLETAEDFRRTMPPGVLTGDFPGWKGWLHKSGAGWIHAKKAMISAFNEAKRLGVRFVTGSPEGNVVSLVYEDGDVVGARTADGRVHKAHRTILSAGAGSDSLLDFKKQLRPTAWTLCHIQMGPEEVKQYRNLPVLFNIAKGFFMEPDEDKHELKICDEHPGYCNFLPDPNRPGQEKSVPFAKHQIPLEAEARARDFLHDTMPHLADRPLSFARICWDADTPDRAFLIDRHPEHPSLLVAVGGSGNGAMQMPTIGGFIADALESKLQKEVKDIVRWRPETAVDRDWRATQNRFGGPDRIMDFQQVGEDQWTKIGESRGP

SEQ ID NO: 204 - protein, 445 aa, synthetic construct
MAPSILSTESSIIVIGAGTWGCSTALHLARRGYKDVTVLDPHPVPSPIAAGNDINKIHEHSELKDGSSDPRSAAFSTFTRAALKAWKTDPVFQPYFHETGFIISGHTPALIDHIRKDEVEPSETNFVKLETAEDFRRTMPPGVLTGDFPGWKGWLHKSGAGWIHAKKAMISAFNEAKRLGVRFVTGSPEGNVVSLVYEDGDVVGARTADGRVHKAHRTILSAGAGSDSLLDFKKQLRPTAWTLCHIQMGPEEVKQYRNLPVLFNIAKGFFMEPDEDKHELKICDEHPGYCNFLPDPNRPGQEKSVPFAKHQIPLEAEARARDFLHDTMPHLADRPLSFARICWDADTPDRAFLIDRHPEHPSLLVAVGGSGNGAMQMPTIGGFIADALESKLQKEVKDIVRWRPETAVDRDWRATQNRFGGPDRIMDFQQVGEDQWTKIGESRGP

SEQ ID NO: 205 - protein, 445 aa, synthetic construct
MAPSILSTESSIIVIGAGTWGCSTALHLARRGYKDVTVLDPHPVPSPIAAGNDINKINEHSELKDGSSDPRSAAFSTFTRAALKAWKTDPVFQPYFHETGFIISGHTPALIDHIRKDEVEPSETNFVKLETAEDFRRTMPPGVLTGDFPGWKGWLHKSGAGWIHAKKAMISAFNEAKRLGVRFVTGSPEGNVVSLVYEDGDVVGARTADGRVHKAHRTILSAGAGSDSLLDFKKQLRPTAWTLCHIQMGPEEVKQYRNLPVLFNIAKGFFMEPDEDKHELKICDEHPGYCNFLPDPNRPGQEKSVPFAKHQIPLEAEARARDFLHDTMPHLADRPLSFARICWDADTPDRAFLIDRHPEHPSLLVAVGGSGNGAMQMPTIGGFIADALESKLQKEVKDIVRWRPETAVDRDWRATQNRFGGPDRIMDFQQVGEDQWTKIGESRGP

SEQ ID NO: 206 - protein, 445 aa, synthetic construct
MAPSILSTESSIIVIGAGTWGCSTALHLARRGYKDVTVLDPHPVPSPIAAGNDINKIQEHSELKDGSSDPRSAAFSTFTRAALKAWKTDPVFQPYFHETGFIISGHTPALIDHIRKDEVEPSETNFVKLETAEDFRRTMPPGVLTGDFPGWKGWLHKSGAGWIHAKKAMISAFNEAKRLGVRFVTGSPEGNVVSLVYEDGDVVGARTADGRVHKAHRTILSAGAGSDSLLDFKKQLRPTAWTLCHIQMGPEEVKQYRNLPVLFNIAKGFFMEPDEDKHELKICDEHPGYCNFLPDPNRPGQEKSVPFAKHQIPLEAEARARDFLHDTMPHLADRPLSFARICWDADTPDRAFLIDRHPEHPSLLVAVGGSGNGAMQMPTIGGFIADALESKLQKEVKDIVRWRPETAVDRDWRATQNRFGGPDRIMDFQQVGEDQWTKIGESRGP

SEQ ID NO: 207 - protein, 445 aa, synthetic construct
MAPSILSTESSIIVIGAGTWGCSTALHLARRGYKDVTVLDPHPVPSPIAAGNDINKISEHSELKDGSSDPRSAAFSTFTRAALKAWKTDPVFQPYFHETGFIISGHTPALIDHIRKDEVEPSETNFVKLETAEDFRRTMPPGVLTGDFPGWKGWLHKSGAGWIHAKKAMISAFNEAKRLGVRFVTGSPEGNVVSLVYEDGDVVGARTADGRVHKAHRTILSAGAGSDSLLDFKKQLRPTAWTLCHIQMGPEEVKQYRNLPVLFNIAKGFFMEPDEDKHELKICDEHPGYCNFLPDPNRPGQEKSVPFAKHQIPLEAEARARDFLHDTMPHLADRPLSFARICWDADTPDRAFLIDRHPEHPSLLVAVGGSGNGAMQMPTIGGFIADALESKLQKEVKDIVRWRPETAVDRDWRATQNRFGGPDRIMDFQQVGEDQWTKIGESRGP

SEQ ID NO: 208 - protein, 445 aa, synthetic construct
MAPSILSTESSIIVIGAGTWGCSTALHLARRGYKDVTVLDPHPVPSPIAAGNDINKITEHSELKDGSSDPRSAAFSTFTRAALKAWKTDPVFQPYFHETGFIISGHTPALIDHIRKDEVEPSETNFVKLETAEDFRRTMPPGVLTGDFPGWKGWLHKSGAGWIHAKKAMISAFNEAKRLGVRFVTGSPEGNVVSLVYEDGDVVGARTADGRVHKAHRTILSAGAGSDSLLDFKKQLRPTAWTLCHIQMGPEEVKQYRNLPVLFNIAKGFFMEPDEDKHELKICDEHPGYCNFLPDPNRPGQEKSVPFAKHQIPLEAEARARDFLHDTMPHLADRPLSFARICWDADTPDRAFLIDRHPEHPSLLVAVGGSGNGAMQMPTIGGFIADALESKLQKEVKDIVRWRPETAVDRDWRATQNRFGGPDRIMDFQQVGEDQWTKIGESRGP

SEQ ID NO: 209 - protein, 445 aa, synthetic construct
MAPSILSTESSIIVIGAGTWGCSTALHLARRGYKDVTVLDPHPVPSPIAAGNDINKIYEHSELKDGSSDPRSAAFSTFTRAALKAWKTDPVFQPYFHETGFIISGHTPALIDHIRKDEVEPSETNFVKLETAEDFRRTMPPGVLTGDFPGWKGWLHKSGAGWIHAKKAMISAFNEAKRLGVRFVTGSPEGNVVSLVYEDGDVVGARTADGRVHKAHRTILSAGAGSDSLLDFKKQLRPTAWTLCHIQMGPEEVKQYRNLPVLFNIAKGFFMEPDEDKHELKICDEHPGYCNFLPDPNRPGQEKSVPFAKHQIPLEAEARARDFLHDTMPHLADRPLSFARICWDADTPDRAFLIDRHPEHPSLLVAVGGSGNGAMQMPTIGGFIADALESKLQKEVKDIVRWRPETAVDRDWRATQNRFGGPDRIMDFQQVGEDQWTKIGESRGP

SEQ ID NO: 210 - protein, 445 aa, synthetic construct
MAPSILSTESSIIVIGAGTWGCSTALHLARRGYKDVTVLDPHPVPSPIAAGNDINKICEHSELKDGSSDPRSAAFSTFTRAALKAWKTDPVFQPYFHETGFIISGHTPALIDHIRKDEVEPSETNFVKLETAEDFRRTMPPGVLTGDFPGWKGWLHKSGAGWIHAKKAMISAFNEAKRLGVRFVTGSPEGNVVSLVYEDGDVVGARTADGRVHKAHRTILSAGAGSDSLLDFKKQLRPTAWTLCHIQMGPEEVKQYRNLPVLFNIAKGFFMEPDEDKHELKICDEHPGYCNFLPDPNRPGQEKSVPFAKHQIPLEAEARARDFLHDTMPHLADRPLSFARICWDADTPDRAFLIDRHPEHPSLLVAVGGSGNGAMQMPTIGGFIADALESKLQKEVKDIVRWRPETAVDRDWRATQNRFGGPDRIMDFQQVGEDQWTKIGESRGP

SEQ ID NO: 211 - protein, 445 aa, synthetic construct
MAPSILSTESSIIVIGAGTWGCSTALHLARRGYKDVTVLDPHPVPSPIAAGNDINKIGEHSELKDGSSDPRSAAFSTFTRAALKAWKTDPVFQPYFHETGFIISGHTPALIDHIRKDEVEPSETNFVKLETAEDFRRTMPPGVLTGDFPGWKGWLHKSGAGWIHAKKAMISAFNEAKRLGVRFVTGSPEGNVVSLVYEDGDVVGARTADGRVHKAHRTILSAGAGSDSLLDFKKQLRPTAWTLCHIQMGPEEVKQYRNLPVLFNIAKGFFMEPDEDKHELKICDEHPGYCNFLPDPNRPGQEKSVPFAKHQIPLEAEARARDFLHDTMPHLADRPLSFARICWDADTPDRAFLIDRHPEHPSLLVAVGGSGNGAMQMPTIGGFIADALESKLQKEVKDIVRWRPETAVDRDWRATQNRFGGPDRIMDFQQVGEDQWTKIGESRGP

SEQ ID NO: 212 - protein, 445 aa, synthetic construct
MAPSILSTESSIIVIGAGTWGCSTALHLARRGYKDVTVLDPHPVPSPIAAGNDINKIAEHSELKDGSSDPRSAAFSTFTRAALKAWKTDPVFQPYFHETGFIISGHTPALIDHIRKDEVEPSETNFVKLETAEDFRRTMPPGVLTGDFPGWKGWLHKSGAGWIHAKKAMISAFNEAKRLGVRFVTGSPEGNVVSLVYEDGDVVGARTADGRVHKAHRTILSAGAGSDSLLDFKKQLRPTAWTLCHIQMGPEEVKQYRNLPVLFNIAKGFFMEPDEDKHELKICDEHPGYCNFLPDPNRPGQEKSVPFAKHQIPLEAEARARDFLHDTMPHLADRPLSFARICWDADTPDRAFLIDRHPEHPSLLVAVGGSGNGAMQMPTIGGFIADALESKLQKEVKDIVRWRPETAVDRDWRATQNRFGGPDRIMDFQQVGEDQWTKIGESRGP

SEQ ID NO: 213 - protein, 445 aa, synthetic construct
MAPSILSTESSIIVIGAGTWGCSTALHLARRGYKDVTVLDPHPVPSPIAAGNDINKIVEHSELKDGSSDPRSAAFSTFTRAALKAWKTDPVFQPYFHETGFIISGHTPALIDHIRKDEVEPSETNFVKLETAEDFRRTMPPGVLTGDFPGWKGWLHKSGAGWIHAKKAMISAFNEAKRLGVRFVTGSPEGNVVSLVYEDGDVVGARTADGRVHKAHRTILSAGAGSDSLLDFKKQLRPTAWTLCHIQMGPEEVKQYRNLPVLFNIAKGFFMEPDEDKHELKICDEHPGYCNFLPDPNRPGQEKSVPFAKHQIPLEAEARARDFLHDTMPHLADRPLSFARICWDADTPDRAFLIDRHPEHPSLLVAVGGSGNGAMQMPTIGGFIADALESKLQKEVKDIVRWRPETAVDRDWRATQNRFGGPDRIMDFQQVGEDQWTKIGESRGP

SEQ ID NO: 214 - protein, 445 aa, synthetic construct
MAPSILSTESSIIVIGAGTWGCSTALHLARRGYKDVTVLDPHPVPSPIAAGNDINKIPEHSELKDGSSDPRSAAFSTFTRAALKAWKTDPVFQPYFHETGFIISGHTPALIDHIRKDEVEPSETNFVKLETAEDFRRTMPPGVLTGDFPGWKGWLHKSGAGWIHAKKAMISAFNEAKRLGVRFVTGSPEGNVVSLVYEDGDVVGARTADGRVHKAHRTILSAGAGSDSLLDFKKQLRPTAWTLCHIQMGPEEVKQYRNLPVLFNIAKGFFMEPDEDKHELKICDEHPGYCNFLPDPNRPGQEKSVPFAKHQIPLEAEARARDFLHDTMPHLADRPLSFARICWDADTPDRAFLIDRHPEHPSLLVAVGGSGNGAMQMPTIGGFIADALESKLQKEVKDIVRWRPETAVDRDWRATQNRFGGPDRIMDFQQVGEDQWTKIGESRGP

SEQ ID NO: 215 - protein, 445 aa, synthetic construct
MAPSILSTESSIIVIGAGTWGCSTALHLARRGYKDVTVLDPHPVPSPIAAGNDINKILEHSELKDGSSDPRSAAFSTFTRAALKAWKTDPVFQPYFHETGFIISGHTPALIDHIRKDEVEPSETNFVKLETAEDFRRTMPPGVLTGDFPGWKGWLHKSGAGWIHAKKAMISAFNEAKRLGVRFVTGSPEGNVVSLVYEDGDVVGARTADGRVHKAHRTILSAGAGSDSLLDFKKQLRPTAWTLCHIQMGPEEVKQYRNLPVLFNIAKGFFMEPDEDKHELKICDEHPGYCNFLPDPNRPGQEKSVPFAKHQIPLEAEARARDFLHDTMPHLADRPLSFARICWDADTPDRAFLIDRHPEHPSLLVAVGGSGNGAMQMPTIGGFIADALESKLQKEVKDIVRWRPETAVDRDWRATQNRFGGPDRIMDFQQVGEDQWTKIGESRGP

SEQ ID NO: 216 - protein, 445 aa, synthetic construct
MAPSILSTESSIIVIGAGTWGCSTALHLARRGYKDVTVLDPHPVPSPIAAGNDINKIIEHSELKDGSSDPRSAAFSTFTRAALKAWKTDPVFQPYFHETGFIISGHTPALIDHIRKDEVEPSETNFVKLETAEDFRRTMPPGVLTGDFPGWKGWLHKSGAGWIHAKKAMISAFNEAKRLGVRFVTGSPEGNVVSLVYEDGDVVGARTADGRVHKAHRTILSAGAGSDSLLDFKKQLRPTAWTLCHIQMGPEEVKQYRNLPVLFNIAKGFFMEPDEDKHELKICDEHPGYCNFLPDPNRPGQEKSVPFAKHQIPLEAEARARDFLHDTMPHLADRPLSFARICWDADTPDRAFLIDRHPEHPSLLVAVGGSGNGAMQMPTIGGFIADALESKLQKEVKDIVRWRPETAVDRDWRATQNRFGGPDRIMDFQQVGEDQWTKIGESRGP

SEQ ID NO: 217 - protein, 445 aa, synthetic construct
MAPSILSTESSIIVIGAGTWGCSTALHLARRGYKDVTVLDPHPVPSPIAAGNDINKIFEHSELKDGSSDPRSAAFSTFTRAALKAWKTDPVFQPYFHETGFIISGHTPALIDHIRKDEVEPSETNFVKLETAEDFRRTMPPGVLTGDFPGWKGWLHKSGAGWIHAKKAMISAFNEAKRLGVRFVTGSPEGNVVSLVYEDGDVVGARTADGRVHKAHRTILSAGAGSDSLLDFKKQLRPTAWTLCHIQMGPEEVKQYRNLPVLFNIAKGFFMEPDEDKHELKICDEHPGYCNFLPDPNRPGQEKSVPFAKHQIPLEAEARARDFLHDTMPHLADRPLSFARICWDADTPDRAFLIDRHPEHPSLLVAVGGSGNGAMQMPTIGGFIADALESKLQKEVKDIVRWRPETAVDRDWRATQNRFGGPDRIMDFQQVGEDQWTKIGESRGP

SEQ ID NO: 218 - protein, 445 aa, synthetic construct
MAPSILSTESSIIVIGAGTWGCSTALHLARRGYKDVTVLDPHPVPSPIAAGNDINKIWEHSELKDGSSDPRSAAFSTFTRAALKAWKTDPVFQPYFHETGFIISGHTPALIDHIRKDEVEPSETNFVKLETAEDFRRTMPPGVLTGDFPGWKGWLHKSGAGWIHAKKAMISAFNEAKRLGVRFVTGSPEGNVVSLVYEDGDVVGARTADGRVHKAHRTILSAGAGSDSLLDFKKQLRPTAWTLCHIQMGPEEVKQYRNLPVLFNIAKGFFMEPDEDKHELKICDEHPGYCNFLPDPNRPGQEKSVPFAKHQIPLEAEARARDFLHDTMPHLADRPLSFARICWDADTPDRAFLIDRHPEHPSLLVAVGGSGNGAMQMPTIGGFIADALESKLQKEVKDIVRWRPETAVDRDWRATQNRFGGPDRIMDFQQVGEDQWTKIGESRGP